European Patent Specification EP 3 473 707 B1, published December 18, 2024. Title: Methods for engineering allogeneic and immunosuppressive resistant T cell for immunotherapy. Applicant: CELLECTIS. The sequence listing filed with the application follows.

SEQUENCE LISTING (170 sequences)

SEQ ID NO: 1 - DNA, 49 bp, Artificialsequence
  GRex2
tattcactgatggactccaaagaatcattaactcctggtagagaagaaa

SEQ ID NO: 2 - DNA, 49 bp, Artificialsequence
  GRex3T2
tgcctggtgtgctctgatgaagcttcaggatgtcattatggagtcttaa

SEQ ID NO: 3 - DNA, 49 bp, Artificialsequence
  GRex3T4
tgctctgatgaagcttcaggatgtcattatggagtcttaacttgtggaa

SEQ ID NO: 4 - DNA, 49 bp, Artificialsequence
  GRex5T1
tggtgtcactgttggaggttattgaacctgaagtgttatatgcaggata

SEQ ID NO: 5 - DNA, 49 bp, Artificialsequence
  GRex5T2
tatgatagctctgttccagactcaacttggaggatcatgactacgctca

SEQ ID NO: 6 - DNA, 49 bp, Artificialsequence
  GRex5T3
ttatatgcaggatatgatagctctgttccagactcaacttggaggatca

SEQ ID NO: 7 - protein, 530 aa, Artificialsequence
  Repeat-GRex2-LPT9-L1
LTPEQVVAIASNIGGKQALETVQALLPVLCQAHGLTPQQVVAIASNGGGKQALETVQRLLPVLCQAHGLTPQQVVAIASNGGGKQALETVQRLLPVLCQAHGLTPEQVVAIASHDGGKQALETVQRLLPVLCQAHGLTPEQVVAIASNIGGKQALETVQALLPVLCQAHGLTPEQVVAIASHDGGKQALETVQRLLPVLCQAHGLTPQQVVAIASNGGGKQALETVQRLLPVLCQAHGLTPQQVVAIASNNGGKQALETVQRLLPVLCQAHGLTPEQVVAIASNIGGKQALETVQALLPVLCQAHGLTPQQVVAIASNGGGKQALETVQRLLPVLCQAHGLTPQQVVAIASNNGGKQALETVQRLLPVLCQAHGLTPQQVVAIASNNGGKQALETVQRLLPVLCQAHGLTPEQVVAIASNIGGKQALETVQALLPVLCQAHGLTPEQVVAIASHDGGKQALETVQRLLPVLCQAHGLTPQQVVAIASNGGGKQALETVQRLLPVLCQAHGLTPQQVVAIASNGGGRPALE

SEQ ID NO: 8 - protein, 530 aa, Artificialsequence
  Repeat-GRex2-LPT9-R1
LTPQQVVAIASNGGGKQALETVQRLLPVLCQAHGLTPQQVVAIASNGGGKQALETVQRLLPVLCQAHGLTPEQVVAIASHDGGKQALETVQRLLPVLCQAHGLTPQQVVAIASNGGGKQALETVQRLLPVLCQAHGLTPQQVVAIASNGGGKQALETVQRLLPVLCQAHGLTPEQVVAIASHDGGKQALETVQRLLPVLCQAHGLTPQQVVAIASNGGGKQALETVQRLLPVLCQAHGLTPEQVVAIASHDGGKQALETVQRLLPVLCQAHGLTPQQVVAIASNGGGKQALETVQRLLPVLCQAHGLTPEQVVAIASNIGGKQALETVQALLPVLCQAHGLTPEQVVAIASHDGGKQALETVQRLLPVLCQAHGLTPEQVVAIASHDGGKQALETVQRLLPVLCQAHGLTPEQVVAIASNIGGKQALETVQALLPVLCQAHGLTPQQVVAIASNNGGKQALETVQRLLPVLCQAHGLTPQQVVAIASNNGGKQALETVQRLLPVLCQAHGLTPQQVVAIASNGGGRPALE

SEQ ID NO: 9 - protein, 530 aa, Artificialsequence
  Repeat-GRex3T2-L1
LTPQQVVAIASNNGGKQALETVQRLLPVLCQAHGLTPEQVVAIASHDGGKQALETVQRLLPVLCQAHGLTPEQVVAIASHDGGKQALETVQRLLPVLCQAHGLTPQQVVAIASNGGGKQALETVQRLLPVLCQAHGLTPQQVVAIASNNGGKQALETVQRLLPVLCQAHGLTPQQVVAIASNNGGKQALETVQRLLPVLCQAHGLTPQQVVAIASNGGGKQALETVQRLLPVLCQAHGLTPQQVVAIASNNGGKQALETVQRLLPVLCQAHGLTPQQVVAIASNGGGKQALETVQRLLPVLCQAHGLTPQQVVAIASNNGGKQALETVQRLLPVLCQAHGLTPEQVVAIASHDGGKQALETVQRLLPVLCQAHGLTPQQVVAIASNGGGKQALETVQRLLPVLCQAHGLTPEQVVAIASHDGGKQALETVQRLLPVLCQAHGLTPQQVVAIASNGGGKQALETVQRLLPVLCQAHGLTPQQVVAIASNNGGKQALETVQRLLPVLCQAHGLTPQQVVAIASNGGGRPALE

SEQ ID NO: 10 - protein, 530 aa, Artificialsequence
  Repeat-GRex3T2-R1
LTPQQVVAIASNGGGKQALETVQRLLPVLCQAHGLTPEQVVAIASNIGGKQALETVQALLPVLCQAHGLTPEQVVAIASNIGGKQALETVQALLPVLCQAHGLTPQQVVAIASNNGGKQALETVQRLLPVLCQAHGLTPEQVVAIASNIGGKQALETVQALLPVLCQAHGLTPEQVVAIASHDGGKQALETVQRLLPVLCQAHGLTPQQVVAIASNGGGKQALETVQRLLPVLCQAHGLTPEQVVAIASHDGGKQALETVQRLLPVLCQAHGLTPEQVVAIASHDGGKQALETVQRLLPVLCQAHGLTPEQVVAIASNIGGKQALETVQALLPVLCQAHGLTPQQVVAIASNGGGKQALETVQRLLPVLCQAHGLTPEQVVAIASNIGGKQALETVQALLPVLCQAHGLTPEQVVAIASNIGGKQALETVQALLPVLCQAHGLTPQQVVAIASNGGGKQALETVQRLLPVLCQAHGLTPQQVVAIASNNGGKQALETVQRLLPVLCQAHGLTPQQVVAIASNGGGRPALE

SEQ ID NO: 11 - protein, 530 aa, Artificialsequence
  Repeat-GRex3T4-L1
LTPQQVVAIASNNGGKQALETVQRLLPVLCQAHGLTPEQVVAIASHDGGKQALETVQRLLPVLCQAHGLTPQQVVAIASNGGGKQALETVQRLLPVLCQAHGLTPEQVVAIASHDGGKQALETVQRLLPVLCQAHGLTPQQVVAIASNGGGKQALETVQRLLPVLCQAHGLTPQQVVAIASNNGGKQALETVQRLLPVLCQAHGLTPEQVVAIASNIGGKQALETVQALLPVLCQAHGLTPQQVVAIASNGGGKQALETVQRLLPVLCQAHGLTPQQVVAIASNNGGKQALETVQRLLPVLCQAHGLTPEQVVAIASNIGGKQALETVQALLPVLCQAHGLTPEQVVAIASNIGGKQALETVQALLPVLCQAHGLTPQQVVAIASNNGGKQALETVQRLLPVLCQAHGLTPEQVVAIASHDGGKQALETVQRLLPVLCQAHGLTPQQVVAIASNGGGKQALETVQRLLPVLCQAHGLTPQQVVAIASNGGGKQALETVQRLLPVLCQAHGLTPQQVVAIASNGGGRPALE

SEQ ID NO: 12 - protein, 530 aa, Artificialsequence
  Repeat-GRex3T4-R1
LTPQQVVAIASNGGGKQALETVQRLLPVLCQAHGLTPEQVVAIASHDGGKQALETVQRLLPVLCQAHGLTPEQVVAIASHDGGKQALETVQRLLPVLCQAHGLTPEQVVAIASNIGGKQALETVQALLPVLCQAHGLTPEQVVAIASHDGGKQALETVQRLLPVLCQAHGLTPEQVVAIASNIGGKQALETVQALLPVLCQAHGLTPEQVVAIASNIGGKQALETVQALLPVLCQAHGLTPQQVVAIASNNGGKQALETVQRLLPVLCQAHGLTPQQVVAIASNGGGKQALETVQRLLPVLCQAHGLTPQQVVAIASNGGGKQALETVQRLLPVLCQAHGLTPEQVVAIASNIGGKQALETVQALLPVLCQAHGLTPEQVVAIASNIGGKQALETVQALLPVLCQAHGLTPQQVVAIASNNGGKQALETVQRLLPVLCQAHGLTPEQVVAIASNIGGKQALETVQALLPVLCQAHGLTPEQVVAIASHDGGKQALETVQRLLPVLCQAHGLTPQQVVAIASNGGGRPALE

SEQ ID NO: 13 - protein, 530 aa, Artificialsequence
  Repeat-GRex5T1-LPT8-L1
LTPQQVVAIASNNGGKQALETVQRLLPVLCQAHGLTPQQVVAIASNNGGKQALETVQRLLPVLCQAHGLTPQQVVAIASNGGGKQALETVQRLLPVLCQAHGLTPQQVVAIASNNGGKQALETVQRLLPVLCQAHGLTPQQVVAIASNGGGKQALETVQRLLPVLCQAHGLTPEQVVAIASHDGGKQALETVQRLLPVLCQAHGLTPEQVVAIASNIGGKQALETVQALLPVLCQAHGLTPEQVVAIASHDGGKQALETVQRLLPVLCQAHGLTPQQVVAIASNGGGKQALETVQRLLPVLCQAHGLTPQQVVAIASNNGGKQALETVQRLLPVLCQAHGLTPQQVVAIASNGGGKQALETVQRLLPVLCQAHGLTPQQVVAIASNGGGKQALETVQRLLPVLCQAHGLTPQQVVAIASNNGGKQALETVQRLLPVLCQAHGLTPQQVVAIASNNGGKQALETVQRLLPVLCQAHGLTPEQVVAIASNIGGKQALETVQALLPVLCQAHGLTPQQVVAIASNGGGRPALE

SEQ ID NO: 14 - protein, 530 aa, Artificialsequence
  Repeat-GRex5T1-LPT8-R1
LTPEQVVAIASNIGGKQALETVQALLPVLCQAHGLTPQQVVAIASNGGGKQALETVQRLLPVLCQAHGLTPEQVVAIASHDGGKQALETVQRLLPVLCQAHGLTPEQVVAIASHDGGKQALETVQRLLPVLCQAHGLTPQQVVAIASNGGGKQALETVQRLLPVLCQAHGLTPQQVVAIASNNGGKQALETVQRLLPVLCQAHGLTPEQVVAIASHDGGKQALETVQRLLPVLCQAHGLTPEQVVAIASNIGGKQALETVQALLPVLCQAHGLTPQQVVAIASNGGGKQALETVQRLLPVLCQAHGLTPEQVVAIASNIGGKQALETVQALLPVLCQAHGLTPQQVVAIASNGGGKQALETVQRLLPVLCQAHGLTPEQVVAIASNIGGKQALETVQALLPVLCQAHGLTPEQVVAIASNIGGKQALETVQALLPVLCQAHGLTPEQVVAIASHDGGKQALETVQRLLPVLCQAHGLTPEQVVAIASNIGGKQALETVQALLPVLCQAHGLTPQQVVAIASNGGGRPALE

SEQ ID NO: 15 - protein, 530 aa, Artificialsequence
  Repeat-GRex5T2-L1
LTPEQVVAIASNIGGKQALETVQALLPVLCQAHGLTPQQVVAIASNGGGKQALETVQRLLPVLCQAHGLTPQQVVAIASNNGGKQALETVQRLLPVLCQAHGLTPEQVVAIASNIGGKQALETVQALLPVLCQAHGLTPQQVVAIASNGGGKQALETVQRLLPVLCQAHGLTPEQVVAIASNIGGKQALETVQALLPVLCQAHGLTPQQVVAIASNNGGKQALETVQRLLPVLCQAHGLTPEQVVAIASHDGGKQALETVQRLLPVLCQAHGLTPQQVVAIASNGGGKQALETVQRLLPVLCQAHGLTPEQVVAIASHDGGKQALETVQRLLPVLCQAHGLTPQQVVAIASNGGGKQALETVQRLLPVLCQAHGLTPQQVVAIASNNGGKQALETVQRLLPVLCQAHGLTPQQVVAIASNGGGKQALETVQRLLPVLCQAHGLTPQQVVAIASNGGGKQALETVQRLLPVLCQAHGLTPEQVVAIASHDGGKQALETVQRLLPVLCQAHGLTPQQVVAIASNGGGRPALE

SEQ ID NO: 16 - protein, 530 aa, Artificialsequence
  Repeat-GRex5T2-R1
LTPQQVVAIASNNGGKQALETVQRLLPVLCQAHGLTPEQVVAIASNIGGKQALETVQALLPVLCQAHGLTPQQVVAIASNNGGKQALETVQRLLPVLCQAHGLTPEQVVAIASHDGGKQALETVQRLLPVLCQAHGLTPQQVVAIASNNGGKQALETVQRLLPVLCQAHGLTPQQVVAIASNGGGKQALETVQRLLPVLCQAHGLTPEQVVAIASNIGGKQALETVQALLPVLCQAHGLTPQQVVAIASNNGGKQALETVQRLLPVLCQAHGLTPQQVVAIASNGGGKQALETVQRLLPVLCQAHGLTPEQVVAIASHDGGKQALETVQRLLPVLCQAHGLTPEQVVAIASNIGGKQALETVQALLPVLCQAHGLTPQQVVAIASNGGGKQALETVQRLLPVLCQAHGLTPQQVVAIASNNGGKQALETVQRLLPVLCQAHGLTPEQVVAIASNIGGKQALETVQALLPVLCQAHGLTPQQVVAIASNGGGKQALETVQRLLPVLCQAHGLTPQQVVAIASNGGGRPALE

SEQ ID NO: 17 - protein, 530 aa, Artificialsequence
  Repeat-GRex5T3-L1
LTPQQVVAIASNGGGKQALETVQRLLPVLCQAHGLTPEQVVAIASNIGGKQALETVQALLPVLCQAHGLTPQQVVAIASNGGGKQALETVQRLLPVLCQAHGLTPEQVVAIASNIGGKQALETVQALLPVLCQAHGLTPQQVVAIASNGGGKQALETVQRLLPVLCQAHGLTPQQVVAIASNNGGKQALETVQRLLPVLCQAHGLTPEQVVAIASHDGGKQALETVQRLLPVLCQAHGLTPEQVVAIASNIGGKQALETVQALLPVLCQAHGLTPQQVVAIASNNGGKQALETVQRLLPVLCQAHGLTPQQVVAIASNNGGKQALETVQRLLPVLCQAHGLTPEQVVAIASNIGGKQALETVQALLPVLCQAHGLTPQQVVAIASNGGGKQALETVQRLLPVLCQAHGLTPEQVVAIASNIGGKQALETVQALLPVLCQAHGLTPQQVVAIASNGGGKQALETVQRLLPVLCQAHGLTPQQVVAIASNNGGKQALETVQRLLPVLCQAHGLTPQQVVAIASNGGGRPALE

SEQ ID NO: 18 - protein, 530 aa, Artificialsequence
  Repeat-GRex5T3-R1
LTPQQVVAIASNNGGKQALETVQRLLPVLCQAHGLTPEQVVAIASNIGGKQALETVQALLPVLCQAHGLTPQQVVAIASNGGGKQALETVQRLLPVLCQAHGLTPEQVVAIASHDGGKQALETVQRLLPVLCQAHGLTPEQVVAIASHDGGKQALETVQRLLPVLCQAHGLTPQQVVAIASNGGGKQALETVQRLLPVLCQAHGLTPEQVVAIASHDGGKQALETVQRLLPVLCQAHGLTPEQVVAIASHDGGKQALETVQRLLPVLCQAHGLTPEQVVAIASNIGGKQALETVQALLPVLCQAHGLTPEQVVAIASNIGGKQALETVQALLPVLCQAHGLTPQQVVAIASNNGGKQALETVQRLLPVLCQAHGLTPQQVVAIASNGGGKQALETVQRLLPVLCQAHGLTPQQVVAIASNGGGKQALETVQRLLPVLCQAHGLTPQQVVAIASNNGGKQALETVQRLLPVLCQAHGLTPEQVVAIASNIGGKQALETVQALLPVLCQAHGLTPQQVVAIASNGGGRPALE

SEQ ID NO: 19 - DNA, 2814 bp, Artificialsequence
  GRex2-L TALEN
atgggcgatcctaaaaagaaacgtaaggtcatcgattacccatacgatgttccagattacgctatcgatatcgccgatctacgcacgctcggctacagccagcagcaacaggagaagatcaaaccgaaggttcgttcgacagtggcgcagcaccacgaggcactggtcggccacgggtttacacacgcgcacatcgttgcgttaagccaacacccggcagcgttagggaccgtcgctgtcaagtatcaggacatgatcgcagcgttgccagaggcgacacacgaagcgatcgttggcgtcggcaaacagtggtccggcgcacgcgctctggaggccttgctcacggtggcgggagagttgagaggtccaccgttacagttggacacaggccaacttctcaagattgcaaaacgtggcggcgtgaccgcagtggaggcagtgcatgcatggcgcaatgcactgacgggtgccccgctcaacttgaccccggagcaggtggtggccatcgccagcaatattggtggcaagcaggcgctggagacggtgcaggcgctgttgccggtgctgtgccaggcccacggcttgaccccccagcaggtggtggccatcgccagcaatggcggtggcaagcaggcgctggagacggtccagcggctgttgccggtgctgtgccaggcccacggcttgaccccccagcaggtggtggccatcgccagcaatggcggtggcaagcaggcgctggagacggtccagcggctgttgccggtgctgtgccaggcccacggcttgaccccggagcaggtggtggccatcgccagccacgatggcggcaagcaggcgctggagacggtccagcggctgttgccggtgctgtgccaggcccacggcttgaccccggagcaggtggtggccatcgccagcaatattggtggcaagcaggcgctggagacggtgcaggcgctgttgccggtgctgtgccaggcccacggcttgaccccggagcaggtggtggccatcgccagccacgatggcggcaagcaggcgctggagacggtccagcggctgttgccggtgctgtgccaggcccacggcttgaccccccagcaggtggtggccatcgccagcaatggcggtggcaagcaggcgctggagacggtccagcggctgttgccggtgctgtgccaggcccacggcttgaccccccagcaggtggtggccatcgccagcaataatggtggcaagcaggcgctggagacggtccagcggctgttgccggtgctgtgccaggcccacggcttgaccccggagcaggtggtggccatcgccagcaatattggtggcaagcaggcgctggagacggtgcaggcgctgttgccggtgctgtgccaggcccacggcttgaccccccagcaggtggtggccatcgccagcaatggcggtggcaagcaggcgctggagacggtccagcggctgttgccggtgctgtgccaggcccacggcttgaccccccagcaggtggtggccatcgccagcaataatggtggcaagcaggcgctggagacggtccagcggctgttgccggtgctgtgccaggcccacggcttgaccccccagcaggtggtggccatcgccagcaataatggtggcaagcaggcgctggagacggtccagcggctgttgccggtgctgtgccaggcccacggcttgaccccggagcaggtggtggccatcgccagcaatattggtggcaagcaggcgctggagacggtgcaggcgctgttgccggtgctgtgccaggcccacggcttgaccccggagcaggtggtggccatcgccagccacgatggcggcaagcaggcgctggagacggtccagcggctgttgccggtgctgtgccaggcccacggcttgaccccccagcaggtggtggccatcgccagcaatggcggtggcaagcaggcgctggagacggtccagcggctgttgccggtgctgtgccaggcccacggcttgacccctcagcaggtggtggccatcgccagcaatggcggcggcaggccggcgctggagagcattgttgcccagttatctcgccctgatccggcgttggccgcgttgaccaacgaccacctcgtcgccttggcctgcctcggcgggcgtcctgcgctggatgcagtgaaaaagggattgggggatcctatcagccgttcccagctggtgaagtccgagctggaggagaagaaatccgagttgaggcacaagctgaagtacgtgccccacgagtacatcgagctgatcgagatcgcccggaacagcacccaggaccgtatcctggagatgaaggtgatggagttcttcatgaaggtgtacggctacaggggcaagcacctgggcggctccaggaagcccgacggcgccatctacaccgtgggctcccccatcgactacggcgtgatcgtggacaccaaggcctactccggcggctacaacctgcccatcggccaggccgacgaaatgcagaggtacgtggaggagaaccagaccaggaacaagcacatcaaccccaacgagtggtggaaggtgtacccctccagcgtgaccgagttcaagttcctgttcgtgtccggccacttcaagggcaactacaaggcccagctgaccaggctgaaccacatcaccaactgcaacggcgccgtgctgtccgtggaggagctcctgatcggcggcgagatgatcaaggccggcaccctgaccctggaggaggtgaggaggaagttcaacaacggcgagatcaacttcgcggccgactgataa

SEQ ID NO: 20 - DNA, 2832 bp, Artificialsequence
  GRex2-R TALEN
atgggcgatcctaaaaagaaacgtaaggtcatcgataaggagaccgccgctgccaagttcgagagacagcacatggacagcatcgatatcgccgatctacgcacgctcggctacagccagcagcaacaggagaagatcaaaccgaaggttcgttcgacagtggcgcagcaccacgaggcactggtcggccacgggtttacacacgcgcacatcgttgcgttaagccaacacccggcagcgttagggaccgtcgctgtcaagtatcaggacatgatcgcagcgttgccagaggcgacacacgaagcgatcgttggcgtcggcaaacagtggtccggcgcacgcgctctggaggccttgctcacggtggcgggagagttgagaggtccaccgttacagttggacacaggccaacttctcaagattgcaaaacgtggcggcgtgaccgcagtggaggcagtgcatgcatggcgcaatgcactgacgggtgccccgctcaacttgaccccccagcaggtggtggccatcgccagcaatggcggtggcaagcaggcgctggagacggtccagcggctgttgccggtgctgtgccaggcccacggcttgaccccccagcaggtggtggccatcgccagcaatggcggtggcaagcaggcgctggagacggtccagcggctgttgccggtgctgtgccaggcccacggcttgaccccggagcaggtggtggccatcgccagccacgatggcggcaagcaggcgctggagacggtccagcggctgttgccggtgctgtgccaggcccacggcttgaccccccagcaggtggtggccatcgccagcaatggcggtggcaagcaggcgctggagacggtccagcggctgttgccggtgctgtgccaggcccacggcttgaccccccagcaggtggtggccatcgccagcaatggcggtggcaagcaggcgctggagacggtccagcggctgttgccggtgctgtgccaggcccacggcttgaccccggagcaggtggtggccatcgccagccacgatggcggcaagcaggcgctggagacggtccagcggctgttgccggtgctgtgccaggcccacggcttgaccccccagcaggtggtggccatcgccagcaatggcggtggcaagcaggcgctggagacggtccagcggctgttgccggtgctgtgccaggcccacggcttgaccccggagcaggtggtggccatcgccagccacgatggcggcaagcaggcgctggagacggtccagcggctgttgccggtgctgtgccaggcccacggcttgaccccccagcaggtggtggccatcgccagcaatggcggtggcaagcaggcgctggagacggtccagcggctgttgccggtgctgtgccaggcccacggcttgaccccggagcaggtggtggccatcgccagcaatattggtggcaagcaggcgctggagacggtgcaggcgctgttgccggtgctgtgccaggcccacggcttgaccccggagcaggtggtggccatcgccagccacgatggcggcaagcaggcgctggagacggtccagcggctgttgccggtgctgtgccaggcccacggcttgaccccggagcaggtggtggccatcgccagccacgatggcggcaagcaggcgctggagacggtccagcggctgttgccggtgctgtgccaggcccacggcttgaccccggagcaggtggtggccatcgccagcaatattggtggcaagcaggcgctggagacggtgcaggcgctgttgccggtgctgtgccaggcccacggcttgaccccccagcaggtggtggccatcgccagcaataatggtggcaagcaggcgctggagacggtccagcggctgttgccggtgctgtgccaggcccacggcttgaccccccagcaggtggtggccatcgccagcaataatggtggcaagcaggcgctggagacggtccagcggctgttgccggtgctgtgccaggcccacggcttgacccctcagcaggtggtggccatcgccagcaatggcggcggcaggccggcgctggagagcattgttgcccagttatctcgccctgatccggcgttggccgcgttgaccaacgaccacctcgtcgccttggcctgcctcggcgggcgtcctgcgctggatgcagtgaaaaagggattgggggatcctatcagccgttcccagctggtgaagtccgagctggaggagaagaaatccgagttgaggcacaagctgaagtacgtgccccacgagtacatcgagctgatcgagatcgcccggaacagcacccaggaccgtatcctggagatgaaggtgatggagttcttcatgaaggtgtacggctacaggggcaagcacctgggcggctccaggaagcccgacggcgccatctacaccgtgggctcccccatcgactacggcgtgatcgtggacaccaaggcctactccggcggctacaacctgcccatcggccaggccgacgaaatgcagaggtacgtggaggagaaccagaccaggaacaagcacatcaaccccaacgagtggtggaaggtgtacccctccagcgtgaccgagttcaagttcctgttcgtgtccggccacttcaagggcaactacaaggcccagctgaccaggctgaaccacatcaccaactgcaacggcgccgtgctgtccgtggaggagctcctgatcggcggcgagatgatcaaggccggcaccctgaccctggaggaggtgaggaggaagttcaacaacggcgagatcaacttcgcggccgactgataa

SEQ ID NO: 21 - DNA, 2814 bp, Artificialsequence
  GRex3T2-L TALEN
atgggcgatcctaaaaagaaacgtaaggtcatcgattacccatacgatgttccagattacgctatcgatatcgccgatctacgcacgctcggctacagccagcagcaacaggagaagatcaaaccgaaggttcgttcgacagtggcgcagcaccacgaggcactggtcggccacgggtttacacacgcgcacatcgttgcgttaagccaacacccggcagcgttagggaccgtcgctgtcaagtatcaggacatgatcgcagcgttgccagaggcgacacacgaagcgatcgttggcgtcggcaaacagtggtccggcgcacgcgctctggaggccttgctcacggtggcgggagagttgagaggtccaccgttacagttggacacaggccaacttctcaagattgcaaaacgtggcggcgtgaccgcagtggaggcagtgcatgcatggcgcaatgcactgacgggtgccccgctcaacttgaccccccagcaggtggtggccatcgccagcaataatggtggcaagcaggcgctggagacggtccagcggctgttgccggtgctgtgccaggcccacggcttgaccccggagcaggtggtggccatcgccagccacgatggcggcaagcaggcgctggagacggtccagcggctgttgccggtgctgtgccaggcccacggcttgaccccggagcaggtggtggccatcgccagccacgatggcggcaagcaggcgctggagacggtccagcggctgttgccggtgctgtgccaggcccacggcttgaccccccagcaggtggtggccatcgccagcaatggcggtggcaagcaggcgctggagacggtccagcggctgttgccggtgctgtgccaggcccacggcttgaccccccagcaggtggtggccatcgccagcaataatggtggcaagcaggcgctggagacggtccagcggctgttgccggtgctgtgccaggcccacggcttgaccccccagcaggtggtggccatcgccagcaataatggtggcaagcaggcgctggagacggtccagcggctgttgccggtgctgtgccaggcccacggcttgaccccccagcaggtggtggccatcgccagcaatggcggtggcaagcaggcgctggagacggtccagcggctgttgccggtgctgtgccaggcccacggcttgaccccccagcaggtggtggccatcgccagcaataatggtggcaagcaggcgctggagacggtccagcggctgttgccggtgctgtgccaggcccacggcttgaccccccagcaggtggtggccatcgccagcaatggcggtggcaagcaggcgctggagacggtccagcggctgttgccggtgctgtgccaggcccacggcttgaccccccagcaggtggtggccatcgccagcaataatggtggcaagcaggcgctggagacggtccagcggctgttgccggtgctgtgccaggcccacggcttgaccccggagcaggtggtggccatcgccagccacgatggcggcaagcaggcgctggagacggtccagcggctgttgccggtgctgtgccaggcccacggcttgaccccccagcaggtggtggccatcgccagcaatggcggtggcaagcaggcgctggagacggtccagcggctgttgccggtgctgtgccaggcccacggcttgaccccggagcaggtggtggccatcgccagccacgatggcggcaagcaggcgctggagacggtccagcggctgttgccggtgctgtgccaggcccacggcttgaccccccagcaggtggtggccatcgccagcaatggcggtggcaagcaggcgctggagacggtccagcggctgttgccggtgctgtgccaggcccacggcttgaccccccagcaggtggtggccatcgccagcaataatggtggcaagcaggcgctggagacggtccagcggctgttgccggtgctgtgccaggcccacggcttgacccctcagcaggtggtggccatcgccagcaatggcggcggcaggccggcgctggagagcattgttgcccagttatctcgccctgatccggcgttggccgcgttgaccaacgaccacctcgtcgccttggcctgcctcggcgggcgtcctgcgctggatgcagtgaaaaagggattgggggatcctatcagccgttcccagctggtgaagtccgagctggaggagaagaaatccgagttgaggcacaagctgaagtacgtgccccacgagtacatcgagctgatcgagatcgcccggaacagcacccaggaccgtatcctggagatgaaggtgatggagttcttcatgaaggtgtacggctacaggggcaagcacctgggcggctccaggaagcccgacggcgccatctacaccgtgggctcccccatcgactacggcgtgatcgtggacaccaaggcctactccggcggctacaacctgcccatcggccaggccgacgaaatgcagaggtacgtggaggagaaccagaccaggaacaagcacatcaaccccaacgagtggtggaaggtgtacccctccagcgtgaccgagttcaagttcctgttcgtgtccggccacttcaagggcaactacaaggcccagctgaccaggctgaaccacatcaccaactgcaacggcgccgtgctgtccgtggaggagctcctgatcggcggcgagatgatcaaggccggcaccctgaccctggaggaggtgaggaggaagttcaacaacggcgagatcaacttcgcggccgactgataa

SEQ ID NO: 22 - DNA, 2832 bp, Artificialsequence
  GRex3T2-R TALEN
atgggcgatcctaaaaagaaacgtaaggtcatcgataaggagaccgccgctgccaagttcgagagacagcacatggacagcatcgatatcgccgatctacgcacgctcggctacagccagcagcaacaggagaagatcaaaccgaaggttcgttcgacagtggcgcagcaccacgaggcactggtcggccacgggtttacacacgcgcacatcgttgcgttaagccaacacccggcagcgttagggaccgtcgctgtcaagtatcaggacatgatcgcagcgttgccagaggcgacacacgaagcgatcgttggcgtcggcaaacagtggtccggcgcacgcgctctggaggccttgctcacggtggcgggagagttgagaggtccaccgttacagttggacacaggccaacttctcaagattgcaaaacgtggcggcgtgaccgcagtggaggcagtgcatgcatggcgcaatgcactgacgggtgccccgctcaacttgaccccccagcaggtggtggccatcgccagcaatggcggtggcaagcaggcgctggagacggtccagcggctgttgccggtgctgtgccaggcccacggcttgaccccggagcaggtggtggccatcgccagcaatattggtggcaagcaggcgctggagacggtgcaggcgctgttgccggtgctgtgccaggcccacggcttgaccccggagcaggtggtggccatcgccagcaatattggtggcaagcaggcgctggagacggtgcaggcgctgttgccggtgctgtgccaggcccacggcttgaccccccagcaggtggtggccatcgccagcaataatggtggcaagcaggcgctggagacggtccagcggctgttgccggtgctgtgccaggcccacggcttgaccccggagcaggtggtggccatcgccagcaatattggtggcaagcaggcgctggagacggtgcaggcgctgttgccggtgctgtgccaggcccacggcttgaccccggagcaggtggtggccatcgccagccacgatggcggcaagcaggcgctggagacggtccagcggctgttgccggtgctgtgccaggcccacggcttgaccccccagcaggtggtggccatcgccagcaatggcggtggcaagcaggcgctggagacggtccagcggctgttgccggtgctgtgccaggcccacggcttgaccccggagcaggtggtggccatcgccagccacgatggcggcaagcaggcgctggagacggtccagcggctgttgccggtgctgtgccaggcccacggcttgaccccggagcaggtggtggccatcgccagccacgatggcggcaagcaggcgctggagacggtccagcggctgttgccggtgctgtgccaggcccacggcttgaccccggagcaggtggtggccatcgccagcaatattggtggcaagcaggcgctggagacggtgcaggcgctgttgccggtgctgtgccaggcccacggcttgaccccccagcaggtggtggccatcgccagcaatggcggtggcaagcaggcgctggagacggtccagcggctgttgccggtgctgtgccaggcccacggcttgaccccggagcaggtggtggccatcgccagcaatattggtggcaagcaggcgctggagacggtgcaggcgctgttgccggtgctgtgccaggcccacggcttgaccccggagcaggtggtggccatcgccagcaatattggtggcaagcaggcgctggagacggtgcaggcgctgttgccggtgctgtgccaggcccacggcttgaccccccagcaggtggtggccatcgccagcaatggcggtggcaagcaggcgctggagacggtccagcggctgttgccggtgctgtgccaggcccacggcttgaccccccagcaggtggtggccatcgccagcaataatggtggcaagcaggcgctggagacggtccagcggctgttgccggtgctgtgccaggcccacggcttgacccctcagcaggtggtggccatcgccagcaatggcggcggcaggccggcgctggagagcattgttgcccagttatctcgccctgatccggcgttggccgcgttgaccaacgaccacctcgtcgccttggcctgcctcggcgggcgtcctgcgctggatgcagtgaaaaagggattgggggatcctatcagccgttcccagctggtgaagtccgagctggaggagaagaaatccgagttgaggcacaagctgaagtacgtgccccacgagtacatcgagctgatcgagatcgcccggaacagcacccaggaccgtatcctggagatgaaggtgatggagttcttcatgaaggtgtacggctacaggggcaagcacctgggcggctccaggaagcccgacggcgccatctacaccgtgggctcccccatcgactacggcgtgatcgtggacaccaaggcctactccggcggctacaacctgcccatcggccaggccgacgaaatgcagaggtacgtggaggagaaccagaccaggaacaagcacatcaaccccaacgagtggtggaaggtgtacccctccagcgtgaccgagttcaagttcctgttcgtgtccggccacttcaagggcaactacaaggcccagctgaccaggctgaaccacatcaccaactgcaacggcgccgtgctgtccgtggaggagctcctgatcggcggcgagatgatcaaggccggcaccctgaccctggaggaggtgaggaggaagttcaacaacggcgagatcaacttcgcggccgactgataa

SEQ ID NO: 23 - DNA, 2814 bp, Artificialsequence
  GRex3T4-L TALEN
atgggcgatcctaaaaagaaacgtaaggtcatcgattacccatacgatgttccagattacgctatcgatatcgccgatctacgcacgctcggctacagccagcagcaacaggagaagatcaaaccgaaggttcgttcgacagtggcgcagcaccacgaggcactggtcggccacgggtttacacacgcgcacatcgttgcgttaagccaacacccggcagcgttagggaccgtcgctgtcaagtatcaggacatgatcgcagcgttgccagaggcgacacacgaagcgatcgttggcgtcggcaaacagtggtccggcgcacgcgctctggaggccttgctcacggtggcgggagagttgagaggtccaccgttacagttggacacaggccaacttctcaagattgcaaaacgtggcggcgtgaccgcagtggaggcagtgcatgcatggcgcaatgcactgacgggtgccccgctcaacttgaccccccagcaggtggtggccatcgccagcaataatggtggcaagcaggcgctggagacggtccagcggctgttgccggtgctgtgccaggcccacggcttgaccccggagcaggtggtggccatcgccagccacgatggcggcaagcaggcgctggagacggtccagcggctgttgccggtgctgtgccaggcccacggcttgaccccccagcaggtggtggccatcgccagcaatggcggtggcaagcaggcgctggagacggtccagcggctgttgccggtgctgtgccaggcccacggcttgaccccggagcaggtggtggccatcgccagccacgatggcggcaagcaggcgctggagacggtccagcggctgttgccggtgctgtgccaggcccacggcttgaccccccagcaggtggtggccatcgccagcaatggcggtggcaagcaggcgctggagacggtccagcggctgttgccggtgctgtgccaggcccacggcttgaccccccagcaggtggtggccatcgccagcaataatggtggcaagcaggcgctggagacggtccagcggctgttgccggtgctgtgccaggcccacggcttgaccccggagcaggtggtggccatcgccagcaatattggtggcaagcaggcgctggagacggtgcaggcgctgttgccggtgctgtgccaggcccacggcttgaccccccagcaggtggtggccatcgccagcaatggcggtggcaagcaggcgctggagacggtccagcggctgttgccggtgctgtgccaggcccacggcttgaccccccagcaggtggtggccatcgccagcaataatggtggcaagcaggcgctggagacggtccagcggctgttgccggtgctgtgccaggcccacggcttgaccccggagcaggtggtggccatcgccagcaatattggtggcaagcaggcgctggagacggtgcaggcgctgttgccggtgctgtgccaggcccacggcttgaccccggagcaggtggtggccatcgccagcaatattggtggcaagcaggcgctggagacggtgcaggcgctgttgccggtgctgtgccaggcccacggcttgaccccccagcaggtggtggccatcgccagcaataatggtggcaagcaggcgctggagacggtccagcggctgttgccggtgctgtgccaggcccacggcttgaccccggagcaggtggtggccatcgccagccacgatggcggcaagcaggcgctggagacggtccagcggctgttgccggtgctgtgccaggcccacggcttgaccccccagcaggtggtggccatcgccagcaatggcggtggcaagcaggcgctggagacggtccagcggctgttgccggtgctgtgccaggcccacggcttgaccccccagcaggtggtggccatcgccagcaatggcggtggcaagcaggcgctggagacggtccagcggctgttgccggtgctgtgccaggcccacggcttgacccctcagcaggtggtggccatcgccagcaatggcggcggcaggccggcgctggagagcattgttgcccagttatctcgccctgatccggcgttggccgcgttgaccaacgaccacctcgtcgccttggcctgcctcggcgggcgtcctgcgctggatgcagtgaaaaagggattgggggatcctatcagccgttcccagctggtgaagtccgagctggaggagaagaaatccgagttgaggcacaagctgaagtacgtgccccacgagtacatcgagctgatcgagatcgcccggaacagcacccaggaccgtatcctggagatgaaggtgatggagttcttcatgaaggtgtacggctacaggggcaagcacctgggcggctccaggaagcccgacggcgccatctacaccgtgggctcccccatcgactacggcgtgatcgtggacaccaaggcctactccggcggctacaacctgcccatcggccaggccgacgaaatgcagaggtacgtggaggagaaccagaccaggaacaagcacatcaaccccaacgagtggtggaaggtgtacccctccagcgtgaccgagttcaagttcctgttcgtgtccggccacttcaagggcaactacaaggcccagctgaccaggctgaaccacatcaccaactgcaacggcgccgtgctgtccgtggaggagctcctgatcggcggcgagatgatcaaggccggcaccctgaccctggaggaggtgaggaggaagttcaacaacggcgagatcaacttcgcggccgactgataa

SEQ ID NO: 24 - DNA, 2832 bp, Artificialsequence
  GRex3T4-R TALEN
atgggcgatcctaaaaagaaacgtaaggtcatcgataaggagaccgccgctgccaagttcgagagacagcacatggacagcatcgatatcgccgatctacgcacgctcggctacagccagcagcaacaggagaagatcaaaccgaaggttcgttcgacagtggcgcagcaccacgaggcactggtcggccacgggtttacacacgcgcacatcgttgcgttaagccaacacccggcagcgttagggaccgtcgctgtcaagtatcaggacatgatcgcagcgttgccagaggcgacacacgaagcgatcgttggcgtcggcaaacagtggtccggcgcacgcgctctggaggccttgctcacggtggcgggagagttgagaggtccaccgttacagttggacacaggccaacttctcaagattgcaaaacgtggcggcgtgaccgcagtggaggcagtgcatgcatggcgcaatgcactgacgggtgccccgctcaacttgaccccccagcaggtggtggccatcgccagcaatggcggtggcaagcaggcgctggagacggtccagcggctgttgccggtgctgtgccaggcccacggcttgaccccggagcaggtggtggccatcgccagccacgatggcggcaagcaggcgctggagacggtccagcggctgttgccggtgctgtgccaggcccacggcttgaccccggagcaggtggtggccatcgccagccacgatggcggcaagcaggcgctggagacggtccagcggctgttgccggtgctgtgccaggcccacggcttgaccccggagcaggtggtggccatcgccagcaatattggtggcaagcaggcgctggagacggtgcaggcgctgttgccggtgctgtgccaggcccacggcttgaccccggagcaggtggtggccatcgccagccacgatggcggcaagcaggcgctggagacggtccagcggctgttgccggtgctgtgccaggcccacggcttgaccccggagcaggtggtggccatcgccagcaatattggtggcaagcaggcgctggagacggtgcaggcgctgttgccggtgctgtgccaggcccacggcttgaccccggagcaggtggtggccatcgccagcaatattggtggcaagcaggcgctggagacggtgcaggcgctgttgccggtgctgtgccaggcccacggcttgaccccccagcaggtggtggccatcgccagcaataatggtggcaagcaggcgctggagacggtccagcggctgttgccggtgctgtgccaggcccacggcttgaccccccagcaggtggtggccatcgccagcaatggcggtggcaagcaggcgctggagacggtccagcggctgttgccggtgctgtgccaggcccacggcttgaccccccagcaggtggtggccatcgccagcaatggcggtggcaagcaggcgctggagacggtccagcggctgttgccggtgctgtgccaggcccacggcttgaccccggagcaggtggtggccatcgccagcaatattggtggcaagcaggcgctggagacggtgcaggcgctgttgccggtgctgtgccaggcccacggcttgaccccggagcaggtggtggccatcgccagcaatattggtggcaagcaggcgctggagacggtgcaggcgctgttgccggtgctgtgccaggcccacggcttgaccccccagcaggtggtggccatcgccagcaataatggtggcaagcaggcgctggagacggtccagcggctgttgccggtgctgtgccaggcccacggcttgaccccggagcaggtggtggccatcgccagcaatattggtggcaagcaggcgctggagacggtgcaggcgctgttgccggtgctgtgccaggcccacggcttgaccccggagcaggtggtggccatcgccagccacgatggcggcaagcaggcgctggagacggtccagcggctgttgccggtgctgtgccaggcccacggcttgacccctcagcaggtggtggccatcgccagcaatggcggcggcaggccggcgctggagagcattgttgcccagttatctcgccctgatccggcgttggccgcgttgaccaacgaccacctcgtcgccttggcctgcctcggcgggcgtcctgcgctggatgcagtgaaaaagggattgggggatcctatcagccgttcccagctggtgaagtccgagctggaggagaagaaatccgagttgaggcacaagctgaagtacgtgccccacgagtacatcgagctgatcgagatcgcccggaacagcacccaggaccgtatcctggagatgaaggtgatggagttcttcatgaaggtgtacggctacaggggcaagcacctgggcggctccaggaagcccgacggcgccatctacaccgtgggctcccccatcgactacggcgtgatcgtggacaccaaggcctactccggcggctacaacctgcccatcggccaggccgacgaaatgcagaggtacgtggaggagaaccagaccaggaacaagcacatcaaccccaacgagtggtggaaggtgtacccctccagcgtgaccgagttcaagttcctgttcgtgtccggccacttcaagggcaactacaaggcccagctgaccaggctgaaccacatcaccaactgcaacggcgccgtgctgtccgtggaggagctcctgatcggcggcgagatgatcaaggccggcaccctgaccctggaggaggtgaggaggaagttcaacaacggcgagatcaacttcgcggccgactgataa

SEQ ID NO: 25 - DNA, 2814 bp, Artificialsequence
  GRex5T1-L TALEN
atgggcgatcctaaaaagaaacgtaaggtcatcgattacccatacgatgttccagattacgctatcgatatcgccgatctacgcacgctcggctacagccagcagcaacaggagaagatcaaaccgaaggttcgttcgacagtggcgcagcaccacgaggcactggtcggccacgggtttacacacgcgcacatcgttgcgttaagccaacacccggcagcgttagggaccgtcgctgtcaagtatcaggacatgatcgcagcgttgccagaggcgacacacgaagcgatcgttggcgtcggcaaacagtggtccggcgcacgcgctctggaggccttgctcacggtggcgggagagttgagaggtccaccgttacagttggacacaggccaacttctcaagattgcaaaacgtggcggcgtgaccgcagtggaggcagtgcatgcatggcgcaatgcactgacgggtgccccgctcaacttgaccccccagcaggtggtggccatcgccagcaataatggtggcaagcaggcgctggagacggtccagcggctgttgccggtgctgtgccaggcccacggcttgaccccccagcaggtggtggccatcgccagcaataatggtggcaagcaggcgctggagacggtccagcggctgttgccggtgctgtgccaggcccacggcttgaccccccagcaggtggtggccatcgccagcaatggcggtggcaagcaggcgctggagacggtccagcggctgttgccggtgctgtgccaggcccacggcttgaccccccagcaggtggtggccatcgccagcaataatggtggcaagcaggcgctggagacggtccagcggctgttgccggtgctgtgccaggcccacggcttgaccccccagcaggtggtggccatcgccagcaatggcggtggcaagcaggcgctggagacggtccagcggctgttgccggtgctgtgccaggcccacggcttgaccccggagcaggtggtggccatcgccagccacgatggcggcaagcaggcgctggagacggtccagcggctgttgccggtgctgtgccaggcccacggcttgaccccggagcaggtggtggccatcgccagcaatattggtggcaagcaggcgctggagacggtgcaggcgctgttgccggtgctgtgccaggcccacggcttgaccccggagcaggtggtggccatcgccagccacgatggcggcaagcaggcgctggagacggtccagcggctgttgccggtgctgtgccaggcccacggcttgaccccccagcaggtggtggccatcgccagcaatggcggtggcaagcaggcgctggagacggtccagcggctgttgccggtgctgtgccaggcccacggcttgaccccccagcaggtggtggccatcgccagcaataatggtggcaagcaggcgctggagacggtccagcggctgttgccggtgctgtgccaggcccacggcttgaccccccagcaggtggtggccatcgccagcaatggcggtggcaagcaggcgctggagacggtccagcggctgttgccggtgctgtgccaggcccacggcttgaccccccagcaggtggtggccatcgccagcaatggcggtggcaagcaggcgctggagacggtccagcggctgttgccggtgctgtgccaggcccacggcttgaccccccagcaggtggtggccatcgccagcaataatggtggcaagcaggcgctggagacggtccagcggctgttgccggtgctgtgccaggcccacggcttgaccccccagcaggtggtggccatcgccagcaataatggtggcaagcaggcgctggagacggtccagcggctgttgccggtgctgtgccaggcccacggcttgaccccggagcaggtggtggccatcgccagcaatattggtggcaagcaggcgctggagacggtgcaggcgctgttgccggtgctgtgccaggcccacggcttgacccctcagcaggtggtggccatcgccagcaatggcggcggcaggccggcgctggagagcattgttgcccagttatctcgccctgatccggcgttggccgcgttgaccaacgaccacctcgtcgccttggcctgcctcggcgggcgtcctgcgctggatgcagtgaaaaagggattgggggatcctatcagccgttcccagctggtgaagtccgagctggaggagaagaaatccgagttgaggcacaagctgaagtacgtgccccacgagtacatcgagctgatcgagatcgcccggaacagcacccaggaccgtatcctggagatgaaggtgatggagttcttcatgaaggtgtacggctacaggggcaagcacctgggcggctccaggaagcccgacggcgccatctacaccgtgggctcccccatcgactacggcgtgatcgtggacaccaaggcctactccggcggctacaacctgcccatcggccaggccgacgaaatgcagaggtacgtggaggagaaccagaccaggaacaagcacatcaaccccaacgagtggtggaaggtgtacccctccagcgtgaccgagttcaagttcctgttcgtgtccggccacttcaagggcaactacaaggcccagctgaccaggctgaaccacatcaccaactgcaacggcgccgtgctgtccgtggaggagctcctgatcggcggcgagatgatcaaggccggcaccctgaccctggaggaggtgaggaggaagttcaacaacggcgagatcaacttcgcggccgactgataa

SEQ ID NO: 26 - DNA, 2832 bp, Artificialsequence
  GRex5T1-R TALEN
atgggcgatcctaaaaagaaacgtaaggtcatcgataaggagaccgccgctgccaagttcgagagacagcacatggacagcatcgatatcgccgatctacgcacgctcggctacagccagcagcaacaggagaagatcaaaccgaaggttcgttcgacagtggcgcagcaccacgaggcactggtcggccacgggtttacacacgcgcacatcgttgcgttaagccaacacccggcagcgttagggaccgtcgctgtcaagtatcaggacatgatcgcagcgttgccagaggcgacacacgaagcgatcgttggcgtcggcaaacagtggtccggcgcacgcgctctggaggccttgctcacggtggcgggagagttgagaggtccaccgttacagttggacacaggccaacttctcaagattgcaaaacgtggcggcgtgaccgcagtggaggcagtgcatgcatggcgcaatgcactgacgggtgccccgctcaacttgaccccggagcaggtggtggccatcgccagcaatattggtggcaagcaggcgctggagacggtgcaggcgctgttgccggtgctgtgccaggcccacggcttgaccccccagcaggtggtggccatcgccagcaatggcggtggcaagcaggcgctggagacggtccagcggctgttgccggtgctgtgccaggcccacggcttgaccccggagcaggtggtggccatcgccagccacgatggcggcaagcaggcgctggagacggtccagcggctgttgccggtgctgtgccaggcccacggcttgaccccggagcaggtggtggccatcgccagccacgatggcggcaagcaggcgctggagacggtccagcggctgttgccggtgctgtgccaggcccacggcttgaccccccagcaggtggtggccatcgccagcaatggcggtggcaagcaggcgctggagacggtccagcggctgttgccggtgctgtgccaggcccacggcttgaccccccagcaggtggtggccatcgccagcaataatggtggcaagcaggcgctggagacggtccagcggctgttgccggtgctgtgccaggcccacggcttgaccccggagcaggtggtggccatcgccagccacgatggcggcaagcaggcgctggagacggtccagcggctgttgccggtgctgtgccaggcccacggcttgaccccggagcaggtggtggccatcgccagcaatattggtggcaagcaggcgctggagacggtgcaggcgctgttgccggtgctgtgccaggcccacggcttgaccccccagcaggtggtggccatcgccagcaatggcggtggcaagcaggcgctggagacggtccagcggctgttgccggtgctgtgccaggcccacggcttgaccccggagcaggtggtggccatcgccagcaatattggtggcaagcaggcgctggagacggtgcaggcgctgttgccggtgctgtgccaggcccacggcttgaccccccagcaggtggtggccatcgccagcaatggcggtggcaagcaggcgctggagacggtccagcggctgttgccggtgctgtgccaggcccacggcttgaccccggagcaggtggtggccatcgccagcaatattggtggcaagcaggcgctggagacggtgcaggcgctgttgccggtgctgtgccaggcccacggcttgaccccggagcaggtggtggccatcgccagcaatattggtggcaagcaggcgctggagacggtgcaggcgctgttgccggtgctgtgccaggcccacggcttgaccccggagcaggtggtggccatcgccagccacgatggcggcaagcaggcgctggagacggtccagcggctgttgccggtgctgtgccaggcccacggcttgaccccggagcaggtggtggccatcgccagcaatattggtggcaagcaggcgctggagacggtgcaggcgctgttgccggtgctgtgccaggcccacggcttgacccctcagcaggtggtggccatcgccagcaatggcggcggcaggccggcgctggagagcattgttgcccagttatctcgccctgatccggcgttggccgcgttgaccaacgaccacctcgtcgccttggcctgcctcggcgggcgtcctgcgctggatgcagtgaaaaagggattgggggatcctatcagccgttcccagctggtgaagtccgagctggaggagaagaaatccgagttgaggcacaagctgaagtacgtgccccacgagtacatcgagctgatcgagatcgcccggaacagcacccaggaccgtatcctggagatgaaggtgatggagttcttcatgaaggtgtacggctacaggggcaagcacctgggcggctccaggaagcccgacggcgccatctacaccgtgggctcccccatcgactacggcgtgatcgtggacaccaaggcctactccggcggctacaacctgcccatcggccaggccgacgaaatgcagaggtacgtggaggagaaccagaccaggaacaagcacatcaaccccaacgagtggtggaaggtgtacccctccagcgtgaccgagttcaagttcctgttcgtgtccggccacttcaagggcaactacaaggcccagctgaccaggctgaaccacatcaccaactgcaacggcgccgtgctgtccgtggaggagctcctgatcggcggcgagatgatcaaggccggcaccctgaccctggaggaggtgaggaggaagttcaacaacggcgagatcaacttcgcggccgactgataa

SEQ ID NO: 27 - DNA, 2814 bp, Artificialsequence
  GRex5T2-L TALEN
atgggcgatcctaaaaagaaacgtaaggtcatcgattacccatacgatgttccagattacgctatcgatatcgccgatctacgcacgctcggctacagccagcagcaacaggagaagatcaaaccgaaggttcgttcgacagtggcgcagcaccacgaggcactggtcggccacgggtttacacacgcgcacatcgttgcgttaagccaacacccggcagcgttagggaccgtcgctgtcaagtatcaggacatgatcgcagcgttgccagaggcgacacacgaagcgatcgttggcgtcggcaaacagtggtccggcgcacgcgctctggaggccttgctcacggtggcgggagagttgagaggtccaccgttacagttggacacaggccaacttctcaagattgcaaaacgtggcggcgtgaccgcagtggaggcagtgcatgcatggcgcaatgcactgacgggtgccccgctcaacttgaccccggagcaggtggtggccatcgccagcaatattggtggcaagcaggcgctggagacggtgcaggcgctgttgccggtgctgtgccaggcccacggcttgaccccccagcaggtggtggccatcgccagcaatggcggtggcaagcaggcgctggagacggtccagcggctgttgccggtgctgtgccaggcccacggcttgaccccccagcaggtggtggccatcgccagcaataatggtggcaagcaggcgctggagacggtccagcggctgttgccggtgctgtgccaggcccacggcttgaccccggagcaggtggtggccatcgccagcaatattggtggcaagcaggcgctggagacggtgcaggcgctgttgccggtgctgtgccaggcccacggcttgaccccccagcaggtggtggccatcgccagcaatggcggtggcaagcaggcgctggagacggtccagcggctgttgccggtgctgtgccaggcccacggcttgaccccggagcaggtggtggccatcgccagcaatattggtggcaagcaggcgctggagacggtgcaggcgctgttgccggtgctgtgccaggcccacggcttgaccccccagcaggtggtggccatcgccagcaataatggtggcaagcaggcgctggagacggtccagcggctgttgccggtgctgtgccaggcccacggcttgaccccggagcaggtggtggccatcgccagccacgatggcggcaagcaggcgctggagacggtccagcggctgttgccggtgctgtgccaggcccacggcttgaccccccagcaggtggtggccatcgccagcaatggcggtggcaagcaggcgctggagacggtccagcggctgttgccggtgctgtgccaggcccacggcttgaccccggagcaggtggtggccatcgccagccacgatggcggcaagcaggcgctggagacggtccagcggctgttgccggtgctgtgccaggcccacggcttgaccccccagcaggtggtggccatcgccagcaatggcggtggcaagcaggcgctggagacggtccagcggctgttgccggtgctgtgccaggcccacggcttgaccccccagcaggtggtggccatcgccagcaataatggtggcaagcaggcgctggagacggtccagcggctgttgccggtgctgtgccaggcccacggcttgaccccccagcaggtggtggccatcgccagcaatggcggtggcaagcaggcgctggagacggtccagcggctgttgccggtgctgtgccaggcccacggcttgaccccccagcaggtggtggccatcgccagcaatggcggtggcaagcaggcgctggagacggtccagcggctgttgccggtgctgtgccaggcccacggcttgaccccggagcaggtggtggccatcgccagccacgatggcggcaagcaggcgctggagacggtccagcggctgttgccggtgctgtgccaggcccacggcttgacccctcagcaggtggtggccatcgccagcaatggcggcggcaggccggcgctggagagcattgttgcccagttatctcgccctgatccggcgttggccgcgttgaccaacgaccacctcgtcgccttggcctgcctcggcgggcgtcctgcgctggatgcagtgaaaaagggattgggggatcctatcagccgttcccagctggtgaagtccgagctggaggagaagaaatccgagttgaggcacaagctgaagtacgtgccccacgagtacatcgagctgatcgagatcgcccggaacagcacccaggaccgtatcctggagatgaaggtgatggagttcttcatgaaggtgtacggctacaggggcaagcacctgggcggctccaggaagcccgacggcgccatctacaccgtgggctcccccatcgactacggcgtgatcgtggacaccaaggcctactccggcggctacaacctgcccatcggccaggccgacgaaatgcagaggtacgtggaggagaaccagaccaggaacaagcacatcaaccccaacgagtggtggaaggtgtacccctccagcgtgaccgagttcaagttcctgttcgtgtccggccacttcaagggcaactacaaggcccagctgaccaggctgaaccacatcaccaactgcaacggcgccgtgctgtccgtggaggagctcctgatcggcggcgagatgatcaaggccggcaccctgaccctggaggaggtgaggaggaagttcaacaacggcgagatcaacttcgcggccgactgataa

SEQ ID NO: 28 - DNA, 2832 bp, Artificialsequence
  GRex5T2-R TALEN
atgggcgatcctaaaaagaaacgtaaggtcatcgataaggagaccgccgctgccaagttcgagagacagcacatggacagcatcgatatcgccgatctacgcacgctcggctacagccagcagcaacaggagaagatcaaaccgaaggttcgttcgacagtggcgcagcaccacgaggcactggtcggccacgggtttacacacgcgcacatcgttgcgttaagccaacacccggcagcgttagggaccgtcgctgtcaagtatcaggacatgatcgcagcgttgccagaggcgacacacgaagcgatcgttggcgtcggcaaacagtggtccggcgcacgcgctctggaggccttgctcacggtggcgggagagttgagaggtccaccgttacagttggacacaggccaacttctcaagattgcaaaacgtggcggcgtgaccgcagtggaggcagtgcatgcatggcgcaatgcactgacgggtgccccgctcaacttgaccccccagcaggtggtggccatcgccagcaataatggtggcaagcaggcgctggagacggtccagcggctgttgccggtgctgtgccaggcccacggcttgaccccggagcaggtggtggccatcgccagcaatattggtggcaagcaggcgctggagacggtgcaggcgctgttgccggtgctgtgccaggcccacggcttgaccccccagcaggtggtggccatcgccagcaataatggtggcaagcaggcgctggagacggtccagcggctgttgccggtgctgtgccaggcccacggcttgaccccggagcaggtggtggccatcgccagccacgatggcggcaagcaggcgctggagacggtccagcggctgttgccggtgctgtgccaggcccacggcttgaccccccagcaggtggtggccatcgccagcaataatggtggcaagcaggcgctggagacggtccagcggctgttgccggtgctgtgccaggcccacggcttgaccccccagcaggtggtggccatcgccagcaatggcggtggcaagcaggcgctggagacggtccagcggctgttgccggtgctgtgccaggcccacggcttgaccccggagcaggtggtggccatcgccagcaatattggtggcaagcaggcgctggagacggtgcaggcgctgttgccggtgctgtgccaggcccacggcttgaccccccagcaggtggtggccatcgccagcaataatggtggcaagcaggcgctggagacggtccagcggctgttgccggtgctgtgccaggcccacggcttgaccccccagcaggtggtggccatcgccagcaatggcggtggcaagcaggcgctggagacggtccagcggctgttgccggtgctgtgccaggcccacggcttgaccccggagcaggtggtggccatcgccagccacgatggcggcaagcaggcgctggagacggtccagcggctgttgccggtgctgtgccaggcccacggcttgaccccggagcaggtggtggccatcgccagcaatattggtggcaagcaggcgctggagacggtgcaggcgctgttgccggtgctgtgccaggcccacggcttgaccccccagcaggtggtggccatcgccagcaatggcggtggcaagcaggcgctggagacggtccagcggctgttgccggtgctgtgccaggcccacggcttgaccccccagcaggtggtggccatcgccagcaataatggtggcaagcaggcgctggagacggtccagcggctgttgccggtgctgtgccaggcccacggcttgaccccggagcaggtggtggccatcgccagcaatattggtggcaagcaggcgctggagacggtgcaggcgctgttgccggtgctgtgccaggcccacggcttgaccccccagcaggtggtggccatcgccagcaatggcggtggcaagcaggcgctggagacggtccagcggctgttgccggtgctgtgccaggcccacggcttgacccctcagcaggtggtggccatcgccagcaatggcggcggcaggccggcgctggagagcattgttgcccagttatctcgccctgatccggcgttggccgcgttgaccaacgaccacctcgtcgccttggcctgcctcggcgggcgtcctgcgctggatgcagtgaaaaagggattgggggatcctatcagccgttcccagctggtgaagtccgagctggaggagaagaaatccgagttgaggcacaagctgaagtacgtgccccacgagtacatcgagctgatcgagatcgcccggaacagcacccaggaccgtatcctggagatgaaggtgatggagttcttcatgaaggtgtacggctacaggggcaagcacctgggcggctccaggaagcccgacggcgccatctacaccgtgggctcccccatcgactacggcgtgatcgtggacaccaaggcctactccggcggctacaacctgcccatcggccaggccgacgaaatgcagaggtacgtggaggagaaccagaccaggaacaagcacatcaaccccaacgagtggtggaaggtgtacccctccagcgtgaccgagttcaagttcctgttcgtgtccggccacttcaagggcaactacaaggcccagctgaccaggctgaaccacatcaccaactgcaacggcgccgtgctgtccgtggaggagctcctgatcggcggcgagatgatcaaggccggcaccctgaccctggaggaggtgaggaggaagttcaacaacggcgagatcaacttcgcggccgactgataa

SEQ ID NO: 29 - DNA, 2814 bp, Artificialsequence
  GRex5T3-L TALEN
atgggcgatcctaaaaagaaacgtaaggtcatcgattacccatacgatgttccagattacgctatcgatatcgccgatctacgcacgctcggctacagccagcagcaacaggagaagatcaaaccgaaggttcgttcgacagtggcgcagcaccacgaggcactggtcggccacgggtttacacacgcgcacatcgttgcgttaagccaacacccggcagcgttagggaccgtcgctgtcaagtatcaggacatgatcgcagcgttgccagaggcgacacacgaagcgatcgttggcgtcggcaaacagtggtccggcgcacgcgctctggaggccttgctcacggtggcgggagagttgagaggtccaccgttacagttggacacaggccaacttctcaagattgcaaaacgtggcggcgtgaccgcagtggaggcagtgcatgcatggcgcaatgcactgacgggtgccccgctcaacttgaccccccagcaggtggtggccatcgccagcaatggcggtggcaagcaggcgctggagacggtccagcggctgttgccggtgctgtgccaggcccacggcttgaccccggagcaggtggtggccatcgccagcaatattggtggcaagcaggcgctggagacggtgcaggcgctgttgccggtgctgtgccaggcccacggcttgaccccccagcaggtggtggccatcgccagcaatggcggtggcaagcaggcgctggagacggtccagcggctgttgccggtgctgtgccaggcccacggcttgaccccggagcaggtggtggccatcgccagcaatattggtggcaagcaggcgctggagacggtgcaggcgctgttgccggtgctgtgccaggcccacggcttgaccccccagcaggtggtggccatcgccagcaatggcggtggcaagcaggcgctggagacggtccagcggctgttgccggtgctgtgccaggcccacggcttgaccccccagcaggtggtggccatcgccagcaataatggtggcaagcaggcgctggagacggtccagcggctgttgccggtgctgtgccaggcccacggcttgaccccggagcaggtggtggccatcgccagccacgatggcggcaagcaggcgctggagacggtccagcggctgttgccggtgctgtgccaggcccacggcttgaccccggagcaggtggtggccatcgccagcaatattggtggcaagcaggcgctggagacggtgcaggcgctgttgccggtgctgtgccaggcccacggcttgaccccccagcaggtggtggccatcgccagcaataatggtggcaagcaggcgctggagacggtccagcggctgttgccggtgctgtgccaggcccacggcttgaccccccagcaggtggtggccatcgccagcaataatggtggcaagcaggcgctggagacggtccagcggctgttgccggtgctgtgccaggcccacggcttgaccccggagcaggtggtggccatcgccagcaatattggtggcaagcaggcgctggagacggtgcaggcgctgttgccggtgctgtgccaggcccacggcttgaccccccagcaggtggtggccatcgccagcaatggcggtggcaagcaggcgctggagacggtccagcggctgttgccggtgctgtgccaggcccacggcttgaccccggagcaggtggtggccatcgccagcaatattggtggcaagcaggcgctggagacggtgcaggcgctgttgccggtgctgtgccaggcccacggcttgaccccccagcaggtggtggccatcgccagcaatggcggtggcaagcaggcgctggagacggtccagcggctgttgccggtgctgtgccaggcccacggcttgaccccccagcaggtggtggccatcgccagcaataatggtggcaagcaggcgctggagacggtccagcggctgttgccggtgctgtgccaggcccacggcttgacccctcagcaggtggtggccatcgccagcaatggcggcggcaggccggcgctggagagcattgttgcccagttatctcgccctgatccggcgttggccgcgttgaccaacgaccacctcgtcgccttggcctgcctcggcgggcgtcctgcgctggatgcagtgaaaaagggattgggggatcctatcagccgttcccagctggtgaagtccgagctggaggagaagaaatccgagttgaggcacaagctgaagtacgtgccccacgagtacatcgagctgatcgagatcgcccggaacagcacccaggaccgtatcctggagatgaaggtgatggagttcttcatgaaggtgtacggctacaggggcaagcacctgggcggctccaggaagcccgacggcgccatctacaccgtgggctcccccatcgactacggcgtgatcgtggacaccaaggcctactccggcggctacaacctgcccatcggccaggccgacgaaatgcagaggtacgtggaggagaaccagaccaggaacaagcacatcaaccccaacgagtggtggaaggtgtacccctccagcgtgaccgagttcaagttcctgttcgtgtccggccacttcaagggcaactacaaggcccagctgaccaggctgaaccacatcaccaactgcaacggcgccgtgctgtccgtggaggagctcctgatcggcggcgagatgatcaaggccggcaccctgaccctggaggaggtgaggaggaagttcaacaacggcgagatcaacttcgcggccgactgataa

SEQ ID NO: 30 - DNA, 2832 bp, Artificialsequence
  GRex5T3-R TALEN
atgggcgatcctaaaaagaaacgtaaggtcatcgataaggagaccgccgctgccaagttcgagagacagcacatggacagcatcgatatcgccgatctacgcacgctcggctacagccagcagcaacaggagaagatcaaaccgaaggttcgttcgacagtggcgcagcaccacgaggcactggtcggccacgggtttacacacgcgcacatcgttgcgttaagccaacacccggcagcgttagggaccgtcgctgtcaagtatcaggacatgatcgcagcgttgccagaggcgacacacgaagcgatcgttggcgtcggcaaacagtggtccggcgcacgcgctctggaggccttgctcacggtggcgggagagttgagaggtccaccgttacagttggacacaggccaacttctcaagattgcaaaacgtggcggcgtgaccgcagtggaggcagtgcatgcatggcgcaatgcactgacgggtgccccgctcaacttgaccccccagcaggtggtggccatcgccagcaataatggtggcaagcaggcgctggagacggtccagcggctgttgccggtgctgtgccaggcccacggcttgaccccggagcaggtggtggccatcgccagcaatattggtggcaagcaggcgctggagacggtgcaggcgctgttgccggtgctgtgccaggcccacggcttgaccccccagcaggtggtggccatcgccagcaatggcggtggcaagcaggcgctggagacggtccagcggctgttgccggtgctgtgccaggcccacggcttgaccccggagcaggtggtggccatcgccagccacgatggcggcaagcaggcgctggagacggtccagcggctgttgccggtgctgtgccaggcccacggcttgaccccggagcaggtggtggccatcgccagccacgatggcggcaagcaggcgctggagacggtccagcggctgttgccggtgctgtgccaggcccacggcttgaccccccagcaggtggtggccatcgccagcaatggcggtggcaagcaggcgctggagacggtccagcggctgttgccggtgctgtgccaggcccacggcttgaccccggagcaggtggtggccatcgccagccacgatggcggcaagcaggcgctggagacggtccagcggctgttgccggtgctgtgccaggcccacggcttgaccccggagcaggtggtggccatcgccagccacgatggcggcaagcaggcgctggagacggtccagcggctgttgccggtgctgtgccaggcccacggcttgaccccggagcaggtggtggccatcgccagcaatattggtggcaagcaggcgctggagacggtgcaggcgctgttgccggtgctgtgccaggcccacggcttgaccccggagcaggtggtggccatcgccagcaatattggtggcaagcaggcgctggagacggtgcaggcgctgttgccggtgctgtgccaggcccacggcttgaccccccagcaggtggtggccatcgccagcaataatggtggcaagcaggcgctggagacggtccagcggctgttgccggtgctgtgccaggcccacggcttgaccccccagcaggtggtggccatcgccagcaatggcggtggcaagcaggcgctggagacggtccagcggctgttgccggtgctgtgccaggcccacggcttgaccccccagcaggtggtggccatcgccagcaatggcggtggcaagcaggcgctggagacggtccagcggctgttgccggtgctgtgccaggcccacggcttgaccccccagcaggtggtggccatcgccagcaataatggtggcaagcaggcgctggagacggtccagcggctgttgccggtgctgtgccaggcccacggcttgaccccggagcaggtggtggccatcgccagcaatattggtggcaagcaggcgctggagacggtgcaggcgctgttgccggtgctgtgccaggcccacggcttgacccctcagcaggtggtggccatcgccagcaatggcggcggcaggccggcgctggagagcattgttgcccagttatctcgccctgatccggcgttggccgcgttgaccaacgaccacctcgtcgccttggcctgcctcggcgggcgtcctgcgctggatgcagtgaaaaagggattgggggatcctatcagccgttcccagctggtgaagtccgagctggaggagaagaaatccgagttgaggcacaagctgaagtacgtgccccacgagtacatcgagctgatcgagatcgcccggaacagcacccaggaccgtatcctggagatgaaggtgatggagttcttcatgaaggtgtacggctacaggggcaagcacctgggcggctccaggaagcccgacggcgccatctacaccgtgggctcccccatcgactacggcgtgatcgtggacaccaaggcctactccggcggctacaacctgcccatcggccaggccgacgaaatgcagaggtacgtggaggagaaccagaccaggaacaagcacatcaaccccaacgagtggtggaaggtgtacccctccagcgtgaccgagttcaagttcctgttcgtgtccggccacttcaagggcaactacaaggcccagctgaccaggctgaaccacatcaccaactgcaacggcgccgtgctgtccgtggaggagctcctgatcggcggcgagatgatcaaggccggcaccctgaccctggaggaggtgaggaggaagttcaacaacggcgagatcaacttcgcggccgactgataa

SEQ ID NO: 31 - DNA, 60 bp, Artificialsequence
  Forward primer GR exon 2
  misc_feature (31); (32); (33); (34); (35); (36); (37); (38); (39); (40): n is a or c or t or g
ccatctcatccctgcgtgtctccgactcagnnnnnnnnnnggttcatttaacaagctgcc

SEQ ID NO: 32 - DNA, 60 bp, Artificialsequence
  Forward primer GR exon 3
  misc_feature (31); (32); (33); (34); (35); (36); (37); (38); (39); (40): n is a or c or t or g
ccatctcatccctgcgtgtctccgactcagnnnnnnnnnngcattctgactatgaagtga

SEQ ID NO: 33 - DNA, 69 bp, Artificialsequence
  Forward primer GR exon 5
  misc_feature (31); (32); (33); (34); (35); (36); (37); (38); (39); (40): n is a or c or t or g
ccatctcatccctgcgtgtctccgactcagnnnnnnnnnntcagcaggccactacaggagtctcacaag

SEQ ID NO: 34 - DNA, 50 bp, Artificialsequence
  Reverse primer GR exon 2
cctatcccctgtgtgccttggcagtctcagagccagtgagggtgaagacg

SEQ ID NO: 35 - DNA, 50 bp, Artificialsequence
  Reverse primer GR exon 3
cctatcccctgtgtgccttggcagtctcaggggctttgcatataatggaa

SEQ ID NO: 36 - DNA, 59 bp, Artificialsequence
  Reverse primer GR exon 5
cctatcccctgtgtgccttggcagtctcagctgactctccccttcatagtccccagaac

SEQ ID NO: 37 - DNA, 49 bp, Artificialsequence
  TRAC_T01
ttgtcccacagatatccagaaccctgaccctgccgtgtaccagctgaga

SEQ ID NO: 38 - DNA, 49 bp, Artificialsequence
  TRBC_T01
tgtgtttgagccatcagaagcagagatctcccacacccaaaaggccaca

SEQ ID NO: 39 - DNA, 50 bp, Artificialsequence
  TRBC_T02
ttcccacccgaggtcgctgtgtttgagccatcagaagcagagatctccca

SEQ ID NO: 40 - DNA, 49 bp, Artificialsequence
  CD52_T02
ttcctcctactcaccatcagcctcctggttatggtacaggtaagagcaa

SEQ ID NO: 41 - protein, 530 aa, Artificialsequence
  Repeat TRAC_T01-L
LTPQQVVAIASNGGGKQALETVQRLLPVLCQAHGLTPQQVVAIASNNGGKQALETVQRLLPVLCQAHGLTPQQVVAIASNGGGKQALETVQRLLPVLCQAHGLTPEQVVAIASHDGGKQALETVQRLLPVLCQAHGLTPEQVVAIASHDGGKQALETVQRLLPVLCQAHGLTPEQVVAIASHDGGKQALETVQRLLPVLCQAHGLTPEQVVAIASNIGGKQALETVQALLPVLCQAHGLTPEQVVAIASHDGGKQALETVQRLLPVLCQAHGLTPEQVVAIASNIGGKQALETVQALLPVLCQAHGLTPQQVVAIASNNGGKQALETVQRLLPVLCQAHGLTPEQVVAIASNIGGKQALETVQALLPVLCQAHGLTPQQVVAIASNGGGKQALETVQRLLPVLCQAHGLTPEQVVAIASNIGGKQALETVQALLPVLCQAHGLTPQQVVAIASNGGGKQALETVQRLLPVLCQAHGLTPEQVVAIASHDGGKQALETVQRLLPVLCQAHGLTPQQVVAIASNGGGRPALE

SEQ ID NO: 42 - protein, 530 aa, Artificialsequence
  Repeat TRAC_T01-R
LTPEQVVAIASHDGGKQALETVQRLLPVLCQAHGLTPQQVVAIASNGGGKQALETVQRLLPVLCQAHGLTPEQVVAIASHDGGKQALETVQRLLPVLCQAHGLTPEQVVAIASNIGGKQALETVQALLPVLCQAHGLTPQQVVAIASNNGGKQALETVQRLLPVLCQAHGLTPEQVVAIASHDGGKQALETVQRLLPVLCQAHGLTPQQVVAIASNGGGKQALETVQRLLPVLCQAHGLTPQQVVAIASNNGGKQALETVQRLLPVLCQAHGLTPQQVVAIASNNGGKQALETVQRLLPVLCQAHGLTPQQVVAIASNGGGKQALETVQRLLPVLCQAHGLTPEQVVAIASNIGGKQALETVQALLPVLCQAHGLTPEQVVAIASHDGGKQALETVQRLLPVLCQAHGLTPEQVVAIASNIGGKQALETVQALLPVLCQAHGLTPEQVVAIASHDGGKQALETVQRLLPVLCQAHGLTPQQVVAIASNNGGKQALETVQRLLPVLCQAHGLTPQQVVAIASNGGGRPALE

SEQ ID NO: 43 - protein, 530 aa, Artificialsequence
  Repeat TRBC_T01-L
LTPQQVVAIASNNGGKQALETVQRLLPVLCQAHGLTPQQVVAIASNGGGKQALETVQRLLPVLCQAHGLTPQQVVAIASNNGGKQALETVQRLLPVLCQAHGLTPQQVVAIASNGGGKQALETVQRLLPVLCQAHGLTPQQVVAIASNGGGKQALETVQRLLPVLCQAHGLTPQQVVAIASNGGGKQALETVQRLLPVLCQAHGLTPQQVVAIASNNGGKQALETVQRLLPVLCQAHGLTPEQVVAIASNIGGKQALETVQALLPVLCQAHGLTPQQVVAIASNNGGKQALETVQRLLPVLCQAHGLTPEQVVAIASHDGGKQALETVQRLLPVLCQAHGLTPEQVVAIASHDGGKQALETVQRLLPVLCQAHGLTPEQVVAIASNIGGKQALETVQALLPVLCQAHGLTPQQVVAIASNGGGKQALETVQRLLPVLCQAHGLTPEQVVAIASHDGGKQALETVQRLLPVLCQAHGLTPEQVVAIASNIGGKQALETVQALLPVLCQAHGLTPQQVVAIASNGGGRPALE

SEQ ID NO: 44 - protein, 530 aa, Artificialsequence
  Repeat TRBC_T01-R
LTPQQVVAIASNNGGKQALETVQRLLPVLCQAHGLTPQQVVAIASNGGGKQALETVQRLLPVLCQAHGLTPQQVVAIASNNGGKQALETVQRLLPVLCQAHGLTPQQVVAIASNNGGKQALETVQRLLPVLCQAHGLTPEQVVAIASHDGGKQALETVQRLLPVLCQAHGLTPEQVVAIASHDGGKQALETVQRLLPVLCQAHGLTPQQVVAIASNGGGKQALETVQRLLPVLCQAHGLTPQQVVAIASNGGGKQALETVQRLLPVLCQAHGLTPQQVVAIASNGGGKQALETVQRLLPVLCQAHGLTPQQVVAIASNGGGKQALETVQRLLPVLCQAHGLTPQQVVAIASNNGGKQALETVQRLLPVLCQAHGLTPQQVVAIASNNGGKQALETVQRLLPVLCQAHGLTPQQVVAIASNNGGKQALETVQRLLPVLCQAHGLTPQQVVAIASNGGGKQALETVQRLLPVLCQAHGLTPQQVVAIASNNGGKQALETVQRLLPVLCQAHGLTPQQVVAIASNGGGRPALE

SEQ ID NO: 45 - protein, 530 aa, Artificialsequence
  Repeat TRBC_T02-L
LTPEQVVAIASHDGGKQALETVQRLLPVLCQAHGLTPEQVVAIASHDGGKQALETVQRLLPVLCQAHGLTPEQVVAIASHDGGKQALETVQRLLPVLCQAHGLTPEQVVAIASNIGGKQALETVQALLPVLCQAHGLTPEQVVAIASHDGGKQALETVQRLLPVLCQAHGLTPEQVVAIASHDGGKQALETVQRLLPVLCQAHGLTPEQVVAIASHDGGKQALETVQRLLPVLCQAHGLTPQQVVAIASNNGGKQALETVQRLLPVLCQAHGLTPEQVVAIASNIGGKQALETVQALLPVLCQAHGLTPQQVVAIASNNGGKQALETVQRLLPVLCQAHGLTPQQVVAIASNNGGKQALETVQRLLPVLCQAHGLTPQQVVAIASNGGGKQALETVQRLLPVLCQAHGLTPEQVVAIASHDGGKQALETVQRLLPVLCQAHGLTPQQVVAIASNNGGKQALETVQRLLPVLCQAHGLTPEQVVAIASHDGGKQALETVQRLLPVLCQAHGLTPQQVVAIASNGGGRPALE

SEQ ID NO: 46 - protein, 530 aa, Artificialsequence
  Repeat TRBC_T02-R
LTPQQVVAIASNNGGKQALETVQRLLPVLCQAHGLTPQQVVAIASNNGGKQALETVQRLLPVLCQAHGLTPQQVVAIASNNGGKQALETVQRLLPVLCQAHGLTPEQVVAIASNIGGKQALETVQALLPVLCQAHGLTPQQVVAIASNNGGKQALETVQRLLPVLCQAHGLTPEQVVAIASNIGGKQALETVQALLPVLCQAHGLTPQQVVAIASNGGGKQALETVQRLLPVLCQAHGLTPEQVVAIASHDGGKQALETVQRLLPVLCQAHGLTPQQVVAIASNGGGKQALETVQRLLPVLCQAHGLTPEQVVAIASHDGGKQALETVQRLLPVLCQAHGLTPQQVVAIASNGGGKQALETVQRLLPVLCQAHGLTPQQVVAIASNNGGKQALETVQRLLPVLCQAHGLTPEQVVAIASHDGGKQALETVQRLLPVLCQAHGLTPQQVVAIASNGGGKQALETVQRLLPVLCQAHGLTPQQVVAIASNGGGKQALETVQRLLPVLCQAHGLTPQQVVAIASNGGGRPALE

SEQ ID NO: 47 - protein, 530 aa, Artificialsequence
  Repeat CD52_T02-L
LTPQQVVAIASNGGGKQALETVQRLLPVLCQAHGLTPEQVVAIASHDGGKQALETVQRLLPVLCQAHGLTPEQVVAIASHDGGKQALETVQRLLPVLCQAHGLTPQQVVAIASNGGGKQALETVQRLLPVLCQAHGLTPEQVVAIASHDGGKQALETVQRLLPVLCQAHGLTPEQVVAIASHDGGKQALETVQRLLPVLCQAHGLTPQQVVAIASNGGGKQALETVQRLLPVLCQAHGLTPEQVVAIASNIGGKQALETVQALLPVLCQAHGLTPEQVVAIASHDGGKQALETVQRLLPVLCQAHGLTPQQVVAIASNGGGKQALETVQRLLPVLCQAHGLTPEQVVAIASHDGGKQALETVQRLLPVLCQAHGLTPEQVVAIASNIGGKQALETVQALLPVLCQAHGLTPEQVVAIASHDGGKQALETVQRLLPVLCQAHGLTPEQVVAIASHDGGKQALETVQRLLPVLCQAHGLTPEQVVAIASNIGGKQALETVQALLPVLCQAHGLTPQQVVAIASNGGGRPALE

SEQ ID NO: 48 - protein, 530 aa, Artificialsequence
  Repeat CD52_T02-R
LTPQQVVAIASNGGGKQALETVQRLLPVLCQAHGLTPQQVVAIASNNGGKQALETVQRLLPVLCQAHGLTPEQVVAIASHDGGKQALETVQRLLPVLCQAHGLTPQQVVAIASNGGGKQALETVQRLLPVLCQAHGLTPEQVVAIASHDGGKQALETVQRLLPVLCQAHGLTPQQVVAIASNGGGKQALETVQRLLPVLCQAHGLTPQQVVAIASNGGGKQALETVQRLLPVLCQAHGLTPEQVVAIASNIGGKQALETVQALLPVLCQAHGLTPEQVVAIASHDGGKQALETVQRLLPVLCQAHGLTPEQVVAIASHDGGKQALETVQRLLPVLCQAHGLTPQQVVAIASNGGGKQALETVQRLLPVLCQAHGLTPQQVVAIASNNGGKQALETVQRLLPVLCQAHGLTPQQVVAIASNGGGKQALETVQRLLPVLCQAHGLTPEQVVAIASNIGGKQALETVQALLPVLCQAHGLTPEQVVAIASHDGGKQALETVQRLLPVLCQAHGLTPQQVVAIASNGGGRPALE

SEQ ID NO: 49 - DNA, 2814 bp, Artificialsequence
  TRAC_T01-L TALEN
atgggcgatcctaaaaagaaacgtaaggtcatcgattacccatacgatgttccagattacgctatcgatatcgccgatctacgcacgctcggctacagccagcagcaacaggagaagatcaaaccgaaggttcgttcgacagtggcgcagcaccacgaggcactggtcggccacgggtttacacacgcgcacatcgttgcgttaagccaacacccggcagcgttagggaccgtcgctgtcaagtatcaggacatgatcgcagcgttgccagaggcgacacacgaagcgatcgttggcgtcggcaaacagtggtccggcgcacgcgctctggaggccttgctcacggtggcgggagagttgagaggtccaccgttacagttggacacaggccaacttctcaagattgcaaaacgtggcggcgtgaccgcagtggaggcagtgcatgcatggcgcaatgcactgacgggtgccccgctcaacttgaccccccagcaggtggtggccatcgccagcaatggcggtggcaagcaggcgctggagacggtccagcggctgttgccggtgctgtgccaggcccacggcttgaccccccagcaggtggtggccatcgccagcaataatggtggcaagcaggcgctggagacggtccagcggctgttgccggtgctgtgccaggcccacggcttgaccccccagcaggtggtggccatcgccagcaatggcggtggcaagcaggcgctggagacggtccagcggctgttgccggtgctgtgccaggcccacggcttgaccccggagcaggtggtggccatcgccagccacgatggcggcaagcaggcgctggagacggtccagcggctgttgccggtgctgtgccaggcccacggcttgaccccggagcaggtggtggccatcgccagccacgatggcggcaagcaggcgctggagacggtccagcggctgttgccggtgctgtgccaggcccacggcttgaccccggagcaggtggtggccatcgccagccacgatggcggcaagcaggcgctggagacggtccagcggctgttgccggtgctgtgccaggcccacggcttgaccccggagcaggtggtggccatcgccagcaatattggtggcaagcaggcgctggagacggtgcaggcgctgttgccggtgctgtgccaggcccacggcttgaccccggagcaggtggtggccatcgccagccacgatggcggcaagcaggcgctggagacggtccagcggctgttgccggtgctgtgccaggcccacggcttgaccccggagcaggtggtggccatcgccagcaatattggtggcaagcaggcgctggagacggtgcaggcgctgttgccggtgctgtgccaggcccacggcttgaccccccagcaggtggtggccatcgccagcaataatggtggcaagcaggcgctggagacggtccagcggctgttgccggtgctgtgccaggcccacggcttgaccccggagcaggtggtggccatcgccagcaatattggtggcaagcaggcgctggagacggtgcaggcgctgttgccggtgctgtgccaggcccacggcttgaccccccagcaggtggtggccatcgccagcaatggcggtggcaagcaggcgctggagacggtccagcggctgttgccggtgctgtgccaggcccacggcttgaccccggagcaggtggtggccatcgccagcaatattggtggcaagcaggcgctggagacggtgcaggcgctgttgccggtgctgtgccaggcccacggcttgaccccccagcaggtggtggccatcgccagcaatggcggtggcaagcaggcgctggagacggtccagcggctgttgccggtgctgtgccaggcccacggcttgaccccggagcaggtggtggccatcgccagccacgatggcggcaagcaggcgctggagacggtccagcggctgttgccggtgctgtgccaggcccacggcttgacccctcagcaggtggtggccatcgccagcaatggcggcggcaggccggcgctggagagcattgttgcccagttatctcgccctgatccggcgttggccgcgttgaccaacgaccacctcgtcgccttggcctgcctcggcgggcgtcctgcgctggatgcagtgaaaaagggattgggggatcctatcagccgttcccagctggtgaagtccgagctggaggagaagaaatccgagttgaggcacaagctgaagtacgtgccccacgagtacatcgagctgatcgagatcgcccggaacagcacccaggaccgtatcctggagatgaaggtgatggagttcttcatgaaggtgtacggctacaggggcaagcacctgggcggctccaggaagcccgacggcgccatctacaccgtgggctcccccatcgactacggcgtgatcgtggacaccaaggcctactccggcggctacaacctgcccatcggccaggccgacgaaatgcagaggtacgtggaggagaaccagaccaggaacaagcacatcaaccccaacgagtggtggaaggtgtacccctccagcgtgaccgagttcaagttcctgttcgtgtccggccacttcaagggcaactacaaggcccagctgaccaggctgaaccacatcaccaactgcaacggcgccgtgctgtccgtggaggagctcctgatcggcggcgagatgatcaaggccggcaccctgaccctggaggaggtgaggaggaagttcaacaacggcgagatcaacttcgcggccgactgataa

SEQ ID NO: 50 - DNA, 2832 bp, Artificialsequence
  TRAC_T01-R TALEN
atgggcgatcctaaaaagaaacgtaaggtcatcgataaggagaccgccgctgccaagttcgagagacagcacatggacagcatcgatatcgccgatctacgcacgctcggctacagccagcagcaacaggagaagatcaaaccgaaggttcgttcgacagtggcgcagcaccacgaggcactggtcggccacgggtttacacacgcgcacatcgttgcgttaagccaacacccggcagcgttagggaccgtcgctgtcaagtatcaggacatgatcgcagcgttgccagaggcgacacacgaagcgatcgttggcgtcggcaaacagtggtccggcgcacgcgctctggaggccttgctcacggtggcgggagagttgagaggtccaccgttacagttggacacaggccaacttctcaagattgcaaaacgtggcggcgtgaccgcagtggaggcagtgcatgcatggcgcaatgcactgacgggtgccccgctcaacttgaccccggagcaggtggtggccatcgccagccacgatggcggcaagcaggcgctggagacggtccagcggctgttgccggtgctgtgccaggcccacggcttgaccccccagcaggtggtggccatcgccagcaatggcggtggcaagcaggcgctggagacggtccagcggctgttgccggtgctgtgccaggcccacggcttgaccccggagcaggtggtggccatcgccagccacgatggcggcaagcaggcgctggagacggtccagcggctgttgccggtgctgtgccaggcccacggcttgaccccggagcaggtggtggccatcgccagcaatattggtggcaagcaggcgctggagacggtgcaggcgctgttgccggtgctgtgccaggcccacggcttgaccccccagcaggtggtggccatcgccagcaataatggtggcaagcaggcgctggagacggtccagcggctgttgccggtgctgtgccaggcccacggcttgaccccggagcaggtggtggccatcgccagccacgatggcggcaagcaggcgctggagacggtccagcggctgttgccggtgctgtgccaggcccacggcttgaccccccagcaggtggtggccatcgccagcaatggcggtggcaagcaggcgctggagacggtccagcggctgttgccggtgctgtgccaggcccacggcttgaccccccagcaggtggtggccatcgccagcaataatggtggcaagcaggcgctggagacggtccagcggctgttgccggtgctgtgccaggcccacggcttgaccccccagcaggtggtggccatcgccagcaataatggtggcaagcaggcgctggagacggtccagcggctgttgccggtgctgtgccaggcccacggcttgaccccccagcaggtggtggccatcgccagcaatggcggtggcaagcaggcgctggagacggtccagcggctgttgccggtgctgtgccaggcccacggcttgaccccggagcaggtggtggccatcgccagcaatattggtggcaagcaggcgctggagacggtgcaggcgctgttgccggtgctgtgccaggcccacggcttgaccccggagcaggtggtggccatcgccagccacgatggcggcaagcaggcgctggagacggtccagcggctgttgccggtgctgtgccaggcccacggcttgaccccggagcaggtggtggccatcgccagcaatattggtggcaagcaggcgctggagacggtgcaggcgctgttgccggtgctgtgccaggcccacggcttgaccccggagcaggtggtggccatcgccagccacgatggcggcaagcaggcgctggagacggtccagcggctgttgccggtgctgtgccaggcccacggcttgaccccccagcaggtggtggccatcgccagcaataatggtggcaagcaggcgctggagacggtccagcggctgttgccggtgctgtgccaggcccacggcttgacccctcagcaggtggtggccatcgccagcaatggcggcggcaggccggcgctggagagcattgttgcccagttatctcgccctgatccggcgttggccgcgttgaccaacgaccacctcgtcgccttggcctgcctcggcgggcgtcctgcgctggatgcagtgaaaaagggattgggggatcctatcagccgttcccagctggtgaagtccgagctggaggagaagaaatccgagttgaggcacaagctgaagtacgtgccccacgagtacatcgagctgatcgagatcgcccggaacagcacccaggaccgtatcctggagatgaaggtgatggagttcttcatgaaggtgtacggctacaggggcaagcacctgggcggctccaggaagcccgacggcgccatctacaccgtgggctcccccatcgactacggcgtgatcgtggacaccaaggcctactccggcggctacaacctgcccatcggccaggccgacgaaatgcagaggtacgtggaggagaaccagaccaggaacaagcacatcaaccccaacgagtggtggaaggtgtacccctccagcgtgaccgagttcaagttcctgttcgtgtccggccacttcaagggcaactacaaggcccagctgaccaggctgaaccacatcaccaactgcaacggcgccgtgctgtccgtggaggagctcctgatcggcggcgagatgatcaaggccggcaccctgaccctggaggaggtgaggaggaagttcaacaacggcgagatcaacttcgcggccgactgataa

SEQ ID NO: 51 - DNA, 2814 bp, Artificialsequence
  TRBC_T01-L TALEN
atgggcgatcctaaaaagaaacgtaaggtcatcgattacccatacgatgttccagattacgctatcgatatcgccgatctacgcacgctcggctacagccagcagcaacaggagaagatcaaaccgaaggttcgttcgacagtggcgcagcaccacgaggcactggtcggccacgggtttacacacgcgcacatcgttgcgttaagccaacacccggcagcgttagggaccgtcgctgtcaagtatcaggacatgatcgcagcgttgccagaggcgacacacgaagcgatcgttggcgtcggcaaacagtggtccggcgcacgcgctctggaggccttgctcacggtggcgggagagttgagaggtccaccgttacagttggacacaggccaacttctcaagattgcaaaacgtggcggcgtgaccgcagtggaggcagtgcatgcatggcgcaatgcactgacgggtgccccgctcaacttgaccccccagcaggtggtggccatcgccagcaataatggtggcaagcaggcgctggagacggtccagcggctgttgccggtgctgtgccaggcccacggcttgaccccccagcaggtggtggccatcgccagcaatggcggtggcaagcaggcgctggagacggtccagcggctgttgccggtgctgtgccaggcccacggcttgaccccccagcaggtggtggccatcgccagcaataatggtggcaagcaggcgctggagacggtccagcggctgttgccggtgctgtgccaggcccacggcttgaccccccagcaggtggtggccatcgccagcaatggcggtggcaagcaggcgctggagacggtccagcggctgttgccggtgctgtgccaggcccacggcttgaccccccagcaggtggtggccatcgccagcaatggcggtggcaagcaggcgctggagacggtccagcggctgttgccggtgctgtgccaggcccacggcttgaccccccagcaggtggtggccatcgccagcaatggcggtggcaagcaggcgctggagacggtccagcggctgttgccggtgctgtgccaggcccacggcttgaccccccagcaggtggtggccatcgccagcaataatggtggcaagcaggcgctggagacggtccagcggctgttgccggtgctgtgccaggcccacggcttgaccccggagcaggtggtggccatcgccagcaatattggtggcaagcaggcgctggagacggtgcaggcgctgttgccggtgctgtgccaggcccacggcttgaccccccagcaggtggtggccatcgccagcaataatggtggcaagcaggcgctggagacggtccagcggctgttgccggtgctgtgccaggcccacggcttgaccccggagcaggtggtggccatcgccagccacgatggcggcaagcaggcgctggagacggtccagcggctgttgccggtgctgtgccaggcccacggcttgaccccggagcaggtggtggccatcgccagccacgatggcggcaagcaggcgctggagacggtccagcggctgttgccggtgctgtgccaggcccacggcttgaccccggagcaggtggtggccatcgccagcaatattggtggcaagcaggcgctggagacggtgcaggcgctgttgccggtgctgtgccaggcccacggcttgaccccccagcaggtggtggccatcgccagcaatggcggtggcaagcaggcgctggagacggtccagcggctgttgccggtgctgtgccaggcccacggcttgaccccggagcaggtggtggccatcgccagccacgatggcggcaagcaggcgctggagacggtccagcggctgttgccggtgctgtgccaggcccacggcttgaccccggagcaggtggtggccatcgccagcaatattggtggcaagcaggcgctggagacggtgcaggcgctgttgccggtgctgtgccaggcccacggcttgacccctcagcaggtggtggccatcgccagcaatggcggcggcaggccggcgctggagagcattgttgcccagttatctcgccctgatccggcgttggccgcgttgaccaacgaccacctcgtcgccttggcctgcctcggcgggcgtcctgcgctggatgcagtgaaaaagggattgggggatcctatcagccgttcccagctggtgaagtccgagctggaggagaagaaatccgagttgaggcacaagctgaagtacgtgccccacgagtacatcgagctgatcgagatcgcccggaacagcacccaggaccgtatcctggagatgaaggtgatggagttcttcatgaaggtgtacggctacaggggcaagcacctgggcggctccaggaagcccgacggcgccatctacaccgtgggctcccccatcgactacggcgtgatcgtggacaccaaggcctactccggcggctacaacctgcccatcggccaggccgacgaaatgcagaggtacgtggaggagaaccagaccaggaacaagcacatcaaccccaacgagtggtggaaggtgtacccctccagcgtgaccgagttcaagttcctgttcgtgtccggccacttcaagggcaactacaaggcccagctgaccaggctgaaccacatcaccaactgcaacggcgccgtgctgtccgtggaggagctcctgatcggcggcgagatgatcaaggccggcaccctgaccctggaggaggtgaggaggaagttcaacaacggcgagatcaacttcgcggccgactgataa

SEQ ID NO: 52 - DNA, 2832 bp, Artificialsequence
  TRBC_T01-R TALEN
atgggcgatcctaaaaagaaacgtaaggtcatcgataaggagaccgccgctgccaagttcgagagacagcacatggacagcatcgatatcgccgatctacgcacgctcggctacagccagcagcaacaggagaagatcaaaccgaaggttcgttcgacagtggcgcagcaccacgaggcactggtcggccacgggtttacacacgcgcacatcgttgcgttaagccaacacccggcagcgttagggaccgtcgctgtcaagtatcaggacatgatcgcagcgttgccagaggcgacacacgaagcgatcgttggcgtcggcaaacagtggtccggcgcacgcgctctggaggccttgctcacggtggcgggagagttgagaggtccaccgttacagttggacacaggccaacttctcaagattgcaaaacgtggcggcgtgaccgcagtggaggcagtgcatgcatggcgcaatgcactgacgggtgccccgctcaacttgaccccccagcaggtggtggccatcgccagcaataatggtggcaagcaggcgctggagacggtccagcggctgttgccggtgctgtgccaggcccacggcttgaccccccagcaggtggtggccatcgccagcaatggcggtggcaagcaggcgctggagacggtccagcggctgttgccggtgctgtgccaggcccacggcttgaccccccagcaggtggtggccatcgccagcaataatggtggcaagcaggcgctggagacggtccagcggctgttgccggtgctgtgccaggcccacggcttgaccccccagcaggtggtggccatcgccagcaataatggtggcaagcaggcgctggagacggtccagcggctgttgccggtgctgtgccaggcccacggcttgaccccggagcaggtggtggccatcgccagccacgatggcggcaagcaggcgctggagacggtccagcggctgttgccggtgctgtgccaggcccacggcttgaccccggagcaggtggtggccatcgccagccacgatggcggcaagcaggcgctggagacggtccagcggctgttgccggtgctgtgccaggcccacggcttgaccccccagcaggtggtggccatcgccagcaatggcggtggcaagcaggcgctggagacggtccagcggctgttgccggtgctgtgccaggcccacggcttgaccccccagcaggtggtggccatcgccagcaatggcggtggcaagcaggcgctggagacggtccagcggctgttgccggtgctgtgccaggcccacggcttgaccccccagcaggtggtggccatcgccagcaatggcggtggcaagcaggcgctggagacggtccagcggctgttgccggtgctgtgccaggcccacggcttgaccccccagcaggtggtggccatcgccagcaatggcggtggcaagcaggcgctggagacggtccagcggctgttgccggtgctgtgccaggcccacggcttgaccccccagcaggtggtggccatcgccagcaataatggtggcaagcaggcgctggagacggtccagcggctgttgccggtgctgtgccaggcccacggcttgaccccccagcaggtggtggccatcgccagcaataatggtggcaagcaggcgctggagacggtccagcggctgttgccggtgctgtgccaggcccacggcttgaccccccagcaggtggtggccatcgccagcaataatggtggcaagcaggcgctggagacggtccagcggctgttgccggtgctgtgccaggcccacggcttgaccccccagcaggtggtggccatcgccagcaatggcggtggcaagcaggcgctggagacggtccagcggctgttgccggtgctgtgccaggcccacggcttgaccccccagcaggtggtggccatcgccagcaataatggtggcaagcaggcgctggagacggtccagcggctgttgccggtgctgtgccaggcccacggcttgacccctcagcaggtggtggccatcgccagcaatggcggcggcaggccggcgctggagagcattgttgcccagttatctcgccctgatccggcgttggccgcgttgaccaacgaccacctcgtcgccttggcctgcctcggcgggcgtcctgcgctggatgcagtgaaaaagggattgggggatcctatcagccgttcccagctggtgaagtccgagctggaggagaagaaatccgagttgaggcacaagctgaagtacgtgccccacgagtacatcgagctgatcgagatcgcccggaacagcacccaggaccgtatcctggagatgaaggtgatggagttcttcatgaaggtgtacggctacaggggcaagcacctgggcggctccaggaagcccgacggcgccatctacaccgtgggctcccccatcgactacggcgtgatcgtggacaccaaggcctactccggcggctacaacctgcccatcggccaggccgacgaaatgcagaggtacgtggaggagaaccagaccaggaacaagcacatcaaccccaacgagtggtggaaggtgtacccctccagcgtgaccgagttcaagttcctgttcgtgtccggccacttcaagggcaactacaaggcccagctgaccaggctgaaccacatcaccaactgcaacggcgccgtgctgtccgtggaggagctcctgatcggcggcgagatgatcaaggccggcaccctgaccctggaggaggtgaggaggaagttcaacaacggcgagatcaacttcgcggccgactgataa

SEQ ID NO: 53 - DNA, 2814 bp, Artificialsequence
  TRBC_T02-L TALEN
atgggcgatcctaaaaagaaacgtaaggtcatcgattacccatacgatgttccagattacgctatcgatatcgccgatctacgcacgctcggctacagccagcagcaacaggagaagatcaaaccgaaggttcgttcgacagtggcgcagcaccacgaggcactggtcggccacgggtttacacacgcgcacatcgttgcgttaagccaacacccggcagcgttagggaccgtcgctgtcaagtatcaggacatgatcgcagcgttgccagaggcgacacacgaagcgatcgttggcgtcggcaaacagtggtccggcgcacgcgctctggaggccttgctcacggtggcgggagagttgagaggtccaccgttacagttggacacaggccaacttctcaagattgcaaaacgtggcggcgtgaccgcagtggaggcagtgcatgcatggcgcaatgcactgacgggtgccccgctcaacttgaccccggagcaggtggtggccatcgccagccacgatggcggcaagcaggcgctggagacggtccagcggctgttgccggtgctgtgccaggcccacggcttgaccccggagcaggtggtggccatcgccagccacgatggcggcaagcaggcgctggagacggtccagcggctgttgccggtgctgtgccaggcccacggcttgaccccggagcaggtggtggccatcgccagccacgatggcggcaagcaggcgctggagacggtccagcggctgttgccggtgctgtgccaggcccacggcttgaccccggagcaggtggtggccatcgccagcaatattggtggcaagcaggcgctggagacggtgcaggcgctgttgccggtgctgtgccaggcccacggcttgaccccggagcaggtggtggccatcgccagccacgatggcggcaagcaggcgctggagacggtccagcggctgttgccggtgctgtgccaggcccacggcttgaccccggagcaggtggtggccatcgccagccacgatggcggcaagcaggcgctggagacggtccagcggctgttgccggtgctgtgccaggcccacggcttgaccccggagcaggtggtggccatcgccagccacgatggcggcaagcaggcgctggagacggtccagcggctgttgccggtgctgtgccaggcccacggcttgaccccccagcaggtggtggccatcgccagcaataatggtggcaagcaggcgctggagacggtccagcggctgttgccggtgctgtgccaggcccacggcttgaccccggagcaggtggtggccatcgccagcaatattggtggcaagcaggcgctggagacggtgcaggcgctgttgccggtgctgtgccaggcccacggcttgaccccccagcaggtggtggccatcgccagcaataatggtggcaagcaggcgctggagacggtccagcggctgttgccggtgctgtgccaggcccacggcttgaccccccagcaggtggtggccatcgccagcaataatggtggcaagcaggcgctggagacggtccagcggctgttgccggtgctgtgccaggcccacggcttgaccccccagcaggtggtggccatcgccagcaatggcggtggcaagcaggcgctggagacggtccagcggctgttgccggtgctgtgccaggcccacggcttgaccccggagcaggtggtggccatcgccagccacgatggcggcaagcaggcgctggagacggtccagcggctgttgccggtgctgtgccaggcccacggcttgaccccccagcaggtggtggccatcgccagcaataatggtggcaagcaggcgctggagacggtccagcggctgttgccggtgctgtgccaggcccacggcttgaccccggagcaggtggtggccatcgccagccacgatggcggcaagcaggcgctggagacggtccagcggctgttgccggtgctgtgccaggcccacggcttgacccctcagcaggtggtggccatcgccagcaatggcggcggcaggccggcgctggagagcattgttgcccagttatctcgccctgatccggcgttggccgcgttgaccaacgaccacctcgtcgccttggcctgcctcggcgggcgtcctgcgctggatgcagtgaaaaagggattgggggatcctatcagccgttcccagctggtgaagtccgagctggaggagaagaaatccgagttgaggcacaagctgaagtacgtgccccacgagtacatcgagctgatcgagatcgcccggaacagcacccaggaccgtatcctggagatgaaggtgatggagttcttcatgaaggtgtacggctacaggggcaagcacctgggcggctccaggaagcccgacggcgccatctacaccgtgggctcccccatcgactacggcgtgatcgtggacaccaaggcctactccggcggctacaacctgcccatcggccaggccgacgaaatgcagaggtacgtggaggagaaccagaccaggaacaagcacatcaaccccaacgagtggtggaaggtgtacccctccagcgtgaccgagttcaagttcctgttcgtgtccggccacttcaagggcaactacaaggcccagctgaccaggctgaaccacatcaccaactgcaacggcgccgtgctgtccgtggaggagctcctgatcggcggcgagatgatcaaggccggcaccctgaccctggaggaggtgaggaggaagttcaacaacggcgagatcaacttcgcggccgactgataa

SEQ ID NO: 54 - DNA, 2832 bp, Artificialsequence
  TRBC_T02-R TALEN
atgggcgatcctaaaaagaaacgtaaggtcatcgataaggagaccgccgctgccaagttcgagagacagcacatggacagcatcgatatcgccgatctacgcacgctcggctacagccagcagcaacaggagaagatcaaaccgaaggttcgttcgacagtggcgcagcaccacgaggcactggtcggccacgggtttacacacgcgcacatcgttgcgttaagccaacacccggcagcgttagggaccgtcgctgtcaagtatcaggacatgatcgcagcgttgccagaggcgacacacgaagcgatcgttggcgtcggcaaacagtggtccggcgcacgcgctctggaggccttgctcacggtggcgggagagttgagaggtccaccgttacagttggacacaggccaacttctcaagattgcaaaacgtggcggcgtgaccgcagtggaggcagtgcatgcatggcgcaatgcactgacgggtgccccgctcaacttgaccccccagcaggtggtggccatcgccagcaataatggtggcaagcaggcgctggagacggtccagcggctgttgccggtgctgtgccaggcccacggcttgaccccccagcaggtggtggccatcgccagcaataatggtggcaagcaggcgctggagacggtccagcggctgttgccggtgctgtgccaggcccacggcttgaccccccagcaggtggtggccatcgccagcaataatggtggcaagcaggcgctggagacggtccagcggctgttgccggtgctgtgccaggcccacggcttgaccccggagcaggtggtggccatcgccagcaatattggtggcaagcaggcgctggagacggtgcaggcgctgttgccggtgctgtgccaggcccacggcttgaccccccagcaggtggtggccatcgccagcaataatggtggcaagcaggcgctggagacggtccagcggctgttgccggtgctgtgccaggcccacggcttgaccccggagcaggtggtggccatcgccagcaatattggtggcaagcaggcgctggagacggtgcaggcgctgttgccggtgctgtgccaggcccacggcttgaccccccagcaggtggtggccatcgccagcaatggcggtggcaagcaggcgctggagacggtccagcggctgttgccggtgctgtgccaggcccacggcttgaccccggagcaggtggtggccatcgccagccacgatggcggcaagcaggcgctggagacggtccagcggctgttgccggtgctgtgccaggcccacggcttgaccccccagcaggtggtggccatcgccagcaatggcggtggcaagcaggcgctggagacggtccagcggctgttgccggtgctgtgccaggcccacggcttgaccccggagcaggtggtggccatcgccagccacgatggcggcaagcaggcgctggagacggtccagcggctgttgccggtgctgtgccaggcccacggcttgaccccccagcaggtggtggccatcgccagcaatggcggtggcaagcaggcgctggagacggtccagcggctgttgccggtgctgtgccaggcccacggcttgaccccccagcaggtggtggccatcgccagcaataatggtggcaagcaggcgctggagacggtccagcggctgttgccggtgctgtgccaggcccacggcttgaccccggagcaggtggtggccatcgccagccacgatggcggcaagcaggcgctggagacggtccagcggctgttgccggtgctgtgccaggcccacggcttgaccccccagcaggtggtggccatcgccagcaatggcggtggcaagcaggcgctggagacggtccagcggctgttgccggtgctgtgccaggcccacggcttgaccccccagcaggtggtggccatcgccagcaatggcggtggcaagcaggcgctggagacggtccagcggctgttgccggtgctgtgccaggcccacggcttgacccctcagcaggtggtggccatcgccagcaatggcggcggcaggccggcgctggagagcattgttgcccagttatctcgccctgatccggcgttggccgcgttgaccaacgaccacctcgtcgccttggcctgcctcggcgggcgtcctgcgctggatgcagtgaaaaagggattgggggatcctatcagccgttcccagctggtgaagtccgagctggaggagaagaaatccgagttgaggcacaagctgaagtacgtgccccacgagtacatcgagctgatcgagatcgcccggaacagcacccaggaccgtatcctggagatgaaggtgatggagttcttcatgaaggtgtacggctacaggggcaagcacctgggcggctccaggaagcccgacggcgccatctacaccgtgggctcccccatcgactacggcgtgatcgtggacaccaaggcctactccggcggctacaacctgcccatcggccaggccgacgaaatgcagaggtacgtggaggagaaccagaccaggaacaagcacatcaaccccaacgagtggtggaaggtgtacccctccagcgtgaccgagttcaagttcctgttcgtgtccggccacttcaagggcaactacaaggcccagctgaccaggctgaaccacatcaccaactgcaacggcgccgtgctgtccgtggaggagctcctgatcggcggcgagatgatcaaggccggcaccctgaccctggaggaggtgaggaggaagttcaacaacggcgagatcaacttcgcggccgactgataa

SEQ ID NO: 55 - DNA, 2814 bp, Artificialsequence
  CD52_T02-L TALEN
atgggcgatcctaaaaagaaacgtaaggtcatcgattacccatacgatgttccagattacgctatcgatatcgccgatctacgcacgctcggctacagccagcagcaacaggagaagatcaaaccgaaggttcgttcgacagtggcgcagcaccacgaggcactggtcggccacgggtttacacacgcgcacatcgttgcgttaagccaacacccggcagcgttagggaccgtcgctgtcaagtatcaggacatgatcgcagcgttgccagaggcgacacacgaagcgatcgttggcgtcggcaaacagtggtccggcgcacgcgctctggaggccttgctcacggtggcgggagagttgagaggtccaccgttacagttggacacaggccaacttctcaagattgcaaaacgtggcggcgtgaccgcagtggaggcagtgcatgcatggcgcaatgcactgacgggtgccccgctcaacttgaccccccagcaggtggtggccatcgccagcaatggcggtggcaagcaggcgctggagacggtccagcggctgttgccggtgctgtgccaggcccacggcttgaccccggagcaggtggtggccatcgccagccacgatggcggcaagcaggcgctggagacggtccagcggctgttgccggtgctgtgccaggcccacggcttgaccccggagcaggtggtggccatcgccagccacgatggcggcaagcaggcgctggagacggtccagcggctgttgccggtgctgtgccaggcccacggcttgaccccccagcaggtggtggccatcgccagcaatggcggtggcaagcaggcgctggagacggtccagcggctgttgccggtgctgtgccaggcccacggcttgaccccggagcaggtggtggccatcgccagccacgatggcggcaagcaggcgctggagacggtccagcggctgttgccggtgctgtgccaggcccacggcttgaccccggagcaggtggtggccatcgccagccacgatggcggcaagcaggcgctggagacggtccagcggctgttgccggtgctgtgccaggcccacggcttgaccccccagcaggtggtggccatcgccagcaatggcggtggcaagcaggcgctggagacggtccagcggctgttgccggtgctgtgccaggcccacggcttgaccccggagcaggtggtggccatcgccagcaatattggtggcaagcaggcgctggagacggtgcaggcgctgttgccggtgctgtgccaggcccacggcttgaccccggagcaggtggtggccatcgccagccacgatggcggcaagcaggcgctggagacggtccagcggctgttgccggtgctgtgccaggcccacggcttgaccccccagcaggtggtggccatcgccagcaatggcggtggcaagcaggcgctggagacggtccagcggctgttgccggtgctgtgccaggcccacggcttgaccccggagcaggtggtggccatcgccagccacgatggcggcaagcaggcgctggagacggtccagcggctgttgccggtgctgtgccaggcccacggcttgaccccggagcaggtggtggccatcgccagcaatattggtggcaagcaggcgctggagacggtgcaggcgctgttgccggtgctgtgccaggcccacggcttgaccccggagcaggtggtggccatcgccagccacgatggcggcaagcaggcgctggagacggtccagcggctgttgccggtgctgtgccaggcccacggcttgaccccggagcaggtggtggccatcgccagccacgatggcggcaagcaggcgctggagacggtccagcggctgttgccggtgctgtgccaggcccacggcttgaccccggagcaggtggtggccatcgccagcaatattggtggcaagcaggcgctggagacggtgcaggcgctgttgccggtgctgtgccaggcccacggcttgacccctcagcaggtggtggccatcgccagcaatggcggcggcaggccggcgctggagagcattgttgcccagttatctcgccctgatccggcgttggccgcgttgaccaacgaccacctcgtcgccttggcctgcctcggcgggcgtcctgcgctggatgcagtgaaaaagggattgggggatcctatcagccgttcccagctggtgaagtccgagctggaggagaagaaatccgagttgaggcacaagctgaagtacgtgccccacgagtacatcgagctgatcgagatcgcccggaacagcacccaggaccgtatcctggagatgaaggtgatggagttcttcatgaaggtgtacggctacaggggcaagcacctgggcggctccaggaagcccgacggcgccatctacaccgtgggctcccccatcgactacggcgtgatcgtggacaccaaggcctactccggcggctacaacctgcccatcggccaggccgacgaaatgcagaggtacgtggaggagaaccagaccaggaacaagcacatcaaccccaacgagtggtggaaggtgtacccctccagcgtgaccgagttcaagttcctgttcgtgtccggccacttcaagggcaactacaaggcccagctgaccaggctgaaccacatcaccaactgcaacggcgccgtgctgtccgtggaggagctcctgatcggcggcgagatgatcaaggccggcaccctgaccctggaggaggtgaggaggaagttcaacaacggcgagatcaacttcgcggccgactgataa

SEQ ID NO: 56 - DNA, 2832 bp, Artificialsequence
  CD52_T02-R TALEN
atgggcgatcctaaaaagaaacgtaaggtcatcgataaggagaccgccgctgccaagttcgagagacagcacatggacagcatcgatatcgccgatctacgcacgctcggctacagccagcagcaacaggagaagatcaaaccgaaggttcgttcgacagtggcgcagcaccacgaggcactggtcggccacgggtttacacacgcgcacatcgttgcgttaagccaacacccggcagcgttagggaccgtcgctgtcaagtatcaggacatgatcgcagcgttgccagaggcgacacacgaagcgatcgttggcgtcggcaaacagtggtccggcgcacgcgctctggaggccttgctcacggtggcgggagagttgagaggtccaccgttacagttggacacaggccaacttctcaagattgcaaaacgtggcggcgtgaccgcagtggaggcagtgcatgcatggcgcaatgcactgacgggtgccccgctcaacttgaccccccagcaggtggtggccatcgccagcaatggcggtggcaagcaggcgctggagacggtccagcggctgttgccggtgctgtgccaggcccacggcttgaccccccagcaggtggtggccatcgccagcaataatggtggcaagcaggcgctggagacggtccagcggctgttgccggtgctgtgccaggcccacggcttgaccccggagcaggtggtggccatcgccagccacgatggcggcaagcaggcgctggagacggtccagcggctgttgccggtgctgtgccaggcccacggcttgaccccccagcaggtggtggccatcgccagcaatggcggtggcaagcaggcgctggagacggtccagcggctgttgccggtgctgtgccaggcccacggcttgaccccggagcaggtggtggccatcgccagccacgatggcggcaagcaggcgctggagacggtccagcggctgttgccggtgctgtgccaggcccacggcttgaccccccagcaggtggtggccatcgccagcaatggcggtggcaagcaggcgctggagacggtccagcggctgttgccggtgctgtgccaggcccacggcttgaccccccagcaggtggtggccatcgccagcaatggcggtggcaagcaggcgctggagacggtccagcggctgttgccggtgctgtgccaggcccacggcttgaccccggagcaggtggtggccatcgccagcaatattggtggcaagcaggcgctggagacggtgcaggcgctgttgccggtgctgtgccaggcccacggcttgaccccggagcaggtggtggccatcgccagccacgatggcggcaagcaggcgctggagacggtccagcggctgttgccggtgctgtgccaggcccacggcttgaccccggagcaggtggtggccatcgccagccacgatggcggcaagcaggcgctggagacggtccagcggctgttgccggtgctgtgccaggcccacggcttgaccccccagcaggtggtggccatcgccagcaatggcggtggcaagcaggcgctggagacggtccagcggctgttgccggtgctgtgccaggcccacggcttgaccccccagcaggtggtggccatcgccagcaataatggtggcaagcaggcgctggagacggtccagcggctgttgccggtgctgtgccaggcccacggcttgaccccccagcaggtggtggccatcgccagcaatggcggtggcaagcaggcgctggagacggtccagcggctgttgccggtgctgtgccaggcccacggcttgaccccggagcaggtggtggccatcgccagcaatattggtggcaagcaggcgctggagacggtgcaggcgctgttgccggtgctgtgccaggcccacggcttgaccccggagcaggtggtggccatcgccagccacgatggcggcaagcaggcgctggagacggtccagcggctgttgccggtgctgtgccaggcccacggcttgacccctcagcaggtggtggccatcgccagcaatggcggcggcaggccggcgctggagagcattgttgcccagttatctcgccctgatccggcgttggccgcgttgaccaacgaccacctcgtcgccttggcctgcctcggcgggcgtcctgcgctggatgcagtgaaaaagggattgggggatcctatcagccgttcccagctggtgaagtccgagctggaggagaagaaatccgagttgaggcacaagctgaagtacgtgccccacgagtacatcgagctgatcgagatcgcccggaacagcacccaggaccgtatcctggagatgaaggtgatggagttcttcatgaaggtgtacggctacaggggcaagcacctgggcggctccaggaagcccgacggcgccatctacaccgtgggctcccccatcgactacggcgtgatcgtggacaccaaggcctactccggcggctacaacctgcccatcggccaggccgacgaaatgcagaggtacgtggaggagaaccagaccaggaacaagcacatcaaccccaacgagtggtggaaggtgtacccctccagcgtgaccgagttcaagttcctgttcgtgtccggccacttcaagggcaactacaaggcccagctgaccaggctgaaccacatcaccaactgcaacggcgccgtgctgtccgtggaggagctcctgatcggcggcgagatgatcaaggccggcaccctgaccctggaggaggtgaggaggaagttcaacaacggcgagatcaacttcgcggccgactgataa

SEQ ID NO: 57 - DNA, 49 bp, Artificialsequence
  TRAC_T02
tttagaaagttcctgtgatgtcaagctggtcgagaaaagctttgaaaca

SEQ ID NO: 58 - DNA, 49 bp, Artificialsequence
  TRAC_T03
tccagtgacaagtctgtctgcctattcaccgattttgattctcaaacaa

SEQ ID NO: 59 - DNA, 49 bp, Artificialsequence
  TRAC_T04
tatatcacagacaaaactgtgctagacatgaggtctatggacttcaaga

SEQ ID NO: 60 - DNA, 49 bp, Artificialsequence
  TRAC_T05
tgaggtctatggacttcaagagcaacagtgctgtggcctggagcaacaa

SEQ ID NO: 61 - DNA, 47 bp, Artificial sequence
  CD52_T01
ttcctcttcctcctaccaccatcagcctcctttacctgtaccataac

SEQ ID NO: 62 - DNA, 43 bp, Artificial sequence
  CD52_T04
ttcctcctactcaccacagcctcctggtcttacctgtaccata

SEQ ID NO: 63 - DNA, 43 bp, Artificial sequence
  CD52_T05
tcctactcaccatcagctcctggttatttgctcttacctgtac

SEQ ID NO: 64 - DNA, 47 bp, Artificial sequence
  CD52_T06
ttatcccacttctcctctacagatacaaactttttgtcctgagagtc

SEQ ID NO: 65 - DNA, 47 bp, Artificial sequence
  CD52_T07
tggactctcaggacaaacgacaccagccaaatgctgaggggctgctg

SEQ ID NO: 66 - DNA, 60 bp, Artificial sequence
  Forward primer CD52
  misc_feature (31); (32); (33); (34); (35); (36); (37); (38); (39); (40): n is a or c or t or g
ccatctcatccctgcgtgtctccgactcagnnnnnnnnnncagatctgcagaaaggaagc

SEQ ID NO: 67 - DNA, 61 bp, Artificial sequence
  Forward primer TRAC
  misc_feature (31); (32); (33); (34); (35); (36); (37); (38); (39); (40): n is a or c or t or g
ccatctcatccctgcgtgtctccgactcagnnnnnnnnnnatcactggcatctggactcca

SEQ ID NO: 68 - DNA, 62 bp, Artificial sequence
  Forward primer TRBC1
  misc_feature (31); (32); (33); (34); (35); (36); (37); (38); (39); (40): n is a or c or t or g
ccatctcatccctgcgtgtctccgactcagnnnnnnnnnnagagcccctaccagaaccagac

SEQ ID NO: 69 - DNA, 62 bp, Artificial sequence
  Forward primer TRBC2
  misc_feature (31); (32); (33); (34); (35); (36); (37); (38); (39); (40): n is a or c or t or g
ccatctcatccctgcgtgtctccgactcagnnnnnnnnnnggacctagtaacataattgtgc

SEQ ID NO: 70 - DNA, 51 bp, Artificial sequence
  Reverse primer GR CD52
cctatcccctgtgtgccttggcagtctcagcctgttggagtccatctgctg

SEQ ID NO: 71 - DNA, 50 bp, Artificial sequence
  Reverse primer GR TRAC
cctatcccctgtgtgccttggcagtctcagcctcatgtctagcacagttt

SEQ ID NO: 72 - DNA, 51 bp, Artificial sequence
  Reverse primer GR TRBC1-2
cctatcccctgtgtgccttggcagtctcagaccagctcagctccacgtggt

SEQ ID NO: 73 - protein, 495 aa, Artificial sequence
  anti-CD19 CAR
METDTLLLWVLLLWVPGSTGEVQLQQSGPELIKPGASVKMSCKASGYTFTSYVMHWVKQKPGQGLEWIGYINPYNDGTKYNEKFKGKATLTSDKSSSTAYMELSSLTSEDSAVYYCARGTYYYGSRVFDYWGQGTTLTVSSGGGGSGGGGSGGGGSDIVMTQAAPSIPVTPGESVSISCRSSKSLLNSNGNTYLYWFLQRPGQSPQLLIYRMSNLASGVPDRFSGSGSGTAFTLRISRVEAEDVGVYYCMQHLEYPFTFGAGTKLELKRSDPTTTPAPRPPTPAPTIASQPLSLRPEACRPAAGGAVHTRGLDFACDIYIWAPLAGTCGVLLLSLVITLYCKRGRKKLLYIFKQPFMRPVQTTQEEDGCSCRFPEEEEGGCELRVKFSRSADAPAYQQGQNQLYNELNLGRREEYDVLDKRRGRDPEMGGKPRRKNPQEGLYNELQKDKMAEAYSEIGMKGERRRGKGHDGLYQGLSTATKDTYDALHMQALPPR

SEQ ID NO: 74 - DNA, 49 bp, Artificial sequence
  CTLA4_T01
tggccctgcactctcctgttttttcttctcttcatccctgtcttctgca

SEQ ID NO: 75 - DNA, 49 bp, Artificial sequence
  CTLA4_T03
ttttccatgctagcaatgcacgtggcccagcctgctgtggtactggcca

SEQ ID NO: 76 - DNA, 49 bp, Artificial sequence
  CTLA4_T04
tccatgctagcaatgcacgtggcccagcctgctgtggtactggccagca

SEQ ID NO: 77 - DNA, 49 bp, Artificial sequence
  PDCD1_T01
ttctccccagccctgctcgtggtgaccgaaggggacaacgccaccttca

SEQ ID NO: 78 - DNA, 49 bp, Artificial sequence
  PDCD1_T03
tacctctgtggggccatctccctggcccccaaggcgcagatcaaagaga

SEQ ID NO: 79 - protein, 530 aa, Artificial sequence
  Repeat CTLA4_T01-L
LTPQQVVAIASNNGGKQALETVQRLLPVLCQAHGLTPQQVVAIASNNGGKQALETVQRLLPVLCQAHGLTPEQVVAIASHDGGKQALETVQRLLPVLCQAHGLTPEQVVAIASHDGGKQALETVQRLLPVLCQAHGLTPEQVVAIASHDGGKQALETVQRLLPVLCQAHGLTPQQVVAIASNGGGKQALETVQRLLPVLCQAHGLTPQQVVAIASNNGGKQALETVQRLLPVLCQAHGLTPEQVVAIASHDGGKQALETVQRLLPVLCQAHGLTPEQVVAIASNIGGKQALETVQALLPVLCQAHGLTPEQVVAIASHDGGKQALETVQRLLPVLCQAHGLTPQQVVAIASNGGGKQALETVQRLLPVLCQAHGLTPEQVVAIASHDGGKQALETVQRLLPVLCQAHGLTPQQVVAIASNGGGKQALETVQRLLPVLCQAHGLTPEQVVAIASHDGGKQALETVQRLLPVLCQAHGLTPEQVVAIASHDGGKQALETVQRLLPVLCQAHGLTPQQVVAIASNGGGRPALE

SEQ ID NO: 80 - protein, 530 aa, Artificial sequence
  Repeat CTLA4_T01-R
LTPQQVVAIASNNGGKQALETVQRLLPVLCQAHGLTPEQVVAIASHDGGKQALETVQRLLPVLCQAHGLTPEQVVAIASNIGGKQALETVQALLPVLCQAHGLTPQQVVAIASNNGGKQALETVQRLLPVLCQAHGLTPEQVVAIASNIGGKQALETVQALLPVLCQAHGLTPEQVVAIASNIGGKQALETVQALLPVLCQAHGLTPQQVVAIASNNGGKQALETVQRLLPVLCQAHGLTPEQVVAIASNIGGKQALETVQALLPVLCQAHGLTPEQVVAIASHDGGKQALETVQRLLPVLCQAHGLTPEQVVAIASNIGGKQALETVQALLPVLCQAHGLTPQQVVAIASNNGGKQALETVQRLLPVLCQAHGLTPQQVVAIASNNGGKQALETVQRLLPVLCQAHGLTPQQVVAIASNNGGKQALETVQRLLPVLCQAHGLTPEQVVAIASNIGGKQALETVQALLPVLCQAHGLTPQQVVAIASNGGGKQALETVQRLLPVLCQAHGLTPQQVVAIASNGGGRPALE

SEQ ID NO: 81 - protein, 530 aa, Artificial sequence
  RepeatCTLA4_T03-L
LTPQQVVAIASNGGGKQALETVQRLLPVLCQAHGLTPQQVVAIASNGGGKQALETVQRLLPVLCQAHGLTPQQVVAIASNGGGKQALETVQRLLPVLCQAHGLTPEQVVAIASHDGGKQALETVQRLLPVLCQAHGLTPEQVVAIASHDGGKQALETVQRLLPVLCQAHGLTPEQVVAIASNIGGKQALETVQALLPVLCQAHGLTPQQVVAIASNGGGKQALETVQRLLPVLCQAHGLTPQQVVAIASNNGGKQALETVQRLLPVLCQAHGLTPEQVVAIASHDGGKQALETVQRLLPVLCQAHGLTPQQVVAIASNGGGKQALETVQRLLPVLCQAHGLTPEQVVAIASNIGGKQALETVQALLPVLCQAHGLTPQQVVAIASNNGGKQALETVQRLLPVLCQAHGLTPEQVVAIASHDGGKQALETVQRLLPVLCQAHGLTPEQVVAIASNIGGKQALETVQALLPVLCQAHGLTPEQVVAIASNIGGKQALETVQALLPVLCQAHGLTPQQVVAIASNGGGRPALE

SEQ ID NO: 82 - protein, 530 aa, Artificial sequence
  Repeat CTLA4_T03-R
LTPQQVVAIASNNGGKQALETVQRLLPVLCQAHGLTPQQVVAIASNNGGKQALETVQRLLPVLCQAHGLTPEQVVAIASHDGGKQALETVQRLLPVLCQAHGLTPEQVVAIASHDGGKQALETVQRLLPVLCQAHGLTPEQVVAIASNIGGKQALETVQALLPVLCQAHGLTPQQVVAIASNNGGKQALETVQRLLPVLCQAHGLTPQQVVAIASNGGGKQALETVQRLLPVLCQAHGLTPEQVVAIASNIGGKQALETVQALLPVLCQAHGLTPEQVVAIASHDGGKQALETVQRLLPVLCQAHGLTPEQVVAIASHDGGKQALETVQRLLPVLCQAHGLTPEQVVAIASNIGGKQALETVQALLPVLCQAHGLTPEQVVAIASHDGGKQALETVQRLLPVLCQAHGLTPEQVVAIASNIGGKQALETVQALLPVLCQAHGLTPQQVVAIASNNGGKQALETVQRLLPVLCQAHGLTPEQVVAIASHDGGKQALETVQRLLPVLCQAHGLTPQQVVAIASNGGGRPALE

SEQ ID NO: 83 - protein, 530 aa, Artificial sequence
  Repeat CTLA4_T04-L
LTPEQVVAIASHDGGKQALETVQRLLPVLCQAHGLTPEQVVAIASHDGGKQALETVQRLLPVLCQAHGLTPEQVVAIASNIGGKQALETVQALLPVLCQAHGLTPQQVVAIASNGGGKQALETVQRLLPVLCQAHGLTPQQVVAIASNNGGKQALETVQRLLPVLCQAHGLTPEQVVAIASHDGGKQALETVQRLLPVLCQAHGLTPQQVVAIASNGGGKQALETVQRLLPVLCQAHGLTPEQVVAIASNIGGKQALETVQALLPVLCQAHGLTPQQVVAIASNNGGKQALETVQRLLPVLCQAHGLTPEQVVAIASHDGGKQALETVQRLLPVLCQAHGLTPEQVVAIASNIGGKQALETVQALLPVLCQAHGLTPEQVVAIASNIGGKQALETVQALLPVLCQAHGLTPQQVVAIASNGGGKQALETVQRLLPVLCQAHGLTPQQVVAIASNNGGKQALETVQRLLPVLCQAHGLTPEQVVAIASHDGGKQALETVQRLLPVLCQAHGLTPQQVVAIASNGGGRPALE

SEQ ID NO: 84 - protein, 530 aa, Artificial sequence
  Repeat CTLA4_T04-R
LTPQQVVAIASNNGGKQALETVQRLLPVLCQAHGLTPEQVVAIASHDGGKQALETVQRLLPVLCQAHGLTPQQVVAIASNGGGKQALETVQRLLPVLCQAHGLTPQQVVAIASNNGGKQALETVQRLLPVLCQAHGLTPQQVVAIASNNGGKQALETVQRLLPVLCQAHGLTPEQVVAIASHDGGKQALETVQRLLPVLCQAHGLTPEQVVAIASHDGGKQALETVQRLLPVLCQAHGLTPEQVVAIASNIGGKQALETVQALLPVLCQAHGLTPQQVVAIASNNGGKQALETVQRLLPVLCQAHGLTPQQVVAIASNGGGKQALETVQRLLPVLCQAHGLTPEQVVAIASNIGGKQALETVQALLPVLCQAHGLTPEQVVAIASHDGGKQALETVQRLLPVLCQAHGLTPEQVVAIASHDGGKQALETVQRLLPVLCQAHGLTPEQVVAIASNIGGKQALETVQALLPVLCQAHGLTPEQVVAIASHDGGKQALETVQRLLPVLCQAHGLTPQQVVAIASNGGGRPALE

SEQ ID NO: 85 - protein, 530 aa, Artificial sequence
  Repeat PDCD1_T01-L
LTPQQVVAIASNGGGKQALETVQRLLPVLCQAHGLTPEQVVAIASHDGGKQALETVQRLLPVLCQAHGLTPQQVVAIASNGGGKQALETVQRLLPVLCQAHGLTPEQVVAIASHDGGKQALETVQRLLPVLCQAHGLTPEQVVAIASHDGGKQALETVQRLLPVLCQAHGLTPEQVVAIASHDGGKQALETVQRLLPVLCQAHGLTPEQVVAIASHDGGKQALETVQRLLPVLCQAHGLTPEQVVAIASNIGGKQALETVQALLPVLCQAHGLTPQQVVAIASNNGGKQALETVQRLLPVLCQAHGLTPEQVVAIASHDGGKQALETVQRLLPVLCQAHGLTPEQVVAIASHDGGKQALETVQRLLPVLCQAHGLTPEQVVAIASHDGGKQALETVQRLLPVLCQAHGLTPQQVVAIASNGGGKQALETVQRLLPVLCQAHGLTPQQVVAIASNNGGKQALETVQRLLPVLCQAHGLTPEQVVAIASHDGGKQALETVQRLLPVLCQAHGLTPQQVVAIASNGGGRPALE

SEQ ID NO: 86 - protein, 529 aa, Artificial sequence
  RepeatPDCD1_T01-R
LTPQQVVAIASNNGGKQALETVQRLLPVLCQAHGLTPEQVVAIASNIGGKQALETVQALLPVLCQAHGLTPEQVVAIASNIGGKQALETVQALLPVLCQAHGLTPQQVVAIASNNGGKQALETVQRLLPVLCQAHGLTPQQVVAIASNNGGKQALETVQRLLPVLCQAHGLTPQQVVAIASNGGGKQALETVQRLLPVLCQAHGLTPQQVVAIASNNGGKQALETVQRLLPVLCQAHGLTPQQVVAIASNNGGKQALETVQRLLPVLCQAHGLTPEQVVAIASNGGKQALETVQRLLPVLCQAHGLTPQQVVAIASNNGGKQALETVQRLLPVLCQAHGLTPQQVVAIASNGGGKQALETVQRLLPVLCQAHGLTPQQVVAIASNGGGKQALETVQRLLPVLCQAHGLTPQQVVAIASNNGGKQALETVQRLLPVLCQAHGLTPQQVVAIASNGGGKQALETVQRLLPVLCQAHGLTPEQVVAIASHDGGKQALETVQRLLPVLCQAHGLTPQQVVAIASNGGGRPALE

SEQ ID NO: 87 - protein, 530 aa, Artificial sequence
  Repeat PDCD1_T03-L
LTPEQVVAIASNIGGKQALETVQALLPVLCQAHGLTPEQVVAIASHDGGKQALETVQRLLPVLCQAHGLTPEQVVAIASHDGGKQALETVQRLLPVLCQAHGLTPQQVVAIASNGGGKQALETVQRLLPVLCQAHGLTPEQVVAIASHDGGKQALETVQRLLPVLCQAHGLTPQQVVAIASNGGGKQALETVQRLLPVLCQAHGLTPQQVVAIASNNGGKQALETVQRLLPVLCQAHGLTPQQVVAIASNGGGKQALETVQRLLPVLCQAHGLTPQQVVAIASNNGGKQALETVQRLLPVLCQAHGLTPQQVVAIASNNGGKQALETVQRLLPVLCQAHGLTPQQVVAIASNNGGKQALETVQRLLPVLCQAHGLTPQQVVAIASNNGGKQALETVQRLLPVLCQAHGLTPEQVVAIASHDGGKQALETVQRLLPVLCQAHGLTPEQVVAIASHDGGKQALETVQRLLPVLCQAHGLTPEQVVAIASNIGGKQALETVQALLPVLCQAHGLTPQQVVAIASNGGGRPALE

SEQ ID NO: 88 - protein, 529 aa, Artificial sequence
  Repeat PDCD1_T03-R
LTPEQVVAIASHDGGKQALETVQRLLPVLCQAHGLTPQQVVAIASNGGGKQALETVQRLLPVLCQAHGLTPEQVVAIASHDGGKQALETVQRLLPVLCQAHGLTPQQVVAIASNGGGKQALETVQRLLPVLCQAHGLTPQQVVAIASNGGGKQALETVQRLLPVLCQAHGLTPQQVVAIASNGGGKQALETVQRLLPVLCQAHGLTPQQVVAIASNNGGKQALETVQRLLPVLCQAHGLTPEQVVAIASNIGGKQALETVQALLPVLCQAHGLTPQQVVAIASNGGGKQALETVQRLLPVLCQAHGLTPEQVVAIASHDGGKQALETVQRLLPVLCQAHGLTPQQVVAIASNGGGKQALETVQRLLPVLCQAHGLTPQQVVAIASNNGGKQALETVQRLLPVLCQAHGLTPEQVVAIASNGGKQALETVQRLLPVLCQAHGLTPQQVVAIASNNGGKQALETVQRLLPVLCQAHGLTPEQVVAIASHDGGKQALETVQRLLPVLCQAHGLTPQQVVAIASNGGGRPALE

SEQ ID NO: 89 - DNA, 2814 bp, Artificial sequence
  CTLA4_T01-L  TALEN
atgggcgatcctaaaaagaaacgtaaggtcatcgattacccatacgatgttccagattacgctatcgatatcgccgatctacgcacgctcggctacagccagcagcaacaggagaagatcaaaccgaaggttcgttcgacagtggcgcagcaccacgaggcactggtcggccacgggtttacacacgcgcacatcgttgcgttaagccaacacccggcagcgttagggaccgtcgctgtcaagtatcaggacatgatcgcagcgttgccagaggcgacacacgaagcgatcgttggcgtcggcaaacagtggtccggcgcacgcgctctggaggccttgctcacggtggcgggagagttgagaggtccaccgttacagttggacacaggccaacttctcaagattgcaaaacgtggcggcgtgaccgcagtggaggcagtgcatgcatggcgcaatgcactgacgggtgccccgctcaacttgaccccccagcaggtggtggccatcgccagcaataatggtggcaagcaggcgctggagacggtccagcggctgttgccggtgctgtgccaggcccacggcttgaccccccagcaggtggtggccatcgccagcaataatggtggcaagcaggcgctggagacggtccagcggctgttgccggtgctgtgccaggcccacggcttgaccccggagcaggtggtggccatcgccagccacgatggcggcaagcaggcgctggagacggtccagcggctgttgccggtgctgtgccaggcccacggcttgaccccggagcaggtggtggccatcgccagccacgatggcggcaagcaggcgctggagacggtccagcggctgttgccggtgctgtgccaggcccacggcttgaccccggagcaggtggtggccatcgccagccacgatggcggcaagcaggcgctggagacggtccagcggctgttgccggtgctgtgccaggcccacggcttgaccccccagcaggtggtggccatcgccagcaatggcggtggcaagcaggcgctggagacggtccagcggctgttgccggtgctgtgccaggcccacggcttgaccccccagcaggtggtggccatcgccagcaataatggtggcaagcaggcgctggagacggtccagcggctgttgccggtgctgtgccaggcccacggcttgaccccggagcaggtggtggccatcgccagccacgatggcggcaagcaggcgctggagacggtccagcggctgttgccggtgctgtgccaggcccacggcttgaccccggagcaggtggtggccatcgccagcaatattggtggcaagcaggcgctggagacggtgcaggcgctgttgccggtgctgtgccaggcccacggcttgaccccggagcaggtggtggccatcgccagccacgatggcggcaagcaggcgctggagacggtccagcggctgttgccggtgctgtgccaggcccacggcttgaccccccagcaggtggtggccatcgccagcaatggcggtggcaagcaggcgctggagacggtccagcggctgttgccggtgctgtgccaggcccacggcttgaccccggagcaggtggtggccatcgccagccacgatggcggcaagcaggcgctggagacggtccagcggctgttgccggtgctgtgccaggcccacggcttgaccccccagcaggtggtggccatcgccagcaatggcggtggcaagcaggcgctggagacggtccagcggctgttgccggtgctgtgccaggcccacggcttgaccccggagcaggtggtggccatcgccagccacgatggcggcaagcaggcgctggagacggtccagcggctgttgccggtgctgtgccaggcccacggcttgaccccggagcaggtggtggccatcgccagccacgatggcggcaagcaggcgctggagacggtccagcggctgttgccggtgctgtgccaggcccacggcttgacccctcagcaggtggtggccatcgccagcaatggcggcggcaggccggcgctggagagcattgttgcccagttatctcgccctgatccggcgttggccgcgttgaccaacgaccacctcgtcgccttggcctgcctcggcgggcgtcctgcgctggatgcagtgaaaaagggattgggggatcctatcagccgttcccagctggtgaagtccgagctggaggagaagaaatccgagttgaggcacaagctgaagtacgtgccccacgagtacatcgagctgatcgagatcgcccggaacagcacccaggaccgtatcctggagatgaaggtgatggagttcttcatgaaggtgtacggctacaggggcaagcacctgggcggctccaggaagcccgacggcgccatctacaccgtgggctcccccatcgactacggcgtgatcgtggacaccaaggcctactccggcggctacaacctgcccatcggccaggccgacgaaatgcagaggtacgtggaggagaaccagaccaggaacaagcacatcaaccccaacgagtggtggaaggtgtacccctccagcgtgaccgagttcaagttcctgttcgtgtccggccacttcaagggcaactacaaggcccagctgaccaggctgaaccacatcaccaactgcaacggcgccgtgctgtccgtggaggagctcctgatcggcggcgagatgatcaaggccggcaccctgaccctggaggaggtgaggaggaagttcaacaacggcgagatcaacttcgcggccgactgataa

SEQ ID NO: 90 - DNA, 2832 bp, Artificial sequence
  CTLA4_T01-R TALEN
atgggcgatcctaaaaagaaacgtaaggtcatcgataaggagaccgccgctgccaagttcgagagacagcacatggacagcatcgatatcgccgatctacgcacgctcggctacagccagcagcaacaggagaagatcaaaccgaaggttcgttcgacagtggcgcagcaccacgaggcactggtcggccacgggtttacacacgcgcacatcgttgcgttaagccaacacccggcagcgttagggaccgtcgctgtcaagtatcaggacatgatcgcagcgttgccagaggcgacacacgaagcgatcgttggcgtcggcaaacagtggtccggcgcacgcgctctggaggccttgctcacggtggcgggagagttgagaggtccaccgttacagttggacacaggccaacttctcaagattgcaaaacgtggcggcgtgaccgcagtggaggcagtgcatgcatggcgcaatgcactgacgggtgccccgctcaacttgaccccccagcaggtggtggccatcgccagcaataatggtggcaagcaggcgctggagacggtccagcggctgttgccggtgctgtgccaggcccacggcttgaccccggagcaggtggtggccatcgccagccacgatggcggcaagcaggcgctggagacggtccagcggctgttgccggtgctgtgccaggcccacggcttgaccccggagcaggtggtggccatcgccagcaatattggtggcaagcaggcgctggagacggtgcaggcgctgttgccggtgctgtgccaggcccacggcttgaccccccagcaggtggtggccatcgccagcaataatggtggcaagcaggcgctggagacggtccagcggctgttgccggtgctgtgccaggcccacggcttgaccccggagcaggtggtggccatcgccagcaatattggtggcaagcaggcgctggagacggtgcaggcgctgttgccggtgctgtgccaggcccacggcttgaccccggagcaggtggtggccatcgccagcaatattggtggcaagcaggcgctggagacggtgcaggcgctgttgccggtgctgtgccaggcccacggcttgaccccccagcaggtggtggccatcgccagcaataatggtggcaagcaggcgctggagacggtccagcggctgttgccggtgctgtgccaggcccacggcttgaccccggagcaggtggtggccatcgccagcaatattggtggcaagcaggcgctggagacggtgcaggcgctgttgccggtgctgtgccaggcccacggcttgaccccggagcaggtggtggccatcgccagccacgatggcggcaagcaggcgctggagacggtccagcggctgttgccggtgctgtgccaggcccacggcttgaccccggagcaggtggtggccatcgccagcaatattggtggcaagcaggcgctggagacggtgcaggcgctgttgccggtgctgtgccaggcccacggcttgaccccccagcaggtggtggccatcgccagcaataatggtggcaagcaggcgctggagacggtccagcggctgttgccggtgctgtgccaggcccacggcttgaccccccagcaggtggtggccatcgccagcaataatggtggcaagcaggcgctggagacggtccagcggctgttgccggtgctgtgccaggcccacggcttgaccccccagcaggtggtggccatcgccagcaataatggtggcaagcaggcgctggagacggtccagcggctgttgccggtgctgtgccaggcccacggcttgaccccggagcaggtggtggccatcgccagcaatattggtggcaagcaggcgctggagacggtgcaggcgctgttgccggtgctgtgccaggcccacggcttgaccccccagcaggtggtggccatcgccagcaatggcggtggcaagcaggcgctggagacggtccagcggctgttgccggtgctgtgccaggcccacggcttgacccctcagcaggtggtggccatcgccagcaatggcggcggcaggccggcgctggagagcattgttgcccagttatctcgccctgatccggcgttggccgcgttgaccaacgaccacctcgtcgccttggcctgcctcggcgggcgtcctgcgctggatgcagtgaaaaagggattgggggatcctatcagccgttcccagctggtgaagtccgagctggaggagaagaaatccgagttgaggcacaagctgaagtacgtgccccacgagtacatcgagctgatcgagatcgcccggaacagcacccaggaccgtatcctggagatgaaggtgatggagttcttcatgaaggtgtacggctacaggggcaagcacctgggcggctccaggaagcccgacggcgccatctacaccgtgggctcccccatcgactacggcgtgatcgtggacaccaaggcctactccggcggctacaacctgcccatcggccaggccgacgaaatgcagaggtacgtggaggagaaccagaccaggaacaagcacatcaaccccaacgagtggtggaaggtgtacccctccagcgtgaccgagttcaagttcctgttcgtgtccggccacttcaagggcaactacaaggcccagctgaccaggctgaaccacatcaccaactgcaacggcgccgtgctgtccgtggaggagctcctgatcggcggcgagatgatcaaggccggcaccctgaccctggaggaggtgaggaggaagttcaacaacggcgagatcaacttcgcggccgactgataa

SEQ ID NO: 91 - DNA, 2814 bp, Artificial sequence
  CTLA4_T03-L TALEN
atgggcgatcctaaaaagaaacgtaaggtcatcgattacccatacgatgttccagattacgctatcgatatcgccgatctacgcacgctcggctacagccagcagcaacaggagaagatcaaaccgaaggttcgttcgacagtggcgcagcaccacgaggcactggtcggccacgggtttacacacgcgcacatcgttgcgttaagccaacacccggcagcgttagggaccgtcgctgtcaagtatcaggacatgatcgcagcgttgccagaggcgacacacgaagcgatcgttggcgtcggcaaacagtggtccggcgcacgcgctctggaggccttgctcacggtggcgggagagttgagaggtccaccgttacagttggacacaggccaacttctcaagattgcaaaacgtggcggcgtgaccgcagtggaggcagtgcatgcatggcgcaatgcactgacgggtgccccgctcaacttgaccccccagcaggtggtggccatcgccagcaatggcggtggcaagcaggcgctggagacggtccagcggctgttgccggtgctgtgccaggcccacggcttgaccccccagcaggtggtggccatcgccagcaatggcggtggcaagcaggcgctggagacggtccagcggctgttgccggtgctgtgccaggcccacggcttgaccccccagcaggtggtggccatcgccagcaatggcggtggcaagcaggcgctggagacggtccagcggctgttgccggtgctgtgccaggcccacggcttgaccccggagcaggtggtggccatcgccagccacgatggcggcaagcaggcgctggagacggtccagcggctgttgccggtgctgtgccaggcccacggcttgaccccggagcaggtggtggccatcgccagccacgatggcggcaagcaggcgctggagacggtccagcggctgttgccggtgctgtgccaggcccacggcttgaccccggagcaggtggtggccatcgccagcaatattggtggcaagcaggcgctggagacggtgcaggcgctgttgccggtgctgtgccaggcccacggcttgaccccccagcaggtggtggccatcgccagcaatggcggtggcaagcaggcgctggagacggtccagcggctgttgccggtgctgtgccaggcccacggcttgaccccccagcaggtggtggccatcgccagcaataatggtggcaagcaggcgctggagacggtccagcggctgttgccggtgctgtgccaggcccacggcttgaccccggagcaggtggtggccatcgccagccacgatggcggcaagcaggcgctggagacggtccagcggctgttgccggtgctgtgccaggcccacggcttgaccccccagcaggtggtggccatcgccagcaatggcggtggcaagcaggcgctggagacggtccagcggctgttgccggtgctgtgccaggcccacggcttgaccccggagcaggtggtggccatcgccagcaatattggtggcaagcaggcgctggagacggtgcaggcgctgttgccggtgctgtgccaggcccacggcttgaccccccagcaggtggtggccatcgccagcaataatggtggcaagcaggcgctggagacggtccagcggctgttgccggtgctgtgccaggcccacggcttgaccccggagcaggtggtggccatcgccagccacgatggcggcaagcaggcgctggagacggtccagcggctgttgccggtgctgtgccaggcccacggcttgaccccggagcaggtggtggccatcgccagcaatattggtggcaagcaggcgctggagacggtgcaggcgctgttgccggtgctgtgccaggcccacggcttgaccccggagcaggtggtggccatcgccagcaatattggtggcaagcaggcgctggagacggtgcaggcgctgttgccggtgctgtgccaggcccacggcttgacccctcagcaggtggtggccatcgccagcaatggcggcggcaggccggcgctggagagcattgttgcccagttatctcgccctgatccggcgttggccgcgttgaccaacgaccacctcgtcgccttggcctgcctcggcgggcgtcctgcgctggatgcagtgaaaaagggattgggggatcctatcagccgttcccagctggtgaagtccgagctggaggagaagaaatccgagttgaggcacaagctgaagtacgtgccccacgagtacatcgagctgatcgagatcgcccggaacagcacccaggaccgtatcctggagatgaaggtgatggagttcttcatgaaggtgtacggctacaggggcaagcacctgggcggctccaggaagcccgacggcgccatctacaccgtgggctcccccatcgactacggcgtgatcgtggacaccaaggcctactccggcggctacaacctgcccatcggccaggccgacgaaatgcagaggtacgtggaggagaaccagaccaggaacaagcacatcaaccccaacgagtggtggaaggtgtacccctccagcgtgaccgagttcaagttcctgttcgtgtccggccacttcaagggcaactacaaggcccagctgaccaggctgaaccacatcaccaactgcaacggcgccgtgctgtccgtggaggagctcctgatcggcggcgagatgatcaaggccggcaccctgaccctggaggaggtgaggaggaagttcaacaacggcgagatcaacttcgcggccgactgataa

SEQ ID NO: 92 - DNA, 2832 bp, Artificial sequence
  CTLA4_T03-RTALEN
atgggcgatcctaaaaagaaacgtaaggtcatcgataaggagaccgccgctgccaagttcgagagacagcacatggacagcatcgatatcgccgatctacgcacgctcggctacagccagcagcaacaggagaagatcaaaccgaaggttcgttcgacagtggcgcagcaccacgaggcactggtcggccacgggtttacacacgcgcacatcgttgcgttaagccaacacccggcagcgttagggaccgtcgctgtcaagtatcaggacatgatcgcagcgttgccagaggcgacacacgaagcgatcgttggcgtcggcaaacagtggtccggcgcacgcgctctggaggccttgctcacggtggcgggagagttgagaggtccaccgttacagttggacacaggccaacttctcaagattgcaaaacgtggcggcgtgaccgcagtggaggcagtgcatgcatggcgcaatgcactgacgggtgccccgctcaacttgaccccccagcaggtggtggccatcgccagcaataatggtggcaagcaggcgctggagacggtccagcggctgttgccggtgctgtgccaggcccacggcttgaccccccagcaggtggtggccatcgccagcaataatggtggcaagcaggcgctggagacggtccagcggctgttgccggtgctgtgccaggcccacggcttgaccccggagcaggtggtggccatcgccagccacgatggcggcaagcaggcgctggagacggtccagcggctgttgccggtgctgtgccaggcccacggcttgaccccggagcaggtggtggccatcgccagccacgatggcggcaagcaggcgctggagacggtccagcggctgttgccggtgctgtgccaggcccacggcttgaccccggagcaggtggtggccatcgccagcaatattggtggcaagcaggcgctggagacggtgcaggcgctgttgccggtgctgtgccaggcccacggcttgaccccccagcaggtggtggccatcgccagcaataatggtggcaagcaggcgctggagacggtccagcggctgttgccggtgctgtgccaggcccacggcttgaccccccagcaggtggtggccatcgccagcaatggcggtggcaagcaggcgctggagacggtccagcggctgttgccggtgctgtgccaggcccacggcttgaccccggagcaggtggtggccatcgccagcaatattggtggcaagcaggcgctggagacggtgcaggcgctgttgccggtgctgtgccaggcccacggcttgaccccggagcaggtggtggccatcgccagccacgatggcggcaagcaggcgctggagacggtccagcggctgttgccggtgctgtgccaggcccacggcttgaccccggagcaggtggtggccatcgccagccacgatggcggcaagcaggcgctggagacggtccagcggctgttgccggtgctgtgccaggcccacggcttgaccccggagcaggtggtggccatcgccagcaatattggtggcaagcaggcgctggagacggtgcaggcgctgttgccggtgctgtgccaggcccacggcttgaccccggagcaggtggtggccatcgccagccacgatggcggcaagcaggcgctggagacggtccagcggctgttgccggtgctgtgccaggcccacggcttgaccccggagcaggtggtggccatcgccagcaatattggtggcaagcaggcgctggagacggtgcaggcgctgttgccggtgctgtgccaggcccacggcttgaccccccagcaggtggtggccatcgccagcaataatggtggcaagcaggcgctggagacggtccagcggctgttgccggtgctgtgccaggcccacggcttgaccccggagcaggtggtggccatcgccagccacgatggcggcaagcaggcgctggagacggtccagcggctgttgccggtgctgtgccaggcccacggcttgacccctcagcaggtggtggccatcgccagcaatggcggcggcaggccggcgctggagagcattgttgcccagttatctcgccctgatccggcgttggccgcgttgaccaacgaccacctcgtcgccttggcctgcctcggcgggcgtcctgcgctggatgcagtgaaaaagggattgggggatcctatcagccgttcccagctggtgaagtccgagctggaggagaagaaatccgagttgaggcacaagctgaagtacgtgccccacgagtacatcgagctgatcgagatcgcccggaacagcacccaggaccgtatcctggagatgaaggtgatggagttcttcatgaaggtgtacggctacaggggcaagcacctgggcggctccaggaagcccgacggcgccatctacaccgtgggctcccccatcgactacggcgtgatcgtggacaccaaggcctactccggcggctacaacctgcccatcggccaggccgacgaaatgcagaggtacgtggaggagaaccagaccaggaacaagcacatcaaccccaacgagtggtggaaggtgtacccctccagcgtgaccgagttcaagttcctgttcgtgtccggccacttcaagggcaactacaaggcccagctgaccaggctgaaccacatcaccaactgcaacggcgccgtgctgtccgtggaggagctcctgatcggcggcgagatgatcaaggccggcaccctgaccctggaggaggtgaggaggaagttcaacaacggcgagatcaacttcgcggccgactgataa

SEQ ID NO: 93 - DNA, 2814 bp, Artificial sequence
  CTLA4_T04-L TALEN
atgggcgatcctaaaaagaaacgtaaggtcatcgattacccatacgatgttccagattacgctatcgatatcgccgatctacgcacgctcggctacagccagcagcaacaggagaagatcaaaccgaaggttcgttcgacagtggcgcagcaccacgaggcactggtcggccacgggtttacacacgcgcacatcgttgcgttaagccaacacccggcagcgttagggaccgtcgctgtcaagtatcaggacatgatcgcagcgttgccagaggcgacacacgaagcgatcgttggcgtcggcaaacagtggtccggcgcacgcgctctggaggccttgctcacggtggcgggagagttgagaggtccaccgttacagttggacacaggccaacttctcaagattgcaaaacgtggcggcgtgaccgcagtggaggcagtgcatgcatggcgcaatgcactgacgggtgccccgctcaacttgaccccggagcaggtggtggccatcgccagccacgatggcggcaagcaggcgctggagacggtccagcggctgttgccggtgctgtgccaggcccacggcttgaccccggagcaggtggtggccatcgccagccacgatggcggcaagcaggcgctggagacggtccagcggctgttgccggtgctgtgccaggcccacggcttgaccccggagcaggtggtggccatcgccagcaatattggtggcaagcaggcgctggagacggtgcaggcgctgttgccggtgctgtgccaggcccacggcttgaccccccagcaggtggtggccatcgccagcaatggcggtggcaagcaggcgctggagacggtccagcggctgttgccggtgctgtgccaggcccacggcttgaccccccagcaggtggtggccatcgccagcaataatggtggcaagcaggcgctggagacggtccagcggctgttgccggtgctgtgccaggcccacggcttgaccccggagcaggtggtggccatcgccagccacgatggcggcaagcaggcgctggagacggtccagcggctgttgccggtgctgtgccaggcccacggcttgaccccccagcaggtggtggccatcgccagcaatggcggtggcaagcaggcgctggagacggtccagcggctgttgccggtgctgtgccaggcccacggcttgaccccggagcaggtggtggccatcgccagcaatattggtggcaagcaggcgctggagacggtgcaggcgctgttgccggtgctgtgccaggcccacggcttgaccccccagcaggtggtggccatcgccagcaataatggtggcaagcaggcgctggagacggtccagcggctgttgccggtgctgtgccaggcccacggcttgaccccggagcaggtggtggccatcgccagccacgatggcggcaagcaggcgctggagacggtccagcggctgttgccggtgctgtgccaggcccacggcttgaccccggagcaggtggtggccatcgccagcaatattggtggcaagcaggcgctggagacggtgcaggcgctgttgccggtgctgtgccaggcccacggcttgaccccggagcaggtggtggccatcgccagcaatattggtggcaagcaggcgctggagacggtgcaggcgctgttgccggtgctgtgccaggcccacggcttgaccccccagcaggtggtggccatcgccagcaatggcggtggcaagcaggcgctggagacggtccagcggctgttgccggtgctgtgccaggcccacggcttgaccccccagcaggtggtggccatcgccagcaataatggtggcaagcaggcgctggagacggtccagcggctgttgccggtgctgtgccaggcccacggcttgaccccggagcaggtggtggccatcgccagccacgatggcggcaagcaggcgctggagacggtccagcggctgttgccggtgctgtgccaggcccacggcttgacccctcagcaggtggtggccatcgccagcaatggcggcggcaggccggcgctggagagcattgttgcccagttatctcgccctgatccggcgttggccgcgttgaccaacgaccacctcgtcgccttggcctgcctcggcgggcgtcctgcgctggatgcagtgaaaaagggattgggggatcctatcagccgttcccagctggtgaagtccgagctggaggagaagaaatccgagttgaggcacaagctgaagtacgtgccccacgagtacatcgagctgatcgagatcgcccggaacagcacccaggaccgtatcctggagatgaaggtgatggagttcttcatgaaggtgtacggctacaggggcaagcacctgggcggctccaggaagcccgacggcgccatctacaccgtgggctcccccatcgactacggcgtgatcgtggacaccaaggcctactccggcggctacaacctgcccatcggccaggccgacgaaatgcagaggtacgtggaggagaaccagaccaggaacaagcacatcaaccccaacgagtggtggaaggtgtacccctccagcgtgaccgagttcaagttcctgttcgtgtccggccacttcaagggcaactacaaggcccagctgaccaggctgaaccacatcaccaactgcaacggcgccgtgctgtccgtggaggagctcctgatcggcggcgagatgatcaaggccggcaccctgaccctggaggaggtgaggaggaagttcaacaacggcgagatcaacttcgcggccgactgataa

SEQ ID NO: 94 - DNA, 2832 bp, Artificial sequence
  CTLA4_T04-R TALEN
atgggcgatcctaaaaagaaacgtaaggtcatcgataaggagaccgccgctgccaagttcgagagacagcacatggacagcatcgatatcgccgatctacgcacgctcggctacagccagcagcaacaggagaagatcaaaccgaaggttcgttcgacagtggcgcagcaccacgaggcactggtcggccacgggtttacacacgcgcacatcgttgcgttaagccaacacccggcagcgttagggaccgtcgctgtcaagtatcaggacatgatcgcagcgttgccagaggcgacacacgaagcgatcgttggcgtcggcaaacagtggtccggcgcacgcgctctggaggccttgctcacggtggcgggagagttgagaggtccaccgttacagttggacacaggccaacttctcaagattgcaaaacgtggcggcgtgaccgcagtggaggcagtgcatgcatggcgcaatgcactgacgggtgccccgctcaacttgaccccccagcaggtggtggccatcgccagcaataatggtggcaagcaggcgctggagacggtccagcggctgttgccggtgctgtgccaggcccacggcttgaccccggagcaggtggtggccatcgccagccacgatggcggcaagcaggcgctggagacggtccagcggctgttgccggtgctgtgccaggcccacggcttgaccccccagcaggtggtggccatcgccagcaatggcggtggcaagcaggcgctggagacggtccagcggctgttgccggtgctgtgccaggcccacggcttgaccccccagcaggtggtggccatcgccagcaataatggtggcaagcaggcgctggagacggtccagcggctgttgccggtgctgtgccaggcccacggcttgaccccccagcaggtggtggccatcgccagcaataatggtggcaagcaggcgctggagacggtccagcggctgttgccggtgctgtgccaggcccacggcttgaccccggagcaggtggtggccatcgccagccacgatggcggcaagcaggcgctggagacggtccagcggctgttgccggtgctgtgccaggcccacggcttgaccccggagcaggtggtggccatcgccagccacgatggcggcaagcaggcgctggagacggtccagcggctgttgccggtgctgtgccaggcccacggcttgaccccggagcaggtggtggccatcgccagcaatattggtggcaagcaggcgctggagacggtgcaggcgctgttgccggtgctgtgccaggcccacggcttgaccccccagcaggtggtggccatcgccagcaataatggtggcaagcaggcgctggagacggtccagcggctgttgccggtgctgtgccaggcccacggcttgaccccccagcaggtggtggccatcgccagcaatggcggtggcaagcaggcgctggagacggtccagcggctgttgccggtgctgtgccaggcccacggcttgaccccggagcaggtggtggccatcgccagcaatattggtggcaagcaggcgctggagacggtgcaggcgctgttgccggtgctgtgccaggcccacggcttgaccccggagcaggtggtggccatcgccagccacgatggcggcaagcaggcgctggagacggtccagcggctgttgccggtgctgtgccaggcccacggcttgaccccggagcaggtggtggccatcgccagccacgatggcggcaagcaggcgctggagacggtccagcggctgttgccggtgctgtgccaggcccacggcttgaccccggagcaggtggtggccatcgccagcaatattggtggcaagcaggcgctggagacggtgcaggcgctgttgccggtgctgtgccaggcccacggcttgaccccggagcaggtggtggccatcgccagccacgatggcggcaagcaggcgctggagacggtccagcggctgttgccggtgctgtgccaggcccacggcttgacccctcagcaggtggtggccatcgccagcaatggcggcggcaggccggcgctggagagcattgttgcccagttatctcgccctgatccggcgttggccgcgttgaccaacgaccacctcgtcgccttggcctgcctcggcgggcgtcctgcgctggatgcagtgaaaaagggattgggggatcctatcagccgttcccagctggtgaagtccgagctggaggagaagaaatccgagttgaggcacaagctgaagtacgtgccccacgagtacatcgagctgatcgagatcgcccggaacagcacccaggaccgtatcctggagatgaaggtgatggagttcttcatgaaggtgtacggctacaggggcaagcacctgggcggctccaggaagcccgacggcgccatctacaccgtgggctcccccatcgactacggcgtgatcgtggacaccaaggcctactccggcggctacaacctgcccatcggccaggccgacgaaatgcagaggtacgtggaggagaaccagaccaggaacaagcacatcaaccccaacgagtggtggaaggtgtacccctccagcgtgaccgagttcaagttcctgttcgtgtccggccacttcaagggcaactacaaggcccagctgaccaggctgaaccacatcaccaactgcaacggcgccgtgctgtccgtggaggagctcctgatcggcggcgagatgatcaaggccggcaccctgaccctggaggaggtgaggaggaagttcaacaacggcgagatcaacttcgcggccgactgataa

SEQ ID NO: 95 - DNA, 2814 bp, Artificial sequence
  PDCD1_T01-L TALEN
atgggcgatcctaaaaagaaacgtaaggtcatcgattacccatacgatgttccagattacgctatcgatatcgccgatctacgcacgctcggctacagccagcagcaacaggagaagatcaaaccgaaggttcgttcgacagtggcgcagcaccacgaggcactggtcggccacgggtttacacacgcgcacatcgttgcgttaagccaacacccggcagcgttagggaccgtcgctgtcaagtatcaggacatgatcgcagcgttgccagaggcgacacacgaagcgatcgttggcgtcggcaaacagtggtccggcgcacgcgctctggaggccttgctcacggtggcgggagagttgagaggtccaccgttacagttggacacaggccaacttctcaagattgcaaaacgtggcggcgtgaccgcagtggaggcagtgcatgcatggcgcaatgcactgacgggtgccccgctcaacttgaccccccagcaggtggtggccatcgccagcaatggcggtggcaagcaggcgctggagacggtccagcggctgttgccggtgctgtgccaggcccacggcttgaccccggagcaggtggtggccatcgccagccacgatggcggcaagcaggcgctggagacggtccagcggctgttgccggtgctgtgccaggcccacggcttgaccccccagcaggtggtggccatcgccagcaatggcggtggcaagcaggcgctggagacggtccagcggctgttgccggtgctgtgccaggcccacggcttgaccccggagcaggtggtggccatcgccagccacgatggcggcaagcaggcgctggagacggtccagcggctgttgccggtgctgtgccaggcccacggcttgaccccggagcaggtggtggccatcgccagccacgatggcggcaagcaggcgctggagacggtccagcggctgttgccggtgctgtgccaggcccacggcttgaccccggagcaggtggtggccatcgccagccacgatggcggcaagcaggcgctggagacggtccagcggctgttgccggtgctgtgccaggcccacggcttgaccccggagcaggtggtggccatcgccagccacgatggcggcaagcaggcgctggagacggtccagcggctgttgccggtgctgtgccaggcccacggcttgaccccggagcaggtggtggccatcgccagcaatattggtggcaagcaggcgctggagacggtgcaggcgctgttgccggtgctgtgccaggcccacggcttgaccccccagcaggtggtggccatcgccagcaataatggtggcaagcaggcgctggagacggtccagcggctgttgccggtgctgtgccaggcccacggcttgaccccggagcaggtggtggccatcgccagccacgatggcggcaagcaggcgctggagacggtccagcggctgttgccggtgctgtgccaggcccacggcttgaccccggagcaggtggtggccatcgccagccacgatggcggcaagcaggcgctggagacggtccagcggctgttgccggtgctgtgccaggcccacggcttgaccccggagcaggtggtggccatcgccagccacgatggcggcaagcaggcgctggagacggtccagcggctgttgccggtgctgtgccaggcccacggcttgaccccccagcaggtggtggccatcgccagcaatggcggtggcaagcaggcgctggagacggtccagcggctgttgccggtgctgtgccaggcccacggcttgaccccccagcaggtggtggccatcgccagcaataatggtggcaagcaggcgctggagacggtccagcggctgttgccggtgctgtgccaggcccacggcttgaccccggagcaggtggtggccatcgccagccacgatggcggcaagcaggcgctggagacggtccagcggctgttgccggtgctgtgccaggcccacggcttgacccctcagcaggtggtggccatcgccagcaatggcggcggcaggccggcgctggagagcattgttgcccagttatctcgccctgatccggcgttggccgcgttgaccaacgaccacctcgtcgccttggcctgcctcggcgggcgtcctgcgctggatgcagtgaaaaagggattgggggatcctatcagccgttcccagctggtgaagtccgagctggaggagaagaaatccgagttgaggcacaagctgaagtacgtgccccacgagtacatcgagctgatcgagatcgcccggaacagcacccaggaccgtatcctggagatgaaggtgatggagttcttcatgaaggtgtacggctacaggggcaagcacctgggcggctccaggaagcccgacggcgccatctacaccgtgggctcccccatcgactacggcgtgatcgtggacaccaaggcctactccggcggctacaacctgcccatcggccaggccgacgaaatgcagaggtacgtggaggagaaccagaccaggaacaagcacatcaaccccaacgagtggtggaaggtgtacccctccagcgtgaccgagttcaagttcctgttcgtgtccggccacttcaagggcaactacaaggcccagctgaccaggctgaaccacatcaccaactgcaacggcgccgtgctgtccgtggaggagctcctgatcggcggcgagatgatcaaggccggcaccctgaccctggaggaggtgaggaggaagttcaacaacggcgagatcaacttcgcggccgactgataa

SEQ ID NO: 96 - DNA, 2829 bp, Artificial sequence
  PDCD1_T01-R TALEN
atgggcgatcctaaaaagaaacgtaaggtcatcgataaggagaccgccgctgccaagttcgagagacagcacatggacagcatcgatatcgccgatctacgcacgctcggctacagccagcagcaacaggagaagatcaaaccgaaggttcgttcgacagtggcgcagcaccacgaggcactggtcggccacgggtttacacacgcgcacatcgttgcgttaagccaacacccggcagcgttagggaccgtcgctgtcaagtatcaggacatgatcgcagcgttgccagaggcgacacacgaagcgatcgttggcgtcggcaaacagtggtccggcgcacgcgctctggaggccttgctcacggtggcgggagagttgagaggtccaccgttacagttggacacaggccaacttctcaagattgcaaaacgtggcggcgtgaccgcagtggaggcagtgcatgcatggcgcaatgcactgacgggtgccccgctcaacttgaccccccagcaagtcgtcgcaatcgccagcaataacggagggaagcaagccctcgaaaccgtgcagcggttgcttcctgtgctctgccaggcccacggccttacccctgagcaggtggtggccatcgcaagtaacattggaggaaagcaagccttggagacagtgcaggccctgttgcccgtgctgtgccaggcacacggcctcacaccagagcaggtcgtggccattgcctccaacatcggggggaaacaggctctggagaccgtccaggccctgctgcccgtcctctgtcaagctcacggcctgactccccaacaagtggtcgccatcgcctctaataacggcgggaagcaggcactggaaacagtgcagagactgctccctgtgctttgccaagctcatgggttgaccccccaacaggtcgtcgctattgcctcaaacaacgggggcaagcaggcccttgagactgtgcagaggctgttgccagtgctgtgtcaggctcacgggctcactccacaacaggtggtcgcaattgccagcaacggcggcggaaagcaagctcttgaaaccgtgcaacgcctcctgcccgtgctctgtcaggctcatggcctgacaccacaacaagtcgtggccatcgccagtaataatggcgggaaacaggctcttgagaccgtccagaggctgctcccagtgctctgccaggcacacgggctgaccccccagcaggtggtggctatcgccagcaataatgggggcaagcaggccctggaaacagtccagcgcctgctgccagtgctttgccaggctcacgggctcactcccgaacaggtcgtggcaatcgcctccaacggagggaagcaggctctggagaccgtgcagagactgctgcccgtcttgtgccaggcccacggactcacacctcagcaggtcgtcgccattgcctctaacaacgggggcaaacaagccctggagacagtgcagcggctgttgcctgtgttgtgccaagcccacggcttgactcctcaacaagtggtcgccatcgcctcaaatggcggcggaaaacaagctctggagacagtgcagaggttgctgcccgtcctctgccaagcccacggcctgactccccaacaggtcgtcgccattgccagcaacggcggaggaaagcaggctctcgaaactgtgcagcggctgcttcctgtgctgtgtcaggctcatgggctgaccccccagcaagtggtggctattgcctctaacaatggaggcaagcaagcccttgagacagtccagaggctgttgccagtgctgtgccaggcccacgggctcacaccccagcaggtggtcgccatcgccagtaacggcgggggcaaacaggcattggaaaccgtccagcgcctgcttccagtgctctgccaggcacacggactgacacccgaacaggtggtggccattgcatcccatgatgggggcaagcaggccctggagaccgtgcagagactcctgccagtgttgtgccaagctcacggcctcacccctcagcaagtcgtggccatcgcctcaaacggggggggccggcctgcactggagagcattgttgcccagttatctcgccctgatccggcgttggccgcgttgaccaacgaccacctcgtcgccttggcctgcctcggcgggcgtcctgcgctggatgcagtgaaaaagggattgggggatcctatcagccgttcccagctggtgaagtccgagctggaggagaagaaatccgagttgaggcacaagctgaagtacgtgccccacgagtacatcgagctgatcgagatcgcccggaacagcacccaggaccgtatcctggagatgaaggtgatggagttcttcatgaaggtgtacggctacaggggcaagcacctgggcggctccaggaagcccgacggcgccatctacaccgtgggctcccccatcgactacggcgtgatcgtggacaccaaggcctactccggcggctacaacctgcccatcggccaggccgacgaaatgcagaggtacgtggaggagaaccagaccaggaacaagcacatcaaccccaacgagtggtggaaggtgtacccctccagcgtgaccgagttcaagttcctgttcgtgtccggccacttcaagggcaactacaaggcccagctgaccaggctgaaccacatcaccaactgcaacggcgccgtgctgtccgtggaggagctcctgatcggcggcgagatgatcaaggccggcaccctgaccctggaggaggtgaggaggaagttcaacaacggcgagatcaacttcgcggccgactgataa

SEQ ID NO: 97 - DNA, 2814 bp, Artificial sequence
  PDCD1_T03-L TALEN
atgggcgatcctaaaaagaaacgtaaggtcatcgattacccatacgatgttccagattacgctatcgatatcgccgatctacgcacgctcggctacagccagcagcaacaggagaagatcaaaccgaaggttcgttcgacagtggcgcagcaccacgaggcactggtcggccacgggtttacacacgcgcacatcgttgcgttaagccaacacccggcagcgttagggaccgtcgctgtcaagtatcaggacatgatcgcagcgttgccagaggcgacacacgaagcgatcgttggcgtcggcaaacagtggtccggcgcacgcgctctggaggccttgctcacggtggcgggagagttgagaggtccaccgttacagttggacacaggccaacttctcaagattgcaaaacgtggcggcgtgaccgcagtggaggcagtgcatgcatggcgcaatgcactgacgggtgccccgctcaacttgaccccggagcaggtggtggccatcgccagcaatattggtggcaagcaggcgctggagacggtgcaggcgctgttgccggtgctgtgccaggcccacggcttgaccccggagcaggtggtggccatcgccagccacgatggcggcaagcaggcgctggagacggtccagcggctgttgccggtgctgtgccaggcccacggcttgaccccggagcaggtggtggccatcgccagccacgatggcggcaagcaggcgctggagacggtccagcggctgttgccggtgctgtgccaggcccacggcttgaccccccagcaggtggtggccatcgccagcaatggcggtggcaagcaggcgctggagacggtccagcggctgttgccggtgctgtgccaggcccacggcttgaccccggagcaggtggtggccatcgccagccacgatggcggcaagcaggcgctggagacggtccagcggctgttgccggtgctgtgccaggcccacggcttgaccccccagcaggtggtggccatcgccagcaatggcggtggcaagcaggcgctggagacggtccagcggctgttgccggtgctgtgccaggcccacggcttgaccccccagcaggtggtggccatcgccagcaataatggtggcaagcaggcgctggagacggtccagcggctgttgccggtgctgtgccaggcccacggcttgaccccccagcaggtggtggccatcgccagcaatggcggtggcaagcaggcgctggagacggtccagcggctgttgccggtgctgtgccaggcccacggcttgaccccccagcaggtggtggccatcgccagcaataatggtggcaagcaggcgctggagacggtccagcggctgttgccggtgctgtgccaggcccacggcttgaccccccagcaggtggtggccatcgccagcaataatggtggcaagcaggcgctggagacggtccagcggctgttgccggtgctgtgccaggcccacggcttgaccccccagcaggtggtggccatcgccagcaataatggtggcaagcaggcgctggagacggtccagcggctgttgccggtgctgtgccaggcccacggcttgaccccccagcaggtggtggccatcgccagcaataatggtggcaagcaggcgctggagacggtccagcggctgttgccggtgctgtgccaggcccacggcttgaccccggagcaggtggtggccatcgccagccacgatggcggcaagcaggcgctggagacggtccagcggctgttgccggtgctgtgccaggcccacggcttgaccccggagcaggtggtggccatcgccagccacgatggcggcaagcaggcgctggagacggtccagcggctgttgccggtgctgtgccaggcccacggcttgaccccggagcaggtggtggccatcgccagcaatattggtggcaagcaggcgctggagacggtgcaggcgctgttgccggtgctgtgccaggcccacggcttgacccctcagcaggtggtggccatcgccagcaatggcggcggcaggccggcgctggagagcattgttgcccagttatctcgccctgatccggcgttggccgcgttgaccaacgaccacctcgtcgccttggcctgcctcggcgggcgtcctgcgctggatgcagtgaaaaagggattgggggatcctatcagccgttcccagctggtgaagtccgagctggaggagaagaaatccgagttgaggcacaagctgaagtacgtgccccacgagtacatcgagctgatcgagatcgcccggaacagcacccaggaccgtatcctggagatgaaggtgatggagttcttcatgaaggtgtacggctacaggggcaagcacctgggcggctccaggaagcccgacggcgccatctacaccgtgggctcccccatcgactacggcgtgatcgtggacaccaaggcctactccggcggctacaacctgcccatcggccaggccgacgaaatgcagaggtacgtggaggagaaccagaccaggaacaagcacatcaaccccaacgagtggtggaaggtgtacccctccagcgtgaccgagttcaagttcctgttcgtgtccggccacttcaagggcaactacaaggcccagctgaccaggctgaaccacatcaccaactgcaacggcgccgtgctgtccgtggaggagctcctgatcggcggcgagatgatcaaggccggcaccctgaccctggaggaggtgaggaggaagttcaacaacggcgagatcaacttcgcggccgactgataa

SEQ ID NO: 98 - DNA, 2829 bp, Artificial sequence
  PDCD1_T03-R TALEN
atgggcgatcctaaaaagaaacgtaaggtcatcgataaggagaccgccgctgccaagttcgagagacagcacatggacagcatcgatatcgccgatctacgcacgctcggctacagccagcagcaacaggagaagatcaaaccgaaggttcgttcgacagtggcgcagcaccacgaggcactggtcggccacgggtttacacacgcgcacatcgttgcgttaagccaacacccggcagcgttagggaccgtcgctgtcaagtatcaggacatgatcgcagcgttgccagaggcgacacacgaagcgatcgttggcgtcggcaaacagtggtccggcgcacgcgctctggaggccttgctcacggtggcgggagagttgagaggtccaccgttacagttggacacaggccaacttctcaagattgcaaaacgtggcggcgtgaccgcagtggaggcagtgcatgcatggcgcaatgcactgacgggtgccccgctcaacttgacccccgagcaagtcgtcgcaatcgccagccatgatggagggaagcaagccctcgaaaccgtgcagcggttgcttcctgtgctctgccaggcccacggccttacccctcagcaggtggtggccatcgcaagtaacggaggaggaaagcaagccttggagacagtgcagcgcctgttgcccgtgctgtgccaggcacacggcctcacaccagagcaggtcgtggccattgcctcccatgacggggggaaacaggctctggagaccgtccagaggctgctgcccgtcctctgtcaagctcacggcctgactccccaacaagtggtcgccatcgcctctaatggcggcgggaagcaggcactggaaacagtgcagagactgctccctgtgctttgccaagctcatgggttgaccccccaacaggtcgtcgctattgcctcaaacggggggggcaagcaggcccttgagactgtgcagaggctgttgccagtgctgtgtcaggctcacgggctcactccacaacaggtggtcgcaattgccagcaacggcggcggaaagcaagctcttgaaaccgtgcaacgcctcctgcccgtgctctgtcaggctcatggcctgacaccacaacaagtcgtggccatcgccagtaataatggcgggaaacaggctcttgagaccgtccagaggctgctcccagtgctctgccaggcacacgggctgacccccgagcaggtggtggctatcgccagcaatattgggggcaagcaggccctggaaacagtccaggccctgctgccagtgctttgccaggctcacgggctcactccccagcaggtcgtggcaatcgcctccaacggcggagggaagcaggctctggagaccgtgcagagactgctgcccgtcttgtgccaggcccacggactcacacctgaacaggtcgtcgccattgcctctcacgatgggggcaaacaagccctggagacagtgcagcggctgttgcctgtgttgtgccaagcccacggcttgactcctcaacaagtggtcgccatcgcctcaaatggcggcggaaaacaagctctggagacagtgcagaggttgctgcccgtcctctgccaagcccacggcctgactccccaacaggtcgtcgccattgccagcaacaacggaggaaagcaggctctcgaaactgtgcagcggctgcttcctgtgctgtgtcaggctcatgggctgacccccgagcaagtggtggctattgcctctaatggaggcaagcaagcccttgagacagtccagaggctgttgccagtgctgtgccaggcccacgggctcacaccccagcaggtggtcgccatcgccagtaacaacgggggcaaacaggcattggaaaccgtccagcgcctgcttccagtgctctgccaggcacacggactgacacccgaacaggtggtggccattgcatcccatgatgggggcaagcaggccctggagaccgtgcagagactcctgccagtgttgtgccaagctcacggcctcacccctcagcaagtcgtggccatcgcctcaaacggggggggccggcctgcactggagagcattgttgcccagttatctcgccctgatccggcgttggccgcgttgaccaacgaccacctcgtcgccttggcctgcctcggcgggcgtcctgcgctggatgcagtgaaaaagggattgggggatcctatcagccgttcccagctggtgaagtccgagctggaggagaagaaatccgagttgaggcacaagctgaagtacgtgccccacgagtacatcgagctgatcgagatcgcccggaacagcacccaggaccgtatcctggagatgaaggtgatggagttcttcatgaaggtgtacggctacaggggcaagcacctgggcggctccaggaagcccgacggcgccatctacaccgtgggctcccccatcgactacggcgtgatcgtggacaccaaggcctactccggcggctacaacctgcccatcggccaggccgacgaaatgcagaggtacgtggaggagaaccagaccaggaacaagcacatcaaccccaacgagtggtggaaggtgtacccctccagcgtgaccgagttcaagttcctgttcgtgtccggccacttcaagggcaactacaaggcccagctgaccaggctgaaccacatcaccaactgcaacggcgccgtgctgtccgtggaggagctcctgatcggcggcgagatgatcaaggccggcaccctgaccctggaggaggtgaggaggaagttcaacaacggcgagatcaacttcgcggccgactgataa

SEQ ID NO: 99 - DNA, 60 bp, Artificial sequence
  Forward primer CTLA4_T01
  misc_feature (31); (32); (33); (34); (35); (36); (37); (38); (39); (40): n is a or c or t or g
ccatctcatccctgcgtgtctccgactcagnnnnnnnnnnctctacttcctgaagacctg

SEQ ID NO: 100 - DNA, 60 bp, Artificial sequence
  Forward primer CTLA4_T03/T04
  misc_feature (31); (32); (33); (34); (35); (36); (37); (38); (39); (40): n is a or c or t or g
ccatctcatccctgcgtgtctccgactcagnnnnnnnnnnacagttgagagatggagggg

SEQ ID NO: 101 - DNA, 59 bp, Artificial sequence
  Forward primer PDCD1_T01
  misc_feature (31); (32); (33); (34); (35); (36); (37); (38); (39); (40): n is a or c or t or g
ccatctcatccctgcgtgtctccgactcagnnnnnnnnnnccacagaggtaggtgccgc

SEQ ID NO: 102 - DNA, 60 bp, Artificial sequence
  Forward primer PDCD1_T03
  misc_feature (31); (32); (33); (34); (35); (36); (37); (38); (39); (40): n is a or c or t or g
ccatctcatccctgcgtgtctccgactcagnnnnnnnnnngacagagatgccggtcacca

SEQ ID NO: 103 - DNA, 50 bp, Artificial sequence
  Reverse primer CTLA4_T01
cctatcccctgtgtgccttggcagtctcagtggaatacagagccagccaa

SEQ ID NO: 104 - DNA, 50 bp, Artificial sequence
  Reverse primer CTLA4_T03/04
cctatcccctgtgtgccttggcagtctcagggtgcccgtgcagatggaat

SEQ ID NO: 105 - DNA, 50 bp, Artificial sequence
  Reverse primer PDCD1_T01
cctatcccctgtgtgccttggcagtctcagggctctgcagtggaggccag

SEQ ID NO: 106 - DNA, 50 bp, Artificial sequence
  Reverse primer PDCD1_T03
cctatcccctgtgtgccttggcagtctcagggacaacgccaccttcacct

SEQ ID NO: 107 - protein, 281 aa, Artificialsequence
  pTalpha-FL
MAGTWLLLLLALGCPALPTGVGGTPFPSLAPPIMLLVDGKQQMVVVCLVLDVAPPGLDSPIWFSAGNGSALDAFTYGPSPATDGTWTNLAHLSLPSEELASWEPLVCHTGPGAEGHSRSTQPMHLSGEASTARTCPQEPLRGTPGGALWLGVLRLLLFKLLLFDLLLTCSCLCDPAGPLPSPATTTRLRALGSHRLHPATETGGREATSSPRPQPRDRRWGDTPPGRKPGSPVWGEGSYLSSYPTCPAQAWCSRSRLRAPSSSLGAFFRGDLPPPLQAGAA

SEQ ID NO: 108 - protein, 263 aa, Artificialsequence
  pTalpha-Delta18
MAGTWLLLLLALGCPALPTGVGGTPFPSLAPPIMLLVDGKQQMVVVCLVLDVAPPGLDSPIWFSAGNGSALDAFTYGPSPATDGTWTNLAHLSLPSEELASWEPLVCHTGPGAEGHSRSTQPMHLSGEASTARTCPQEPLRGTPGGALWLGVLRLLLFKLLLFDLLLTCSCLCDPAGPLPSPATTTRLRALGSHRLHPATETGGREATSSPRPQPRDRRWGDTPPGRKPGSPVWGEGSYLSSYPTCPAQAWCSRSRLRAPSSS

SEQ ID NO: 109 - protein, 233 aa, Artificialsequence
  pTalpha-Delta48
MAGTWLLLLLALGCPALPTGVGGTPFPSLAPPIMLLVDGKQQMVVVCLVLDVAPPGLDSPIWFSAGNGSALDAFTYGPSPATDGTWTNLAHLSLPSEELASWEPLVCHTGPGAEGHSRSTQPMHLSGEASTARTCPQEPLRGTPGGALWLGVLRLLLFKLLLFDLLLTCSCLCDPAGPLPSPATTTRLRALGSHRLHPATETGGREATSSPRPQPRDRRWGDTPPGRKPGSPV

SEQ ID NO: 110 - protein, 219 aa, Artificialsequence
  pTalpha-Delta62
MAGTWLLLLLALGCPALPTGVGGTPFPSLAPPIMLLVDGKQQMVVVCLVLDVAPPGLDSPIWFSAGNGSALDAFTYGPSPATDGTWTNLAHLSLPSEELASWEPLVCHTGPGAEGHSRSTQPMHLSGEASTARTCPQEPLRGTPGGALWLGVLRLLLFKLLLFDLLLTCSCLCDPAGPLPSPATTTRLRALGSHRLHPATETGGREATSSPRPQPRDRR

SEQ ID NO: 111 - protein, 203 aa, Artificialsequence
  pTalpha-Delta78
MAGTWLLLLLALGCPALPTGVGGTPFPSLAPPIMLLVDGKQQMVVVCLVLDVAPPGLDSPIWFSAGNGSALDAFTYGPSPATDGTWTNLAHLSLPSEELASWEPLVCHTGPGAEGHSRSTQPMHLSGEASTARTCPQEPLRGTPGGALWLGVLRLLLFKLLLFDLLLTCSCLCDPAGPLPSPATTTRLRALGSHRLHPATETG

SEQ ID NO: 112 - protein, 189 aa, Artificialsequence
  pTalpha-Delta92
MAGTWLLLLLALGCPALPTGVGGTPFPSLAPPIMLLVDGKQQMVVVCLVLDVAPPGLDSPIWFSAGNGSALDAFTYGPSPATDGTWTNLAHLSLPSEELASWEPLVCHTGPGAEGHSRSTQPMHLSGEASTARTCPQEPLRGTPGGALWLGVLRLLLFKLLLFDLLLTCSCLCDPAGPLPSPATTTRLR

SEQ ID NO: 113 - protein, 171 aa, Artificialsequence
  pTalpha-Delta110
MAGTWLLLLLALGCPALPTGVGGTPFPSLAPPIMLLVDGKQQMVVVCLVLDVAPPGLDSPIWFSAGNGSALDAFTYGPSPATDGTWTNLAHLSLPSEELASWEPLVCHTGPGAEGHSRSTQPMHLSGEASTARTCPQEPLRGTPGGALWLGVLRLLLFKLLLFDLLLTCSC

SEQ ID NO: 114 - protein, 167 aa, Artificialsequence
  pTalpha-Delta114
MAGTWLLLLLALGCPALPTGVGGTPFPSLAPPIMLLVDGKQQMVVVCLVLDVAPPGLDSPIWFSAGNGSALDAFTYGPSPATDGTWTNLAHLSLPSEELASWEPLVCHTGPGAEGHSRSTQPMHLSGEASTARTCPQEPLRGTPGGALWLGVLRLLLFKLLLFDLLL

SEQ ID NO: 115 - protein, 344 aa, Artificialsequence [sequence omitted]

SEQ ID NO: 116 - protein, 311 aa, Artificialsequence
  pTalpha-FL-CD8
MAGTWLLLLLALGCPALPTGVGGTPFPSLAPPIMLLVDGKQQMVVVCLVLDVAPPGLDSPIWFSAGNGSALDAFTYGPSPATDGTWTNLAHLSLPSEELASWEPLVCHTGPGAEGHSRSTQPMHLSGEASTARTCPQEPLRGTPGGALWLGVLRLLLFKLLLFDLLLTCSCLCDPAGPLPSPATTTRLRALGSHRLHPATETGGREATSSPRPQPRDRRWGDTPPGRKPGSPVWGEGSYLSSYPTCPAQAWCSRSRLRAPSSSLGAFFRGDLPPPLQAGAAASHRNRRRVCKCPRPVVKSGDKPSLSARYV

SEQ ID NO: 117 - protein, 325 aa, Artificialsequence
  pTalpha-FL-41BB
MAGTWLLLLLALGCPALPTGVGGTPFPSLAPPIMLLVDGKQQMVVVCLVLDVAPPGLDSPIWFSAGNGSALDAFTYGPSPATDGTWTNLAHLSLPSEELASWEPLVCHTGPGAEGHSRSTQPMHLSGEASTARTCPQEPLRGTPGGALWLGVLRLLLFKLLLFDLLLTCSCLCDPAGPLPSPATTTRLRALGSHRLHPATETGGREATSSPRPQPRDRRWGDTPPGRKPGSPVWGEGSYLSSYPTCPAQAWCSRSRLRAPSSSLGAFFRGDLPPPLQAGAAGSKRGRKKLLYIFKQPFMRPVQTTQEEDGCSCRFPEEEEGGCEL

SEQ ID NO: 118 - protein, 296 aa, Artificialsequence
  pTalpha-Delta48-CD28
MAGTWLLLLLALGCPALPTGVGGTPFPSLAPPIMLLVDGKQQMVVVCLVLDVAPPGLDSPIWFSAGNGSALDAFTYGPSPATDGTWTNLAHLSLPSEELASWEPLVCHTGPGAEGHSRSTQPMHLSGEASTARTCPQEPLRGTPGGALWLGVLRLLLFKLLLFDLLLTCSCLCDPAGPLPSPATTTRLRALGSHRLHPATETGGREATSSPRPQPRDRRWGDTPPGRKPGSPVASGGVLACYSLLVTVAFIIFWVRSKRSRGGHSDYMNMTPRRPGPTRKHYQPYAPPRDFAAYRS

SEQ ID NO: 119 - protein, 263 aa, Artificialsequence
  pTalpha-Delta48-CD8
MAGTWLLLLLALGCPALPTGVGGTPFPSLAPPIMLLVDGKQQMVVVCLVLDVAPPGLDSPIWFSAGNGSALDAFTYGPSPATDGTWTNLAHLSLPSEELASWEPLVCHTGPGAEGHSRSTQPMHLSGEASTARTCPQEPLRGTPGGALWLGVLRLLLFKLLLFDLLLTCSCLCDPAGPLPSPATTTRLRALGSHRLHPATETGGREATSSPRPQPRDRRWGDTPPGRKPGSPVASHRNRRRVCKCPRPVVKSGDKPSLSARYV

SEQ ID NO: 120 - protein, 277 aa, Artificialsequence
  pTalpha-Delta48-41BB
MAGTWLLLLLALGCPALPTGVGGTPFPSLAPPIMLLVDGKQQMVVVCLVLDVAPPGLDSPIWFSAGNGSALDAFTYGPSPATDGTWTNLAHLSLPSEELASWEPLVCHTGPGAEGHSRSTQPMHLSGEASTARTCPQEPLRGTPGGALWLGVLRLLLFKLLLFDLLLTCSCLCDPAGPLPSPATTTRLRALGSHRLHPATETGGREATSSPRPQPRDRRWGDTPPGRKPGSPVGSKRGRKKLLYIFKQPFMRPVQTTQEEDGCSCRFPEEEEGGCEL

SEQ ID NO: 121 - protein, 172 aa, Artificialsequence
  pTalpha-Delta114-TCRalpha.IC
MAGTWLLLLLALGCPALPTGVGGTPFPSLAPPIMLLVDGKQQMVVVCLVLDVAPPGLDSPIWFSAGNGSALDAFTYGPSPATDGTWTNLAHLSLPSEELASWEPLVCHTGPGAEGHSRSTQPMHLSGEASTARTCPQEPLRGTPGGALWLGVLRLLLFKLLLFDLLLRLWSS

SEQ ID NO: 122 - protein, 173 aa, Artificialsequence
  pTalpha.EC-TCRalpha. TM. IC
MAGTWLLLLLALGCPALPTGVGGTPFPSLAPPIMLLVDGKQQMVVVCLVLDVAPPGLDSPIWFSAGNGSALDAFTYGPSPATDGTWTNLAHLSLPSEELASWEPLVCHTGPGAEGHSRSTQPMHLSGEASTARTCPQEPLRGTPGGLSVIGFRILLLKVAGFNLLMTLRLWSS

SEQ ID NO: 123 - protein, 233 aa, Artificialsequence
  pTalpha.EC-Delta48-1xMUT
MAGTWLLLLLALGCPALPTGVGGTPFPSLAPPIMLLVDGKQQMVVVCLVLDVAPPGLDSPIRFSAGNGSALDAFTYGPSPATDGTWTNLAHLSLPSEELASWEPLVCHTGPGAEGHSRSTQPMHLSGEASTARTCPQEPLRGTPGGALWLGVLRLLLFKLLLFDLLLTCSCLCDPAGPLPSPATTTRLRALGSHRLHPATETGGREATSSPRPQPRDRRWGDTPPGRKPGSPV

SEQ ID NO: 124 - protein, 233 aa, Artificialsequence
  pTalpha.EC-Delta48-4xMUT
MAGTWLLLLLALGCPALPTGVGGTPFPSLAPPIMLLVAGAQQMVVVCLVLDVAPPGLDSPIWFSAGNGSALDAFTYGPSPATDGTWTNLAHLSLPSEELASWEPLVCHTGPGAEGHSASTQPMHLSGEASTAATCPQEPLRGTPGGALWLGVLRLLLFKLLLFDLLLTCSCLCDPAGPLPSPATTTRLRALGSHRLHPATETGGREATSSPRPQPRDRRWGDTPPGRKPGSPV

SEQ ID NO: 125 - protein, 848 aa, Artificialsequence
  Multi-chain CAR
MAPAMESPTLLCVALLFFAPDGVLAEVQLQQSGPELIKPGASVKMSCKASGYTFTSYVMHWVKQKPGQGLEWIGYINPYNDGTKYNEKFKGKATLTSDKSSSTAYMELSSLTSEDSAVYYCARGTYYYGSRVFDYWGQGTTLTVSSGGGGSGGGGSGGGGSDIVMTQAAPSIPVTPGESVSISCRSSKSLLNSNGNTYLYWFLQRPGQSPQLLIYRMSNLASGVPDRFSGSGSGTAFTLRISRVEAEDVGVYYCMQHLEYPFTFGAGTKLELKRADTTTPAPRPPTPAPTIASQPLSLRPEACRPAAGGAVHTRGLDFACDFFIPLLVVILFAVDTGLFISTQQQVTFLLKIKRTRKGFRLLNPHPKPNPKNNRAEGRGSLLTCGDVEENPGPMDTESNRRANLALPQEPSSVPAFEVLEISPQEVSSGRLLKSASSPPLHTWLTVLKKEQEFLGVTQILTAMICLCFGTVVCSVLDISHIEGDIFSSFKAGYPFWGAIFFSISGMLSIISERRNATYLVRGSLGANTASSIAGGTGITILIINLKKSLAYIHIHSCQKFFETKCFMASFSTEIVVMMLFLTILGLGSAVSLTICGAGEELKGNKVPEKRGRKKLLYIFKQPFMRPVQTTQEEDGCSCRFPEEEEGGCELGSGVKQTLNFDLLKLAGDVESNPGPMIPAVVLLLLLLVEQAAALGEPQLCYILDAILFLYGIVLTLLYCRLKIQVRKAAITSYEKSRVKFSRSADAPAYQQGQNQLYNELNLGRREEYDVLDKRRGRDPEMGGKPRRKNPQEGLYNELQKDKMAEAYSEIGMKGERRRGKGHDGLYQGLSTATKDTYDALHMQALPPR

SEQ ID NO: 126 - DNA, 2547 bp, Artificialsequence
  Multi-chain CAR
atggctcctgccatggaatcccctactctactgtgtgtagccttactgttcttcgctccagatggcgtgttagcagaggtgcagttgcagcagtcagggccagagttgattaagcccggagcctccgtcaagatgtcctgcaaggccagcgggtacactttcaccagctacgtcatgcattgggtgaagcagaagccaggccaggggcttgagtggattgggtacatcaacccctacaacgacgggaccaaatacaacgagaaattcaagggcaaagccacactcacctccgataagtcctcctctaccgcctacatggagctcagctccctgacctccgaggatagcgctgtgtattactgcgcaaggggcacatactactatggctctagggtgttcgactactgggggcagggcactactctcacagtgagctcaggcggaggaggcagtggcggagggggaagtgggggcggcggcagcgatattgtcatgacccaggcagcccctagtatccctgtgactccaggcgagagcgtgagcatcagctgccggtccagcaagagcctgctgaacagtaacggaaacacatacctctactggtttctgcagaggcccggccagagccctcagctgctgatttaccgcatgtcaaatcttgcctctggggtgcccgatagatttagtgggagcggatccggcacagcttttacattgcggatctccagagtcgaggccgaagacgtgggggtctattactgtatgcaacacctggaatacccctttaccttcggagccggcacaaagctggagctgaagcgggctgacaccacaacccccgctccaaggccccctacccccgcaccaactattgcctcccagccactctcactgcggcctgaggcctgtcggcccgctgctggaggcgcagtgcatacaaggggcctcgatttcgcctgcgatttttttatcccattgttggtggtgattctgtttgctgtggacacaggattatttatctcaactcagcagcaggtcacatttctcttgaagattaagagaaccaggaaaggcttcagacttctgaacccacatcctaagccaaaccccaaaaacaacagagccgagggcagaggcagcctgctgacctgcggcgacgtggaggagaacccaggccccatggacacagaaagtaataggagagcaaatcttgctctcccacaggagccttccagtgtgcctgcatttgaagtcttggaaatatctccccaggaagtatcttcaggcagactattgaagtcggcctcatccccaccactgcatacatggctgacagttttgaaaaaagagcaggagttcctgggggtaacacaaattctgactgctatgatatgcctttgttttggaacagttgtctgctctgtacttgatatttcacacattgagggagacattttttcatcatttaaagcaggttatccattctggggagccatatttttttctatttctggaatgttgtcaattatatctgaaaggagaaatgcaacatatctggtgagaggaagcctgggagcaaacactgccagcagcatagctgggggaacgggaattaccatcctgatcatcaacctgaagaagagcttggcctatatccacatccacagttgccagaaattttttgagaccaagtgctttatggcttccttttccactgaaattgtagtgatgatgctgtttctcaccattctgggacttggtagtgctgtgtcactcacaatctgtggagctggggaagaactcaaaggaaacaaggttccagagaaacggggccggaagaagctcctctacatttttaagcagcctttcatgcggccagtgcagacaacccaagaggaggatgggtgttcctgcagattccctgaggaagaggaaggcgggtgcgagctgggttctggcgtgaaacagactttgaattttgaccttctcaagttggcgggagacgtggagtccaacccagggcccatgattccagcagtggtcttgctcttactccttttggttgaacaagcagcggccctgggagagcctcagctctgctatatcctggatgccatcctgtttctgtatggaattgtcctcaccctcctctactgtcgactgaagatccaagtgcgaaaggcagctataaccagctatgagaaatcaagagtgaagttctccaggagcgcagatgcccccgcctatcaacagggccagaaccagctctacaacgagcttaacctcgggaggcgcgaagaatacgacgtgttggataagagaagggggcgggaccccgagatgggaggaaagccccggaggaagaaccctcaggagggcctgtacaacgagctgcagaaggataagatggccgaggcctactcagagatcgggatgaagggggagcggcgccgcgggaaggggcacgatgggctctaccaggggctgagcacagccacaaaggacacatacgacgccttgcacatgcaggcccttccaccccggtga

SEQ ID NO: 127 - DNA, 17 bp, Artificial Sequence
  TRAC Left Half Target
ttgtcccacagatatcc

SEQ ID NO: 128 - DNA, 18 bp, Artificial Sequence
  TRAC Right Half Target
ccgtgtacccagctgaga

SEQ ID NO: 129 - DNA, 17 bp, Artificial Sequence
  CD52 Left Half Target
ttcctcctactcaccat

SEQ ID NO: 130 - DNA, 17 bp, Artificial Sequence
  CD52 Right Half Target
ggtacaggtaagagcaa

SEQ ID NO: 131 - DNA, 17 bp, Artificial Sequence
  Left Matched Sequence of Potential offsite target 1
ttgctctcaccagtata

SEQ ID NO: 132 - DNA, 17 bp, Artificial Sequence
  Right Matched Sequence of Potential offsite target 1
ttttcaggtaagtgcaa

SEQ ID NO: 133 - DNA, 17 bp, Artificial Sequence
  Left Matched Sequence of Potential offsite target 2
tcactcttacctggacc

SEQ ID NO: 134 - DNA, 18 bp, Artificial Sequence
  Right Matched Sequence of Potential offsite target 2
cctacaggttaagggcca

SEQ ID NO: 135 - DNA, 17 bp, Artificial Sequence
  Left Matched Sequence of Potential offsite target 3
tctcagatgatacaccc

SEQ ID NO: 136 - DNA, 17 bp, Artificial Sequence
  Right Matched Sequence of Potential offsite target 3
agtacaggcatgagcca

SEQ ID NO: 137 - DNA, 17 bp, Artificial Sequence
  Left Matched Sequence of Potential offsite target 4
tgatcccacagaaatac

SEQ ID NO: 138 - DNA, 17 bp, Artificial Sequence
  Right Matched Sequence of Potential offsite target 4
gcatttctgtgggatca

SEQ ID NO: 139 - DNA, 17 bp, Artificial Sequence
  Left Matched Sequence of Potential offsite target 5
ttcctctaacctgtatt

SEQ ID NO: 140 - DNA, 17 bp, Artificial Sequence
  Right Matched Sequence of Potential offsite target 5
gatccaggtaaggtcaa

SEQ ID NO: 141 - DNA, 17 bp, Artificial Sequence
  Left Matched Sequence of Potential offsite target 6
tagtcccccagatatga

SEQ ID NO: 142 - DNA, 17 bp, Artificial Sequence
  Right Matched Sequence of Potential offsite target 6
aaggtgtggatgaggaa

SEQ ID NO: 143 - DNA, 17 bp, Artificial Sequence
  Left Matched Sequence of Potential offsite target 7
ttgtcacacatataccg

SEQ ID NO: 144 - DNA, 17 bp, Artificial Sequence
  Right Matched Sequence of Potential offsite target 7
tggtatttgtgtgacaa

SEQ ID NO: 145 - DNA, 17 bp, Artificial Sequence
  Left Matched Sequence of Potential offsite target 8
taactcttacctgtagt

SEQ ID NO: 146 - DNA, 17 bp, Artificial Sequence
  Right Matched Sequence of Potential offsite target 8
agatttctctggggcaa

SEQ ID NO: 147 - DNA, 17 bp, Artificial Sequence
  Left Matched Sequence of Potential offsite target 9
ttactccaactaactat

SEQ ID NO: 148 - DNA, 17 bp, Artificial Sequence
  Right Matched Sequence of Potential offsite target 9
ccgtttaccggcttaga

SEQ ID NO: 149 - DNA, 17 bp, Artificial Sequence
  Left Matched Sequence of Potential offsite target 10
tggctcatacctgtagt

SEQ ID NO: 150 - DNA, 17 bp, Artificial Sequence
  Right Matched Sequence of Potential offsite target 10
aggatgaggtggaggaa

SEQ ID NO: 151 - DNA, 17 bp, Artificial Sequence
  Left Matched Sequence of Potential offsite target 11
ttgctcatacatgtgca

SEQ ID NO: 152 - DNA, 17 bp, Artificial Sequence
  Right Matched Sequence of Potential offsite target 11
atgctgtgtaggtggta

SEQ ID NO: 153 - DNA, 17 bp, Artificial Sequence
  Left Matched Sequence of Potential offsite target 12
ttgtcccacagacattc

SEQ ID NO: 154 - DNA, 17 bp, Artificial Sequence
  Right Matched Sequence of Potential offsite target 12
ccacgtagcagctggga

SEQ ID NO: 155 - DNA, 17 bp, Artificial Sequence
  Left Matched Sequence of Potential offsite target 13
tcacacctggtacatag

SEQ ID NO: 156 - DNA, 17 bp, Artificial Sequence
  Right Matched Sequence of Potential offsite target 13
gtgtttagtagggggaa

SEQ ID NO: 157 - DNA, 17 bp, Artificial Sequence
  Left Matched Sequence of Potential offsite target 14
ttgtcccacagctaccc

SEQ ID NO: 158 - DNA, 17 bp, Artificial Sequence
  Right Matched Sequence of Potential offsite target 14
gagtctttgtaggacaa

SEQ ID NO: 159 - DNA, 17 bp, Artificial Sequence
  Left Matched Sequence of Potential offsite target 15
tctcaactgaaacaagg

SEQ ID NO: 160 - DNA, 17 bp, Artificial Sequence
  Right Matched Sequence of Potential offsite target 15
tgtaatgtcaagagcaa

SEQ ID NO: 161 - DNA, 116 bp, Artificial Sequence
  Wild Type Sequence (TRAC locus)
catgtcctaaccctgatcctcttgtcccacagatatccagaaccctgaccctgccgtgtaccagctgagagactctaaatccagtgacaagtctgtctgcctattcaccgattttg

SEQ ID NO: 162 - DNA, 99 bp, Artificial Sequence
  Mutated sequence (TRAC locus)
catgtcctaaccctgatcctcttgtcccacagatatccgtgtaccagctgagagactctaaatccagtgacaagtctgtctgcctattcaccgattttg

SEQ ID NO: 163 - DNA, 107 bp, Artificial Sequence
  Mutated sequence (TRAC locus)
catgtcctaaccctgatcctcttgtcccacagatatccagatatccgtgtaccagctgagagactctaaatccagtgacaagtctgtctgcctattcaccgattttg

SEQ ID NO: 164 - DNA, 85 bp, Artificial Sequence
  Mutated sequence (TRAC locus)
catgtcctaaccctcgatcctgccgtgtaccagctgagagactctaaatccagtgacaagtctgtctgcctattcaccgattttg

SEQ ID NO: 165 - DNA, 111 bp, Artificial Sequence
  Mutated sequence (TRAC locus)
catgtcctaaccctgatcctcttgtcccacagatatccagatatcctgccgtgtaccagctgagagactctaaatccagtgacaagtctgtctgcctattcaccgattttg

SEQ ID NO: 166 - DNA, 104 bp, Artificial Sequence
  Mutated sequence (TRAC locus)
catgtcctaaccctgatcctcttgtcccacagatatccagaaccctgaccagctgagagactctaaatccagtgacaagtctgtctgcctattcaccgattttg

SEQ ID NO: 167 - DNA, 45 bp, Artificial Sequence
  Mutated sequence (TRAC locus)
catgtcctaaccctgatcctcttgtcccacagatatccgattttg

SEQ ID NO: 168 - DNA, 78 bp, Artificial Sequence
  Mutated sequence (TRAC locus)
catgtcctaaccctgatcctcttgtcccacgagactctaaatccagtgacaagtctgtctgcctattcaccgattttg

SEQ ID NO: 169 - DNA, 109 bp, Artificial Sequence
  Mutated sequence (TRAC locus)
catgtcctaaccctgatcctcttgtcccacagatatccagaacctgccgtgtaccagctgagagactctaaatccagtgacaagtctgtctgcctattcaccgattttg

SEQ ID NO: 170 - DNA, 89 bp, Artificial Sequence
  Mutated sequence (TRAC locus)
catgtcctaaccctgatcctcttgtcccacagaccagctgagagactctaaatccagtgacaagtctgtctgcctattcaccgattttg